European Patent Specification EP 3 485 907 B1, published June 28, 2023. Title: PROTEINS AND NUCLEIC ACIDS USEFUL IN VACCINES TARGETING KLEBSIELLA PNEUMONIAE. Applicant: EVAXION BIOTECH APS. The sequence listing filed with the application follows.

SEQUENCE LISTING (102 sequences)

SEQ ID NO: 1 - protein, 94 aa, Klebsiella pneumoniae
MKKLALLSAVMTLGMSSWAFAADNPPPPPEKGAQHQGKPPVKNGQHEGKQAQYNRKQPQRDGKQPQHDGKQPQHNGKQPPKGSEHSGKPLPPKA

SEQ ID NO: 2 - protein, 117 aa, Klebsiella pneumoniae
MKRYATALLFCTLSLTSLAARADIIDDAIGNIQQAINDAYNPGSSRSDDDDRYDDDGRYDDGRYQGSRQQSRDSQRQYDERQRQLDERRRQLDERQRQLDRDRRQLESDQRRLDDSY

SEQ ID NO: 3 - protein, 119 aa, Klebsiella pneumoniae
MFRSLILAAVLLAAGPLVANAGEITLLPSVKLQIGDRDNYGNYWDGGSWRDRDYWRRHYEWRDNRWHRHDNGWHKGWYKGRDKAWERGYRAGWNDRDDHRGGWGRGPGGRGHGHGHGHH

SEQ ID NO: 4 - protein, 120 aa, Klebsiella pneumoniae
MKEIGLPLLLLTALASPAFAADCQPNGIGGSFCINDDGTTTDTVPNEVNGMDTYSNNGGYTSSLPDRSGADEALEGSSLSTQQGVGSGQSDSALAGRDWHSPANLNDGAATSSMSLLDKP

SEQ ID NO: 5 - protein, 121 aa, Klebsiella pneumoniae
MNMKKLTTLLLTATLGLASGAALAADTGAQSNNGQANSSADAGQVAPDARENVAPNNVDNSQINSGSGGTTGSTMTQDNMSSNEVHKNSMCKDGRCPDTGKKLDNGGNTTQDNSKTDGTTQ

SEQ ID NO: 6 - protein, 122 aa, Klebsiella pneumoniae
MKHRIALLLVLTSLSASALAASPCQEKEQDIQREISYAEKHHNQSRIDGLNTALRQVRENCSDSKLKADHQQKIAKQREEIAERQRDLQEARKKGDADKINKRQHKLNEAQQELKTLESRDY

SEQ ID NO: 7 - protein, 141 aa, Klebsiella pneumoniae
MRLITRHVREDIMKKAMIALSAILVAAPVFAATTHATDDTVAAANANANTAKEKLHQAQHEGEEQQLKAKHAAEGKQDSVGSQVSEGAQKTWNKTKEGTEKGWDKTKEVSEKGWNATKSGAEKGWDKTKTGAEELKNKVTE

SEQ ID NO: 8 - protein, 151 aa, Klebsiella pneumoniae
MKKMISLAVILSCVLSVPAFADGPNDGHRPEQPTVWQNGPDHDGHAPQGGPDAHHQGDHDQRGPDRDGHDKRDLARHEQDHFAWRGNDFRKGHPAPAPFRGDEYRVRDWSDRGLPPPPEGHHWSYIDGNYVLIAAATGIITSILVSGALGH

SEQ ID NO: 9 - protein, 168 aa, Klebsiella pneumoniae
MKKPTSATRGKSGRKSREELNQEARDRKRQKKHRGHAAGSRANGGDAASAGKKQRQAQDPRVGSKKPIPLGVSESSVPAPKQHKPKSEKPMLSPQAELELLENDERLDALLERLEEGGTLNAEEQSWVDAKLDRIDELMQQLGLSYDDEDEEEEERQEDMMRLLKGGN

SEQ ID NO: 10 - protein, 229 aa, Klebsiella pneumoniae
MASKFQNRLVGTIVLVALGVIILPGLLDGQKKHYQDEFAAIPLVPKPGDRDEPDMLPAATQALPSQPPEGAAEEVRAGDAAAPSLDPSRIPVNSNSFDDVQEPVVAAKPQPKPQPKPQPQQQASTPTPPPAKPQQQQPPQQQAALPAPTGKAYVVQLGALKNADKVNEIVGKLRASGFKVYTSPSTPVQGKITRILVGPDASKDKLKGQLGDLQQISGLSGVVMGFTPN

SEQ ID NO: 11 - protein, 322 aa, Klebsiella pneumoniae
MAQRDYVRRSQPASSRRKKSTTRSSRNKQSSLPAISPAMVAIAAAVLVAFIGGLYFITHHKKEEAEAMQNRQAAGNGLPPKPEERWRYIKELESRQPGVRAPTEPTAGGEVMKPEQLTDEQRQLLAQMQADMRQQPTQLTEVPWNEQTPAQRQQTLQRQRLAQQQQQAQQQQWAQTQAQTVQQQPPRVQQPKPVQQQQPKQTASNQQPYQDLLQTPAHTNTTQPRTQAAAPVTRVEEAPKTTAEKKDDRSWMIQCGSFKGAEQAETVRAQLAFEGFASHITTNNGWNRVVIGPLKGKESANEMITRLKMAGHANCIRLAARG

SEQ ID NO: 12 - protein, 376 aa, Klebsiella pneumoniae
MSAGSTKFTVSRIAALSLVSLWLAGCTNTNNPPAPVSSAGGAASSSTNSGMLITPPPSGVKSAPQAQPIQPMQTQTIQPAPVAQEPVQTVNGRIVYNRKYGDIPKGSYTGGSTYTVKRGDTLFYIAWVTGNDFRDLAQRNNIPAPYALNVGQVLQVGNASGQPITGENAVSQASARASGGATTSTTSAQKSTAVVASQPTITYSESSGEQSATKMLPNNKPATTTTTVVAPVTAPTTVSTTQPTASSTSTSSPISAWRWPTDGKVIENFSGAEGGNKGIDIAGSKGQAIVATADGRVVYAGNALRGYGNLIIIKHNDDYLSAYAHNDTMLVREQQEVKAGQKIATMGSTGTSSTRLHFEIRYKGKSVNPLQYLPQR

SEQ ID NO: 13 - protein, 382 aa, Klebsiella pneumoniae
MRKQWLGICIAAGLLAACSSDDVQQKTVSTPQPAVCNGPTVEISGADPQYETPNATANQDYERDGKSYKIVQDPANFTQAGFAAIYDAEPNSNLTASGEAFDPTQLTAAHPTLPIPSYARITNLANGRMIVVRINDRGPYGNDRVISLSRASADRLNTSNNTKVRIDPIIVAPDGSLSGPGMACTTVAKQTYALPARPNLDGGDAAGMSQPAPTDVRPISNSTLTPADSVGAPVNSGGFLGAPTPLNNGVLESSEPAAAAATAPAAGATPTAPVTAPGSIQGNVVPAAATAAAAGAVAASSSATSSASGNFVVQVGAVSDQTRAQQYQQRLSQQFSVPGRVMQNGAVWRIQLGPFADKAQASAVQQRLQSEAQLQSFITRAN

SEQ ID NO: 14 - protein, 428 aa, Klebsiella pneumoniae
MDDFKPEDDMKADRNDRRAGRSRQSSERDADPQINFDDVDLDADEGRPTRAGKARREREEEEFEEELDAQDEEMLEEQPVERRPRKRKKAPAKPASRQYIMMGVGILVLLLLIVGIGSALKSPSSSSQQTASGEKSINLSDDQSASMPAAGQDQTAAANSTSQQDVTVPPIAANPTQGQAAVAPQGQQRIEVQGDLNNALTQQQGQLDGAVANSTLPTEPATVAPIRNGANGTAAPRQATERQTAATPRPAERKHTVIEAKPQSKPQAVAKTPVESKPVQPKHVESTATTAPAKTSVSESKPVATAQSKPTTTTAAPAATAAAAAPAAKTGKTAGDVSSMKTAPSGHYTLQLSSSSNYDNLNNWAKKEKLDKYVVYETSRNGQPWYVLVSGIYASKDEAKRAVTSLPADVQAKNPWAKPLHQVQADLK

SEQ ID NO: 15 - protein, 441 aa, Klebsiella pneumoniae
MSKATEQNDKLKRAIIISVALHIILIALLIWSSFDEHLDASAGGGGGSSIDAVMVDPGAVVNNYNRQQQQQASARRAAEQREKQAQQQAEELREKQAAEQERLKQLEQERLQAQEAAKEAKEQQKQAEEAAAKAAAAAKAKADAQAKEAQEAAAKAAAEAKAKADAQAKAAEQAAAKAAADAKKQAEAAAAKAAAEAKKQAEAEAAKAAAEAQKKAEAAAAKKAQQEAEKKAQQEAAKQAAAEKAAAEKAAEKAAAQKAAAEKAAAEKAAAAEKAAAAKAAAAEKAAADKAAKAAAAKAAAAKKAAAAKEADGVDNLLGDLSSGKNAPKTGGGAKGNNASAAGSGNTKNSASGADINNYAGQIKSAIESKFYDASSYAGKTCTLRIKLAPDGLLLNIQSEGGDPALCQAALAAARQAKFPKPPSQAVYEVFKNAPLDFKPQ

SEQ ID NO: 16 - protein, 484 aa, Klebsiella pneumoniae
MFFLSIFYMEMTKVKLSALFIALIPLLGSPVIHAETTAAPVLENRAAQGDITTPGGARRLTGDQTEALRASLINKPAKNVILLIGDGMGDSEITAARNYAEGAGGFFKGIDALPLTGQYTHYSLDKKTGKPDYVTDSAASATAWTTGVKTYNGALGVDIHENAHQTILELAKAAGLATGNVSTAELQDATPAALVAHVTSRKCYGPTVTSEKCPSNALEKGGKGSITEQLLNARPDVTLGGGAKTFTETATAGEWQGKTLREQAQARGYQIVTDAASLAAATEASQDKPLLGLFADGNMPVRWEGPKASYHGNIDKPPVTCTPNPKRDASVPTLAQMTEKAIDLLSRNEKGFFLQVEGASIDKQDHAANPCGQIGETVDLDEAVQKALEFARKDGNTLVIVTADHAHASQIIPADSKAPGLTQALNTHDGAVMVMSYGNSEEESMEHTGTQLRIAAYGPHAANVVGLTDQTDLFTTMKAALSLK

SEQ ID NO: 17 - protein, 535 aa, Klebsiella pneumoniae
MSLPFKPHIIALLCSAGLLAAAGTLYVQSRTPATIAEPPAQQAPAPAASTTQPVAATYTQAQIDQWVAPIALYPDSLLSQVLMASTYPDNVLQAVQWSQDNPAMKGDAAVQAVASQPWDPSVKSLVAFPALLAMMGENPPWVENLGNAFLAQPHDVMDSVQRLRAIAQQTGTLKSTPQQKVIVTPAAPVSASSSTAATATAHTAAPAPTQVIKIEPTNPQVVYVPSYNPSTVYGTWPNSAYPPVYLPPPPGEQFTDSFVKGFGYSLGVATTWALFSSIDWDDDDHHHHDDDYHHGDYSHNGDNININVNNFNHITGENLPGNHVNWQHNPAYRGHTPYPDNTVAQRFHQTNVSGGLSATQHAPVDREAQRQAAMTQLQHNVPTATAGNLAANNASRDAQRQAASAQLKQATQRSNYRGYDSTPTQQQRREAAKTQLKNPTPQQQQRREAARSHEQNRTPQQQQRRQQFQSATPAQRQQTLSHLRANALSGNESRAPSWQAQQERGLQSRQFSGVNRELRDGTRERLSEHHELRRR

SEQ ID NO: 18 - protein, 597 aa, Klebsiella pneumoniae
MFKFKASYVALAAVLTSSVVYADPTSYTHSSGATVIDIEKPNAAGVSHNLYRDFNVGANGTILNNSGDDVSHSTFGNIARNNNLTAGSASVILNEVTSKNASSLKGFIEVNGQKADVVIANPNGITCSGCSFVNTNKAILTTGKVNMTDDGAIGSYTVTGGTLTIGENGMNAANGYAVLLADAININGKVQANNALVSAGNFTMDNSSGSVTSAGKKATLIQMTVNPQYSIDVSSLGGIEANSISMVGNNIGFGVRNKGSIVANSSLQLTSNGNLLNKGTIKSNGLLSQVATASGITNDGSIAGAYYLMLSSGDYIVNTGSLSGGQLIATANGNITNGDSGTMTGTSGLSLTSGGKIRNEEKASLLSNNQIAATAIGDFLNEGKISAKHTSLTFVGDSFKNTGNINSTGQTTIQSLKQDGSANTGEIYNLGNITGENINLQTNGTLAQSSSGRIEATNAITAHSYWLNQNGYMNAADITTDHGVVNNYGNITAKNISITTYSDITNEGQISSTGDLTLNTKNKGAIYNYSTLSAGGNMTLTATKVVNGGKSCGILGLAKCGVGTLTADKLVLNSSQKYVSDMGGKQYFKSTEVNTVK

SEQ ID NO: 19 - protein, 624 aa, Klebsiella pneumoniae
MMDNLRTAANSVVLKIIFGIIIVSFILTGVSGYLIGGGKNYAAKVNGQEIGRGQFENAVASERNRMQQQLGDQFSELAANENYMKTMRQQVLNRLIDESLLDQYARELGLSISDEQVKQAIFQTQAFQTNGKFDNQRFSGIVAQMGMTTDQYAQALRNQLTTQQLINAIAGTDFMLPGESDQLAALVSQQRVVREATINVNALAAKQTASDEEINAFWQQNQARFMAPEQFRVSYIKMDAASMQESASDEEIQSWYDQHKDQFTQPQRNRYSVIQTKTEADAKAVLAELQKGADFATLAKEKSTDIISARNGGDMGWMEDASTVPELKDAGLKEKGQLSGVIKSSVGFLVARLDDVQPAQVKPLADVRNDIAAKVKQEKALDAYYALQQKVSDAASNDNESLASAAQVAGLKVVETGWFGRDNLPEELNFKPVADAIFNGGLVGENGAPGSNSDIITVDGDRAFVLRISEHKAEAVKPLAEVKAQVSDIVKHNKAEQQAKLEADKLLAALKDGKGDEAMKAAGLSFGAPQTLSRTGQDPLSQLAFTLPLPQQGKPVYGVGSNMQGDVVLVALDEVKAGSMPEEQKKAMVQGITQNNAQIAFEALMSNLRKAAKIKLGDSIDQQQ

SEQ ID NO: 20 - protein, 657 aa, Klebsiella pneumoniae
MFRLNPFIRAGLSASVVSLAFPALADVNEETLVVTASATEQNVKDAPASISVITQQDLQRKPVQNLKDVLRDVPGVQLTNEGDNRKGVSIRGLSSSYTLILVDGKRVNSRNAVFRHNDFDLNWIPVDAIERIEVVRGPMSSLYGSDALGGVVNIITKKIGQKWTGTLSADTTIQEHRDRGDTWNGQFFTSGPLIDGVLGMKAYGSLAKRAKDDPQSSSNATGETPRIEGFTSRDGNVEFAWTPNENHDFTAGYGFDRQDRDSDSLDRNRLERENYSLSHNGRWDIGNSELKFYGEKVDNKNPGQSGTITSESNAIDGKYVLPLGMINQLVTFGGEWRHDKLKDPVNLSSGGQSTSASQYALFIEDEWRIIEPLALTTGIRMDDHQTYGDHWSPRAYLVYNATDTVTVKGGWATAFKAPSLLQLNPDWTTNSCRGSCSIVGNPDLKPETSESFELGLYYRGEEGWLENVEGSITTFQNNVDDMIDVLRTSSASEAPGYPNFVGWKTVNGKRVPIFRYFNVNKARIKGVETEVKIPFGDEWKLTVNYTYNDGRDLSNGGDKPLQTLPFHTANGTLDWKPLDDWSFYVTANYTGQQRAVSATGKTPGGYTLFDVGAAWQVTKNVKLRSGVQNVGDKDLSRDDYSYTEEGRRYFMAVDYRF

SEQ ID NO: 21 - protein, 675 aa, Klebsiella pneumoniae
MNRAATLTLNAPLLMLVAALALSTPFTAGAAPAFLDYAQQQTQQSQAQEKNDAASAKQTQESRQSADNKKTGTSTSQLQKRITSQQAAIAQKDKLIQQLKKQLAATPQTDTAGANEQAALNKRINELQVALSAATAEKEALIKKAGVVQNNNLQQSQAAARQQIQQLTTQIQQAEAENKRLSASFTTLNKDKHALMTQLAATEKEKQAALEQVKALNADKQPLTTRLAAAEKEKQAVLEQVKALNADKQSLTIRLAAAEKAQQAAVDQAKALNADKQPLATRLAAAEKEKQAVLEQVKALSADKQSLTIRLAAAEKAQQAALDQAKALNADKQPLATRLAAAEKEKQAVLEQVKALNADKQSLTIRLAAAEKTQQAALDQVKALNADKQSLSTRLAAADKAPHGPANDAAAPKNEPPEMAAIVAAYRLQADKDNAQLRMKEDEIELLRTQLSVQSKTRSGESAAAKLSASGEQQAYAIGASMGSEALNVLTTRRTQGVTVDAGLVLQGIEDAFRGQLRLGEQERNKALFDVSQQVFQNLNKIEQKNISAGKKYQQAFARKKDVVFKEGVYSRVDYLGKGKISGNDLVTVVIKEMLTDGTVINDMEAKDQALTQKLDAYPPVFREPLKRLQNHGSVTLVVPPEKAYGSKGLPPKIPPGATMVYSVRIVDSQPEPAK

SEQ ID NO: 22 - protein, 701 aa, Klebsiella pneumoniae
MKILSVRHAALPALLLPLIAAAQAADEQTMVVTAAPTTVSELDTPAAVSVVNGDEMRQAAPRVNLSESLGAVPGLQVQNRQNYAQDLQLSIRGFGSRSTYGVRGLRIYVDGIPATMPDGQGQTSNIDIGSVDTIEVLRGPFSALYGNSSGGVINVTSQTGTQPPTVEASSYYGSFGTWHYGMKATGAVGDGSHAGDVDYTVSTNRFTTHGYRDHSGARKNLANARLGVRINDVSKLTLLLNSVDIKANDAGGLTADEWRDNPRQSPRGDQYNTRKNTRQTQAGLRYERQLSAQDDLSVMMYAGERETTQFQSIPRAPQLKPSHAGGVIDLTRHYQGIDTRLTHRGELLVPVTLTAGLDYENMSERRKGYENFVMVNGAPQYGEQGALRRNERNLMWNVDPYLQTQWQLTDKLSLDAGVRYSSVWFDSNDYYITPGNGDDSGDASYHKWLPAGSLKYALTDAWNVYLSAGRGFETPTINELSYRSDNQSGLNFGLKPSTNDTVEIGSKTRIGNGLFTAALFQTNTDNEIVVDSSSGGRTSYKNAGKTRRQGMELGLDQQFGESWRLKAAWTWLDATYRTNVCDDASCNGNRIPGIARNMGYASFGYQPEQGWYAGSDIRYMSDIMANDENTAKAPSWTVVGLTTGYKWSYGRMDMDLFGRIDNLFDREYVGSVIVNESNGRYYEPAPGRNYGIGLNLAWRFE

SEQ ID NO: 23 - protein, 752 aa, Klebsiella pneumoniae
MKYTSHFPLGIVIPLLACSVPLQAAENMTEQSTPDESAATAENHEETMVITAARQNLQAPGVSTITAEEIRKHPPARDVSELIRTQPGVNLTGNSTSGQRGNNRQIDIRGMGPENTLVLVDGKPVTSRNSVRYGWRGDRDSRGDTSWVPAEMIDHIDVIRGPAAARYGNGAMGGVVNIVTKPTTREWHGSWNTYMNAPQHRKEGATKRTNFSLNGPLSDSVSFNLWGNLSKTQADAQDINAGHEAERTGSYAGSYPAGREGVVNKDIHSKLRWEFAPMQALEFEAGYSRQGNLYAGDTQNTNTSTLVKSMYGKETNRLYRQTYGVTWTGGWDNGVTSNSYAQYEHTRNSRMDEGLAGGTEGIFSSSEFSDIDLADVLLHSEVNIPFTLGVDQNLTLGAEWNQQRMKDGVSTTQALSYGTIDGVSATGRSPYSSAEIFSLFTEDNMALTDSTMLTPALRFDHHSIVGNNWSPSLNLSQELTDDWTLKLGIARAYKAPNLYQLNPNYILYSNGQGCYASSSACYLMGNSDLKAETSVNKEIGLEYKHDGYQAGITWFRNDYHNKIESGYAAVGTASNGTTNIYQWENVPKALVEGLEGTLNLPVGEAVNWSNNLTWMLQSKNKTTGDRLSVIPQFTLNSTLSWQVREDLSLQSTFTWYGRQKPKRFNYKGEAVSGSELNEVSPYSIVGLSATWDVNKNLSFTSGIDNLFDIRHYRAGNAQTTGNATTGAYLYGAGAETYNESGRTFFMSVNTHF

SEQ ID NO: 24 - protein, 761 aa, Klebsiella pneumoniae
MEKNASLPFGSFNSLALFTGLCLGASPAAGIAAENSVKNSEETLVVEAAPPSLYSPGASADPKFNKPLVDTTRTITVIPEQVIKDQGVTNLTDALKNVPGVGAFYAGENGSSTTGDAIFMRGVDTSNSIYVDGIRDIGSVTRDTFNTQQVEVIKGPAGTDYGRSAPSGSINMISKQPRLDSGIDGSASIGSAWSRRGTLDLNQAFSDNAAFRLNLMGEKTHDAGRDRIENERYGIAPSLAFGLDTPTRLYLNYLHVRQNNTPDGGIPTVGLPGYSAPSPKYAALNSAGKVDTSNFYGTDSDYDKSTTDSGTLRFEHDLTENTTVRNTTRWSRVKQEYLLTAVMGGANNITAPDINDVNTWSWSRLVNTKDVSNRILTNQTNITSTFNTGSIGHDVSAGVEFTRENQTNYGVNARTAPAVNLYHPVSNLSIGGLDRNGANANGQTDTFGIYAFDTLTLTERIEINGGLRLDNYHTKYDSATACGGSGRGAIACPPGQSTGSPVTTVDTAKSGNLVNWKAGALYRLTEQGNVYVNYAISQQPPGGSSFALAASGSGNSANRTDFKPQKAKSSELGTKWQIFDNRLLLSAALFRTDIENEVAANDDGTWSQYGKKRVEGYELSATGNLTPDWTIIAGYTQQHATVTEGQNVAQDGSSALAYTPKHAFTLWTQYQATSDLSVGGGVRYVGSLRRGSDGAVGTPDHTEGYWVADAKLGYRVNSNLDLQLNMYNLFDTDYVASINKSGYRYHPGEPRTFMLTANVHF

SEQ ID NO: 25 - protein, 790 aa, Klebsiella pneumoniae
MATMYKSTPSAAWCKKRLLVTSLFAAIYQTSAIAADTSAVSGEAVDDTSEQMTVTAPAPVQKAGSEHSISARELENKGANDFGSIMRYEPLISATGASGGSGNGKSGFDRGGYTGYNIRGMESNRVGIDVDGIAQPNATGRGYVGRAGLNTFGIGRDYIDPYMYGSVDIQSGATSTETANSAIGGNVSFRPKSADDYLRPGKTSAFGYRSGYDSADRSWHNGVTVAGGDEFLRGILVYSRRDGQETENNSGTVDAYPANWHSDAFLASGIWQPNDEHKLTSTFDYYHKTNHTHYDTWDSSGNSTIGTANQTSQTRRWGLSLKDDWTPMNDYLDSVSTKIYYQHTEAHDWTYMPDSVTRKMQTVNSNYDTDTWGLQTALAKTLGRHDLSAGFNASTSKTQRPFSQSPIPSVYSEIMQPEADSRSYTLGGFVQDKINFDLDSHNFAVIPGVRVVHQSTKPENLSDLAANSSVLSESSVANLYGKNSDTQVLPSLTFQYDLTPRLMTYLQYQRGAQFPNASQLYGSWNLGSSYAGSQQYALIGNTDLKTETSDNLEWGLKGEVTEGITLRTALFYNSYKNFIAYTRYTRANNPGQFTNVPSNIYTIYQAENRDKAYIYGGEISTKFNFGTWFEQVDGLSATLALGYSEGKSKSSYSGDKYVDLDSVAPMKAIVGVAWDDPAKRYGTALTATFVKGKQATATNRESYSNSGSAITDASSDYMRVPGYGMLDWTAYWQVAKNVRLNGGVYNLTDRKYWDYLSSRNIETGTNQDANDKALAVMPGRTWQLGVNVDF

SEQ ID NO: 26 - protein, 809 aa, Klebsiella pneumoniae
MAMKKLLIASLLFSSATVYGAEGFVVKDIHFEGLQRVAVGAALLSMPVRPGDTVTDDDISNTIRALFATGNFEDVRVLRDGDTLLVQVKERPTIASITFSGNKSVKDDMLKQNLEASGVRVGESLDRTTIADIEKGLEDFYYSVGKYSASVKAVVTPLPRNRVDLKLVFQEGVSAKIQQINIVGNHAFSTDELISHFQLRDEVPWWNVVGDRKYQKQKLAGDLETLRSYYLDRGYARFNIDSTQVSLTPDKKGIYITVNITEGDQYKFSGVQVTGNLAGHSAEIEALTKVEPGELYNGAKVTKMENDIKKLLGRYGYAYPRVQSQPEINDSDKTVKLHVNVDAGNRYYVRKIRFEGNDTSKDAVLRREMRQMEGAWLGSDLVDQGKDRLNRLGFFETVDTDTQRVPGSPDQVDVVYKVKERNTGSFNFGIGYGTESGVSFQAGVQQDNWLGTGYAVGINGTKNDYQTYTELSVTNPYFTVDGVSLGGRVFYNDFDANDADLSDYTNKSYGTDITLGFPVNEYNTLRAGVGYVHNSLSNMQPQVAMWRYLNSMGQYPDNTNDRNSFSANDFTFNYGWTYNKLDRGFFPTEGSRVNLNGKVTIPGSDNEYYKATLDTATYVPIDNDHQWVVLGRTRFGYGDGIGGKEMPFYENFYAGGSSTVRGFQSNTIGPKAVYFPASSRHDDDDSYDNECKSTESAPCKSDDAVGGNAMAVASLELITPTPFISDKYANSVRTSVFWDMGTVWDTHWDSSAYAGYPDYSDPSNIRMSAGIAVQWMSPLGPLVFSYAQPFKKYDGDKAEQFQFNIGKTW

SEQ ID NO: 27 - protein, 896 aa, Klebsiella pneumoniae
MTDVTIKALASEIQTSVDRLIQQFADAGIRKSADDSVTSQEKQTLLTHLNREHGSAPDKLTLQRKTRSTLNIPGTGGKSKSVQIEVRKKRTFVKRDPQEAERLAAEEQAQREAEEQARREAEEAAKREAQLKAEREAAEQAKREVADKAKREAAEKDKVSNQHTDEMTKTAQAEKIRRENEAAELKRKSEEEARRKLEEEARRVAEEARRMAEENEKNWSETSDSPEDSSDYHVTTSQHARQAEDDNDREVEGGRGRSRSSKAARPAKKGNKHAESKADREEARAAVRGGKGGKHRKGSALQQGFQKPAQAVNRDVVIGETITVGELANKMAVKGSQVIKAMMKLGAMATINQVIDQETAQLVAEEMGHKVILRRENELEEAVMSDRDTGAAAEPRAPVVTIMGHVDHGKTSLLDYIRSTKVASGEAGGITQHIGAYHVETDNGMITFLDTPGHAAFTSMRARGAQATDIVVLVVAADDGVMPQTIEAIQHAKAAQVPVVVAVNKIDKPEADPDRVKNELSQYGILPEEWGGESQFVHVSAKAGTGIDDLLDAILLQAEVLELKAVRNGMASGAVIESFLDKGRGPVATVLVREGTLHKGDIVLCGFEYGRVRAMRDELGREVLEAGPSIPVEILGLSGVPAAGDEVTVVRDEKKAREVALYRQGKFREVKLARQQKSKLENMFANMTEGEVHEVNIVLKADVQGSVEAISDSLLKLSTDEVKVKIIGSGVGGITETDATLAAASNAILVGFNVRADASARKVIEAESLDLRYYSVIYNLIDEVKAAMSGMLSPELKQQIIGLAEVRDVFKSPKFGAIAGCMVTEGTIKRHNPIRVLRDNVVIYEGELESLRRFKDDVNEVRNGMECGIGVKNYNDVRVGDMIEVFEIIEIQRSID

SEQ ID NO: 28 - protein, 1077 aa, Klebsiella pneumoniae
MKRMLINATQQEELRVALVDGQRLYDLDIESPGHEQKKANIYKGKITRIEPSLEAAFVDYGAERHGFLPLKEIAREYFPANYNAHGRPNIKDVLREGQEVIVQIDKEERGNKGAALTTFISLAGSYLVLMPNNPRAGGISRRIEGDDRTELKEALASLELPDGMGLIVRTAGVGKSAEALQWDLSFRLKHWEAIQKAAESRPAPFLIHQESNVIVRAFRDYLRQDIGEILIDNPKVLELARQHIAALGRPDFSSKIKLYTGEIPLFSHYQIESQIESAFQREVRLPSGGSIVIDSTEALTAIDINSARATRGGDIEETAFNTNLEAADEIARQLRLRDLGGLIVIDFIDMTPVRHQRAVENRLREAVRQDRARIQISHISRFGLLEMSRQRLSPSLGESSHHVCPRCSGTGTVRDNESLSLSILRLIEEEALKENTKEVHAIVPVPIASYLLNEKRAAVSAIESRQGDVRVIIVPNDEMQTPHYSVLRVRKGEETSTLSYLLPKLHEEEMALPGDDEPAERKRPEQPALAAFVMPDAPPAPMLEEPAAAPVAAAAPVAAAAPAQPGLLSRFFSALKNIFSGAEEAKPAEVQVEKKAEEKPERQQERRKPRANNRRDRNDRRDNRDNRDNRDNRDNRDTRADNAEGREPRESREENRRNRREKPSQNVEARDVRQTSGDDAEKAKSRDEQQPRRERTRRRSDDKRQAQQEAKAQTREEPVVQETEQEERVQTLPRRKPRQLAQKVRVESAVVEPVAEIVPEAVVAEVIAPHSEPVKAELPAGVESVADQDENGESREANGMPRRSRRSPRHLRVSGQRRRRYRDERYPTQSPMPLTVACASPEMASGKVWIRYPVVRPQDQQPEEVQVQDASVAKTVEAVAAPVAVVETVTAAPVTVEPATMEPVTAEPVVVEPVAAAEPLVVDAAEVVAPAAVEPAPQEPVTEAPAVEAPQAIAPVTLDAEPVVVEPEAVETTPVVAAPVETIAPVAETVEQAPVTEAAPAEPVKAEPPVSKPVVVAGHRHATAPMTRAPAPDYVPEAPRHSTWVRPPFAFEGKGAAGGHSATHKATAEPTRPQPVE

SEQ ID NO: 29 - protein, 1159 aa, Klebsiella pneumoniae
MRKLSLSLLTLSLGVALLPLAQAATTPAQEHLLEQVRLGEASNREDLVRQSLYRLELIDPNNPELIAARMRYLLRQGDAAGAQKELERLTKQAPDSPELKASRNEMKSNTGEGRQALQQARLLGVAGKVDEAIAAYEKLYGGVPDDVDVAIEYWTLVARLPARHSEGVSQLKKLNASAPGNVSLLTSLAKQMFADNKPQEGFAYLAEMARSASGRGIAADMWFSEVKSMPVSKASVQALQQFLLQFPTGSVAANARVLLDQQQAQLQDPTFRARSEGLAAVKSGNTTQAVADLQKAVQADSRDSDAVGALGQAYSQRGDRARAVAQLSKAIAMDPDSPNRGKWDSLLQTNRYWLLIKQGDNALKAGQLSQAQNYYAQAQRVDRTDSYAVLGLGDVAAARKEAAAAERYYQQALRLDRGNNLAVRGLANLYRAESPEKASAWIAGLPPAQRRSIDDIERSLTNDRLEKQAQALESQGNWAQAAEVQRRRLALDPDSVWITYRLARDLVSAGERQEADALMRTMVNRQPQDAERVYASGLYLSGNDQDDLALAQIAALPRSAWTDNIRELEARLQSDRVLRQANQLRDSGNEAQAIALIRQQPASVRYDLTLADWAQQRGDSQTAIANYQRVLRQEADNGDARLGLAEVYLAEGDKPAARAQVMQLKGAETESMNMQRRVALARAGLGDTADAQRIFNQIVPQAKAQPPSMESALVLRDAARFATQSGAPQQALTHYREAMVASGITPAQPQDNDTFTRLTRNDSHDDWLKRGIRSDAADLYRQQDLNVTLEHDFWGSSGTGGYSDLKAHTTMLQMDAPLADGRMFFRTDLVNMDAGSFSTHSDGSYSPSWGTCGEIACTSGSKNQTDSGASVAVGWKNDTWSGDIGTTPMGFNVVDVVGGLSYSSDVGPVGYTVNVHRRPISSSLLSFGGQKDSSSHTGATWGGVRADGGGLSLSYDRGEAHGIWSSLGADSLTGKNVADNWRVRWMTGYYYKVINENNRRVTVGLNNMIWHYDKDLSGYTLGQGGYYSPQEYLSFAVPVTWRQRTENWSWELGGSVSWSHSRTQTQARYPLLNLIPSDYRQRASELTEEGSSSHGFGYTARALVERRVTSNWFVGAAVDIQQAKDYTPSHALLYVRYSAAGWQGDLDMPPQPLVPYADW

SEQ ID NO: 30 - protein, 1411 aa, Klebsiella pneumoniae
MSQEYTEDKEVKLTKLSSGRRLLEAMLILCSLFAIWLMAALLSFNPSDPSWSQTAWHEPIHNLGGAPGAWLADTLFFIFGVMAYTIPVIIIGGCWFAWRHQENDEYIDYFAVSLRLIGALALILTSCGLAAINADDIWYFASGGVIGSLLSTTLQPLLHSSGGTIALLCIWAAGLTLFTGWSWVSIAEKLGGGILSVLTFASNRTRRDDTWVDEGEYEDDEEEYDDEEAARPQESRRARILRSALARRKRLAEKFTNPMGRKTDAALFSGKRMDDGEEVVQYSASGAPVAADDVLFSGASAARPAEDDVLFSGASAVRPGDFDPYDPLLNGHSIAEPVSAAAAATAAPQAWAESPVGHHGAAPAYQPEASYPPQQAYQPEPAPFQQAYQPEPAPFQQAAYQPPAGQTAPQAYQPEPAPYQQPVYDPRAGQPAPQAYQPEPAPYQQPAYDPYAGQPAPQAYQPEPAPYQQPAYDPHAGQPAPQAYQPEPAPYQQPAYDPYAGQPAPQAYQPEPAPYQQPTYDPYAGQPAPQTYQQPAYDPNAGQPAPQPYQPEPAAYQPQSAPVPPPEPEPEVVQEEVKRPPLYYFEEVEEKRARERELLASWYQPIPEPESPIATKPLTPPTTASKPPVETTVVSAVAAGVHQATAASGGAAAATSSTAASAAATPLFSPASSGPRVQVKEGIGPKLPRPNRVRVPTRRELASYGIKLPSQREAEQRARQAERDPHYDDELLSDEEADAMEQDELARQFAATQQQRYGHRWEDDNATDDDEADAAAEAELARQFAATQQQRYATEQPPGANPFSPADYEFSPMKTLVNDGPSEPLFTPTPEVQPQQPAQRYQQPAAAPQQGYQPAQHQPIHHQPVPPQPQSYPTASQPVQPQQPVAPQGHQPAAPAPQESLIHPLLMRNGDSRPLQKPTTPLPSLDLLTPPPSEVEPVDTFALEQMARLVEARLADFRIKADVVNYSPGPVITRFELNLAPGVKAARISNLSRDLARSLSTVAVRVVEVIPGKPYVGLELPNKKRQTVYLREVLDNAKFRDNPSPLTVVLGKDIAGDPVVADLAKMPHLLVAGTTGSGKSVGVNAMILSMLYKAQPEDVRFIMIDPKMLELSVYEGIPHLLTEVVTDMKDAANALRWSVNEMERRYKLMSALGVRNLAGYNEKIAEAARMGRPIPDPYWKPGDSMDAVHPVLEKLPYIVVLVDEFADLMMTVGKKVEELIARLAQKARAAGIHLVLATQRPSVDVITGLIKANIPTRIAFTVSSKIDSRTILDQGGAESLLGMGDMLYSGPNSTTPVRVHGAFVRDQEVHAVVQDWKARGRPQYVDGITSDSESEGGGGGFDGGEELDPLFDQAVNFVTEKRKASISGVQRQFRIGYNRAARIIEQMEAQGIVSEQGHNGNREVLAPPPFE

SEQ ID NO: 31 - DNA, 285 bp, Klebsiella pneumoniae
atgaagaagttagctttactctccgccgtaatgacgcttggaatgtcgtcatgggcttttgctgccgacaacccgccgccgccgccggaaaaaggcgcgcagcatcagggtaaaccgccggtgaaaaacggccaacacgaaggtaagcaagcgcaatacaacagaaaacagccacaacgagacggcaaacagccgcagcacgacggtaaacagccgcagcacaacggcaagcagccgccaaaagggagcgagcacagcgggaaaccgctgccgccgaaagcgtaa

SEQ ID NO: 32 - DNA, 354 bp, Klebsiella pneumoniae
atgaaacgttacgcaaccgcactgctcttttgcactctgtcgctgaccagcctggccgctcgcgccgatattatcgatgacgcgatcggcaatattcagcaagccattaacgacgcctataaccccggcagcagtcgctccgatgacgacgacagatacgatgacgatggccggtatgatgacgggcgctatcaggggagccgtcagcagagccgtgacagtcagcgccagtatgacgagcggcaacgccagctggacgagcgccgccgccagctggatgaacgccagcgtcagctcgaccgcgatcgtcgtcagttagaaagcgaccagcgtcgtctggatgatagctactga

SEQ ID NO: 33 - DNA, 360 bp, Klebsiella pneumoniae
atgttcaggtcactgattctggcagcagtactgctggccgcagggccactggtcgctaacgctggtgaaatcaccctgctgccatcggtaaaattacaaataggcgatcgtgacaattacggtaactactgggacggtggcagctggcgcgaccgtgattactggcgtcgtcactatgaatggcgtgataaccgttggcatcgtcatgacaacggctggcacaaaggctggtacaaaggcagagataaagcctgggagcgcggctatcgtgctggctggaacgaccgcgatgaccaccgcggcggctggggtcgcggcccgggcgggcgcggtcacggtcatggacatggccatcactaa

SEQ ID NO: 34 - DNA, 363 bp, Klebsiella pneumoniae
atgaaggaaatcggcttaccgttattgctactgaccgcgctggccagtccggcttttgctgcagactgtcagccaaacggcattggcggctcgttttgcattaacgatgacggtacgactaccgacacggtgcctaacgaagtcaacggcatggatacgtactcgaataatggcggctataccagttccctgcccgatcggtcaggggcggatgaagcactggaaggttcatcgctgtcgacgcagcaaggcgtcggcagcggacagagcgacagtgcgctggcgggtcgcgactggcattcgcccgccaatctgaatgatggcgccgccacctccagtatgagcctgctggataaaccctga

SEQ ID NO: 35 - DNA, 366 bp, Klebsiella pneumoniae
atgaatatgaaaaaactgacgacccttttgctcaccgccaccttaggtcttgccagcggcgcggccctggcggcagacaccggcgcccagtccaataatggccaggccaactcttccgcggatgccggtcaggtggcgccggatgcccgtgagaacgtggcgccgaacaacgtggacaatagtcagatcaactctggctctgggggcaccacgggctcgacgatgacccaggataatatgtcgagcaatgaggtacataaaaactcgatgtgtaaagacggccgctgtccggacaccggtaaaaaactggacaacggtggcaatacgacccaagacaacagcaaaaccgacggcaccacccagtaa

SEQ ID NO: 36 - DNA, 369 bp, Klebsiella pneumoniae
atgaaacaccgcatcgctctgcttctggtcctgacttcacttagcgccagcgccctagccgcctctccctgccaggaaaaagagcaggatattcaacgagagatcagctacgccgaaaagcatcataatcaaagtcgcattgatgggctaaataccgcgctacgtcaggttcgggaaaactgtagcgacagtaaactcaaagccgatcatcagcaaaaaattgccaaacagcgggaagagatcgctgaacgtcagcgcgatctgcaggaagcccggaagaaaggcgatgcggacaaaattaacaaacgccagcataaactcaatgaagcgcaacaggagttaaaaacgctggagtctcgggattactaa

SEQ ID NO: 37 - DNA, 426 bp, Klebsiella pneumoniae
atgcgactcataacacgacacgtgagagaggatattatgaaaaaagcaatgattgcgttatcggctattctggttgcggctccggtttttgctgcgacaacacatgcaacagatgataccgtcgcggcggcgaatgccaacgccaacaccgctaaagagaagctgcatcaggcccagcacgagggcgaagagcagcagctgaaggcgaaacacgccgccgaaggcaagcaggacagcgtcggcagccaggtgagcgaaggcgcgcagaaaacctggaacaagaccaaagaaggcaccgagaaggggtgggataagaccaaagaggtcagtgaaaaaggctggaacgccaccaaatccggtgcggaaaagggctgggataaaaccaaaaccggcgccgaagagttaaaaaataaagtgactgaataa

SEQ ID NO: 38 - DNA, 456 bp, Klebsiella pneumoniae
atgaaaaagatgatttctctggcagtaattttatcctgtgtgctgagcgtcccggcctttgccgatggcccgaacgacggccatcgcccggagcagcccacggtgtggcagaacggtccggaccatgacgggcatgcaccgcagggcggacctgacgcgcatcatcagggcgaccatgaccagcgtggcccggatcgcgacggccatgacaaacgcgatctggcacgtcatgagcaggaccatttcgcctggcgcgggaacgatttccgcaaaggccacccggctccggcgccgttccgtggcgatgaatatcgcgtccgcgactggagcgaccgcggcctgccgcccccgccggaaggccatcactggtcctatatcgacggtaactatgtgctgatcgccgcggcgaccgggatcatcacctcgattctggtgagcggcgccctcggccactaa

SEQ ID NO: 39 - DNA, 507 bp, Klebsiella pneumoniae
atgaaaaaaccgacatccgccacccgtggcaaatccggccgcaagtcgcgtgaagagttaaatcaggaagctcgcgatcgcaaacggcagaagaaacatcgtggccacgcggcaggcagtcgcgcgaacggcggcgatgcggcttcagcgggtaaaaaacagcgtcaggcgcaagatccgcgcgtgggtagcaaaaaaccgatcccgctgggcgtgagcgaaagcagcgttccagctcccaagcagcataaaccaaagagcgagaaacctatgctttcaccgcaggctgagctggagttgctggagaatgatgagcgcctggacgcgctgctggaacgtctggaagagggcggcaccctgaatgctgaagagcagagctgggtggacgccaaactggatcgcattgatgagctgatgcagcagctcggcctctcttacgatgatgaagatgaagaagaggaagagcgtcaggaagatatgatgcgtctgctgaagggtggaaactaa

SEQ ID NO: 40 - DNA, 690 bp, Klebsiella pneumoniae
atggcgagtaagtttcagaaccgtttagtcgggacaatcgtgctggtggcgctgggggtgattatcctgccagggctgctggacgggcagaaaaagcattaccaggatgagtttgccgcgatcccgctggtaccgaaaccaggcgatcgcgatgaaccggatatgttgccggcggcaacccaggcgttgccttcgcaaccgccggaaggggcggcggaagaggtgcgggcgggcgatgccgccgcgccatcgttagatccatcgcgtattccggtgaacagcaacagcttcgatgacgttcaggagccggtggtggccgcgaaaccgcagcccaagccgcagccgaaaccgcagccgcaacagcaggcctcgacgccaacgccgccgccggctaagccacagcagcaacagccaccgcagcagcaggcggccctgccggcgccgaccggcaaagcctatgtggttcagctgggcgcgttgaagaacgccgataaggtgaatgagattgtcggtaaactgcgggcctcgggtttcaaagtctatacgtcgccttcgacgccggtacagggtaaaattacccgcatcctcgtcggcccggatgcgtcaaaagacaagctgaaaggccagctgggcgatctgcagcagatctccgggcttagcggggtggtgatgggcttcaccccgaactga

SEQ ID NO: 41 - DNA, 969 bp, Klebsiella pneumoniae
atggcacaacgagattatgtacgccgcagccaaccggcttcttcgcggcgcaaaaagagcacgacccgaagctcaaggaataagcaaagcagccttccggcgatttcaccggcgatggtggcgatcgcggcggctgtgctggtggcctttatcggtggcctctatttcattacgcatcataagaaagaagaagcggaagcgatgcaaaatcgccaggccgccggcaacggcttgccgcccaaaccggaagagcgctggcgctatattaaagagctggaaagccgccagcctggcgtccgcgcgccgaccgaaccgaccgccggtggcgaagtcatgaaaccggaacagctgaccgacgagcagcgccagctgctcgcccagatgcaggccgatatgcgccagcagccgacccagctgaccgaagtgccgtggaacgaacaaacgccggcgcagcgccagcagacgcttcagcgtcagcgtttagcgcagcaacagcagcaggcgcagcagcaacagtgggcgcagactcaggcgcagaccgtccaacagcagccgccgcgcgttcagcagccgaagccggttcagcagcaacagccgaagcagaccgcgtcaaaccagcagccgtaccaggatctgctgcagacgccagcgcataccaataccacgcagccgcgtacccaggccgcggcgccggtaactcgggtggaagaagcgccgaaaaccaccgccgagaagaaagacgatcgtagctggatgatccagtgcggctcttttaaaggcgccgagcaggccgaaaccgtccgcgctcagctggctttcgaagggtttgcttcgcacattaccactaacaacggctggaaccgcgtggttattggcccgttgaaaggcaaagaaagcgccaacgagatgatcacccgcctgaagatggctggacacgcgaactgcattcgtctcgccgccaggggttga

SEQ ID NO: 42 - DNA, 1131 bp, Klebsiella pneumoniae
atgagcgcgggaagcaccaaatttaccgtcagccgtattgcggctctttcactggtttcactctggctggccgggtgtaccaacaccaataatccgcctgcgccggttagctctgccggcggcgccgcctcttccagcaccaactccggcatgctgattacgccgccaccctccggcgtcaagtccgctcctcaggcgcagccgattcagccgatgcagacccagaccattcagccggcgccggtggcgcaggagccggtacagacggtaaatggccggatcgtttacaaccgcaaatatggcgatattccgaaaggtagctataccggcggcagtacctatacggtaaaacgcggcgacacgctattctatatcgcctgggtcaccggcaacgatttccgcgacctggcgcaacgtaacaatatcccggccccgtacgcgctgaacgtggggcaggtactgcaggtcggtaacgcctcaggccagccgatcaccggcgaaaacgccgtttctcaggccagcgcaagagcgagcggcggtgcgacgaccagcacaacttctgcacaaaaatcgaccgcggtggttgcttcacaaccgactattacgtattctgaatcttcaggtgaacagagtgctaccaagatgttgcctaataataaaccagcgaccacaaccacaacggttgtcgcgccggtgacggcaccaacaacggtgagcacaacccagccgactgcaagcagtacgtcaaccagttcgccgatctcagcatggcgctggccgactgatggcaaggttatcgagaactttagcggcgcggaaggcggcaataaaggcatcgatattgcaggcagtaagggacaggctattgtcgcgaccgccgatgggcgcgtcgtctatgccggtaacgcactgcgcggctacggtaatcttattatcatcaaacacaacgatgattacctgagtgcctacgctcataacgataccatgctggttcgggagcaacaggaagtcaaagcggggcagaaaatcgctaccatgggtagcaccggaaccagctcaacaagattacattttgaaattcgttacaaggggaaatccgtcaacccgctgcagtacttaccgcagcgataa

SEQ ID NO: 43 - DNA, 1149 bp, Klebsiella pneumoniae
atgcgtaagcaatggctggggatctgcatagcagcggggctgctggcggcatgttcgagtgatgacgtgcaacaaaaaacggtcagtactccacagccggccgtctgtaatggcccgacggttgagatcagcggcgccgatccgcagtatgaaacgccgaacgccacggcgaatcaggattatgagcgcgacggtaaaagctacaaaatcgttcaggatccggccaactttactcaggccggtttcgcggcgatctatgacgcagaacccaacagcaacctgaccgccagcggcgaagccttcgatccgactcagttgaccgcagcgcacccgacgctgccgatcccgagctacgcgcggatcactaaccttgccaacggacggatgatcgtcgtgcggattaacgatcgcggtccctatggcaacgatcgggtcatctcgctttcccgcgcatccgctgaccgcctgaacacctccaacaacaccaaagtgcgcatcgaccccatcatcgtcgcgcctgacggttcgctttccggcccggggatggcctgtaccaccgtcgccaaacagacttacgccctgcccgcccgtccgaatctggacggtggggacgccgctggcatgagccagcccgcgcccactgacgttcgcccgatcagcaacagcacgctgacgccggcagacagcgtgggcgcgccggtgaacagcggcggtttcctcggcgcgccgacgcccctgaacaacggcgtgctggagagtagcgaaccagcggcagccgccgcgacggctcctgccgccggcgccacgccaacagcgccagtgaccgcgcctggctccattcagggtaatgtggtgcccgctgcggccaccgccgcagccgctggcgccgtggcggcctcgtcctccgcgacctccagcgccagcggtaattttgttgtccaggtgggcgcagtaagcgaccagacgcgggcgcagcagtatcagcagcgcctgagccagcagttttctgtgccaggccgggtcatgcaaaacggcgcggtctggcgtattcagctgggtccctttgctgataaagcacaggccagcgccgtgcagcagcgcctgcaaagcgaagcgcagctgcagtcctttattactcgcgccaactaa

SEQ ID NO: 44 - DNA, 1287 bp, Klebsiella pneumoniae
atggatgatttcaaaccagaagacgatatgaaagccgatcgcaacgatcgtcgtgctggtcgttcccgtcagtcttccgagcgtgatgccgatccgcagatcaattttgacgatgttgatcttgatgccgatgaaggccgtccgacgcgcgctggtaaggcccgtcgcgagcgtgaagaggaagagttcgaagaagaactggatgcgcaagacgaggagatgctcgaagagcagcctgtagagcgtcgtccgcgcaagcgtaaaaaagcgccggccaaaccggcctcccgccagtacatcatgatgggtgtggggattctggtgctgctgctgttgatcgtgggtatcggttccgcactgaaatcgccatcatcttccagccagcagaccgcttccggcgagaagagcattaatctgtctgacgaccagtccgccagcatgcctgctgccggccaggaccagactgccgccgctaacagcacctcacagcaggacgtaacggtaccgcctattgccgcgaacccgacgcagggccaggcagcggttgcgccgcagggccagcagcgtatcgaagttcagggcgatctgaacaatgccttgacccagcagcagggccaactggacggcgccgtggctaactcgacgctgccgactgaaccggctaccgtcgcgccaatccggaatggcgccaatggcaccgcggcgccgcgccaggcgaccgagcgtcagacagcagcgaccccgcgtccggctgaacgtaagcataccgttatcgaagcgaagccgcagtcgaagccacaggccgtggcgaaaacgccggtagaatcgaagccggtccagccgaagcatgttgaaagcacggcgaccaccgctccggcgaaaacgtccgtcagcgaaagcaaaccggtggccaccgctcagagcaaaccgaccacgacgaccgcagcgccagcggcaacggcagctgcggcagcgccggcagcgaagaccgggaagacggcaggtgacgtcagctcaatgaaaactgcgccgtcgggtcactatactctgcagctcagcagctcctctaactacgacaacctcaacaactgggcgaagaaagagaagctggataaatatgttgtctatgaaacgtcgcgtaacggccaaccatggtacgtgctggtgagcggtatctatgcatcgaaagatgaagcgaaacgtgctgtcacctcgctgccggcggacgtgcaggcgaaaaatccatgggcaaaaccgctgcatcaggttcaggctgacctgaaataa

SEQ ID NO: 45 - DNA, 1326 bp, Klebsiella pneumoniae
atgtcaaaggcaaccgaacaaaacgacaagcttaaacgagcgatcatcatttcagtcgcgctgcacatcattctgatcgcgctgctgatctggagttcgtttgacgagcatctggatgcctctgccggcggcggcggcggatcgtcgattgatgccgtcatggtcgatccgggggcggtggtaaataactataaccgtcagcaacagcagcaggccagcgcacgtcgcgccgctgaacagcgtgaaaaacaggcgcagcagcaggcggaagagttacgtgagaaacaggcggcggaacaggaacggctgaaacagctcgaacaggagcggctgcaggcgcaggaagcggcgaaagaagcgaaggagcagcagaagcaggctgaagaagcggctgccaaggccgccgcggcggcaaaagccaaagcggacgcacaggcaaaagaagcgcaggaagccgctgccaaagcggccgccgaggcgaaagcgaaggcggatgcccaggcgaaagcggcagaacaggcggcggccaaggcggctgctgacgcgaaaaagcaggccgaagccgctgcagcgaaagccgctgccgaggcgaagaaacaggcggaagctgaagcggcgaaagctgcggccgaggcgcagaagaaagcggaagcggcggctgcgaagaaagcgcaacaggaagcggagaaaaaagcccagcaggaagcggctaagcaggcggcagctgaaaaagcggctgccgaaaaagccgctgagaaagccgccgcgcaaaaagcggccgctgagaaggccgccgccgagaaagccgcagccgctgaaaaagcggcggcagcgaaagcggctgcagcagagaaggctgcagctgataaagcggccaaagcggcagcagcaaaagccgcggcggcgaagaaagcggcggctgcgaaagaagcggacggcgttgacaacctgctcggcgatctgagttctggtaagaatgcgcctaaaacaggcggtggggccaaaggaaacaatgcctccgctgccgggagtggtaatactaaaaacagtgcctcaggggctgatatcaacaactatgccggacagataaaatcggcgattgaaagtaagttttatgacgcatcgtcctatgcgggcaaaacatgtaccttgcgtatcaaacttgctcctgacggcctgttgttaaatatacagtccgaaggtggtgatcctgctctgtgccaggccgctcttgccgcagcccgacaggctaagtttccgaaaccacctagccaggcagtatatgaagtcttcaaaaatgcgccactggacttcaaacctcagtga

SEQ ID NO: 46 - DNA, 1455 bp, Klebsiella pneumoniae
atgttttttttaagtattttttacatggagatgacaaaagtgaaattaagcgctctgtttattgccctgattcctctactgggctcgccggttattcatgcagaaactactgctgcgccggttctggaaaatcgcgctgcgcagggagatatcaccactcctggcggcgcgcgtcgtttaacaggcgatcaaaccgaagcgctgcgcgcctcgttaatcaataagccagctaaaaacgttattttgctgattggcgatggcatgggtgattcggaaattaccgctgcgcgaaactatgccgagggggcgggcggtttctttaaaggaattgatgctctgccgttaaccgggcagtacacgcattattcgctggataaaaaaaccgggaaaccggactacgtgaccgactcggcggcctccgccaccgcctggaccaccggcgtgaagacttataacggcgcgctgggcgtcgatattcatgagaatgcgcatcagaccatcctcgagctggcgaaagcggcggggctggccaccggcaacgtttccaccgccgagctgcaggacgccacccccgcggcgttggtagcgcatgtgacatcgcgtaaatgctacggcccgacggtcaccagcgaaaaatgccccagcaatgcgctggaaaaagggggcaaaggctccattaccgaacagctgctgaacgcccgaccggatgtcaccttgggcggcggcgcgaagacctttaccgaaacggcgacggcgggcgagtggcagggcaaaaccctgcgcgagcaggcgcaagcgcgcggctaccagattgtgaccgacgcggcttctcttgccgccgcgacggaagccagtcaggataaaccgctgctgggactctttgccgatggcaatatgccggtacgctgggaagggccgaaggcgtcttatcacggtaatatcgataagccgccggtgacctgtacgccaaacccgaagcgtgacgcctcggtgccgacgctggcgcagatgacggagaaagcgattgacctgctcagtcgcaacgagaaaggtttcttcctgcaagtcgaaggcgcttccatcgataagcaggaccatgcggcgaatccgtgcggccagatcggcgaaacggttgatcttgacgaagcggtgcagaaggcgctggaattcgcgcgaaaagacggtaataccctggtgatcgtcaccgccgaccatgcgcatgccagccagatcatcccggcggatagcaaagccccggggctgacccaggctctgaacacgcacgatggcgcggtgatggtgatgagctacggcaactctgaggaagagtcgatggagcacaccggcacccaactgcgcattgcggcctacggtccgcatgcggctaacgtcgtaggcctgaccgatcagaccgacctgttcacgaccatgaaagctgccctgagtctcaaataa

SEQ ID NO: 47 - DNA, 1608 bp, Klebsiella pneumoniae
atgtcactgccgttcaaaccccatattatcgccctgctctgtagcgctggcttactcgcggcggcaggaacactctatgtgcaaagccgaaccccagcgacgatcgctgaaccgcctgcgcagcaagcgccagcgcccgcagcgtcgacgacacagccggtggccgccacttacacccaggcgcaaattgatcagtgggtcgcccctatcgcgctctacccggacagcctgctgtcgcaggtgttgatggcctccacttatcccgacaacgtcctgcaggcggtccagtggtcccaggataaccccgcgatgaaaggggatgcggccgtgcaggcggttgccagccagccgtgggaccctagcgtcaaatctcttgtcgctttccctgccctgctggcgatgatgggcgagaatccgccctgggtggaaaatcttggcaatgcgtttttggcccagccgcatgatgtgatggattcagtgcagcgcctgcgcgccattgcccaacaaaccgggacgctgaaatccacaccgcagcagaaagtgattgtcacccctgccgcaccggtttcagccagcagcagcacggcagcaaccgcaaccgcccacacagcggcgcctgcgcccacgcaggtcattaaaatagagccgaccaatccacaggtggtctatgttcccagctataacccctccaccgtctatggtacctggccgaacagcgcctatccgccggtctatctgccgccccctcccggggagcagtttaccgatagcttcgtcaaaggcttcgggtacagcctcggcgtggccaccacctgggcgctgttcagcagtatcgactgggatgatgatgaccatcaccatcacgatgacgactaccaccacggcgattactcgcataatggcgataacatcaatattaatgtaaataatttcaatcatataacaggagaaaacctgccgggaaaccacgttaactggcagcacaatcctgcctatcgcggacacacaccgtatcccgataatacggtagctcagcgcttccatcagaccaacgtttccggcggactgagcgcgacccaacatgcgccagtcgatcgcgaagcgcagcgccaggcagcgatgacccagctgcagcataacgtaccgacggccacagcgggcaacctggcggcaaacaacgcctcacgcgacgcccagcgtcaggcggcctcggcgcagctgaagcaagccacccaacgcagtaattaccgcggttacgacagtacgccgacccaacagcagcgtcgcgaggcggcaaaaacgcagctgaaaaaccccacgccgcagcaacagcagcgtcgagaagccgccaggagccacgagcagaaccgcacacctcagcagcagcagcgccggcagcagttccagtccgccacgccagcccagcgtcagcagacgctcagccatctgcgcgccaacgcccttagcggcaacgaaagccgcgccccctcctggcaagcgcagcaggaacgaggactgcagagccgccagttttccggcgtaaaccgcgagttacgcgatggcaccagagaacgtctttccgaacaccatgaactgcgtcgccgctaa

SEQ ID NO: 48 - DNA, 1794 bp, Klebsiella pneumoniae
atgtttaagtttaaggcttcttatgtcgcactggcggcagtattaacctcgtcggtagtttatgccgaccccacaagctatacgcactcttccggcgccacggttatcgatattgaaaagccgaacgccgccggtgtctcccataacctgtaccgcgacttcaacgtcggcgccaatggcaccatcctcaataacagcggcgatgatgtcagccacagcacatttggcaatatcgcccgcaacaataatctgaccgccggcagcgcttcggtgattttgaacgaggtgacctccaaaaacgccagtagcctgaagggctttatcgaagtcaacggtcagaaagcggatgtggtaatcgccaacccgaacggcatcacctgttccggctgtagctttgttaataccaacaaggctatcctgaccaccggcaaggttaatatgaccgacgatggcgctatcggcagctataccgtaacgggcggcaccctcaccatcggcgaaaatggcatgaacgccgccaacggctatgcggttctgctcgccgacgcgatcaatatcaacggtaaagtgcaggccaacaacgccctggtcagcgcgggcaacttcaccatggataacagctctggctcggtgacctccgctggtaaaaaggccaccctgatccagatgacggttaacccgcagtacagcatcgacgtcagcagccttggcggcattgaggccaacagcatcagcatggtcggcaataacatcggctttggcgtacgtaataaaggctctatcgtcgcgaatagttcgctgcagctcaccagcaacggtaatctgctgaacaaaggcacgatcaaaagcaacggtctgctgagtcaggtcgccaccgcctcgggcatcaccaatgacggtagcatcgccggcgcctattatttaatgctctccagtggcgattatatcgttaacaccggttctctctccggcggccagctgattgccaccgctaacggcaacatcaccaacggcgactcaggcacgatgaccggcaccagtggattaagcctgaccagcggcgggaaaatccgcaacgaagaaaaagcctccctgctgtcaaataaccagattgccgccacggcaatcggtgatttcctcaatgaaggcaaaatcagcgccaaacacaccagcctgacgtttgtcggcgacagctttaaaaacactggcaatattaactctactggccaaaccaccattcagtcgcttaaacaggacggcagcgccaatacgggcgagatctataacctcggcaatatcaccggcgaaaatatcaatctgcagaccaatggcacgctggcgcaaagcagcagtggtcgtattgaggcaaccaacgccattaccgcccacagctactggctgaaccaaaatggttatatgaatgccgccgatatcaccaccgatcacggcgtagtgaataattatggcaatattactgccaaaaatatttcaatcacgacctactcagatatcaccaacgaagggcagatcagcagcaccggcgacctgaccttaaataccaaaaataaaggcgcgatctacaattattcaaccctcagcgcgggcggcaacatgacgttaaccgccaccaaagtggtcaatggtggtaaaagttgcggcatactgggcctggcgaaatgcggcgtcgggacgttaactgctgacaagctggtactgaactcatcgcagaaatatgttagcgacatgggtggaaaacagtatttcaagagcaccgaagtcaacacggtgaaataa

SEQ ID NO: 49 - DNA, 1875 bp, Klebsiella pneumoniae
atgatggacaacctacgcacggccgccaacagcgtcgtgctcaagattattttcggtatcattatcgtctcgttcattttgaccggggtgagtggttacctgattggcggtggcaaaaactatgccgcaaaagtgaatggccaggagattggccgtgggcagtttgaaaacgccgtcgccagcgaacgtaaccgtatgcagcagcagcttggcgatcaattctccgagctggcggcgaacgaaaactacatgaaaaccatgcgccagcaggtgctgaaccgcctgatcgatgagtcgcttctggatcagtatgcccgcgagctgggcctcagcatcagcgatgagcaggtgaagcaggcgatcttccagacccaggcgttccagacgaacggtaagttcgacaaccagcgtttcagtggtattgtcgcccagatggggatgaccaccgatcagtacgcccaggcgctgcgtaaccagctgaccacgcagcagctgattaacgccattgcgggtaccgacttcatgctgccgggcgagtccgatcagctggcggcgctggtatctcaacagcgggtggtccgcgaagcgaccatcaacgtaaatgccctggcggcaaaacagaccgccagcgatgaggaaatcaacgccttctggcagcagaatcaggcccgttttatggcgccggagcagttccgcgtcagctacatcaaaatggatgccgccagcatgcaggagagcgcctctgacgaagagattcagtcatggtacgaccagcacaaggatcagttcactcagccgcagcgcaaccgctacagcgtgattcagaccaaaactgaagccgatgcgaaagcggtactggccgagctgcaaaaaggagcggacttcgccacgctggcgaaagaaaaatcgaccgatattatctctgcccgcaacggtggcgatatggggtggatggaagatgcctctaccgtgcctgagctgaaagatgccgggctgaaagagaaaggccagctgtctggcgtgatcaaatcctcggttggcttcctggtagctcgtctggacgacgtccagccggcgcaggtgaagccgctggctgacgtgcgtaatgacattgcggcgaaagtgaagcaggaaaaagcgttggatgcttactacgcgctgcagcagaaggtgagcgatgcggccagcaacgataatgaatcgctggcgagcgcagcgcaggtcgccgggctgaaggtcgtagaaaccggctggtttggccgcgataacctgccggaggagctgaactttaaaccggtcgctgacgctattttcaacggcggtctggtgggtgagaacggcgcgccgggcagcaactccgatatcattaccgttgacggcgatcgcgcttttgttctgcgcattagcgaacacaaagccgaggcggtgaagccgctggccgaagtgaaggcacaggttagcgatatcgttaagcacaataaagcggaacagcaggcgaaactggaggccgacaagctgctggcggcgctgaaagacggcaaaggcgatgaagcgatgaaggcggctggcctgagctttggcgcgccgcagacgctttctcgtaccggccaggatccgctgagccagctggcatttaccctgccgctgccgcagcagggtaaaccggtctacggcgtgggcagcaatatgcaaggcgatgtggtgctggtagcgctggatgaggtgaaagccggcagcatgccggaagagcagaagaaggccatggttcaggggatcacccagaacaatgcccaaatcgctttcgaagcgctgatgagcaacctgcgcaaggcggcgaaaattaagctcggcgacagcatcgaccagcagcagtaa

SEQ ID NO: 50 - DNA, 1974 bp, Klebsiella pneumoniae
atgttcaggttaaacccttttatccgggcgggattgtctgcgtccgtcgtatcgttggcgtttccggctctggccgatgtgaatgaagaaacgctggtggtgaccgcctcggccactgaacagaatgtcaaagacgcgccggcgagcatcagcgtcatcacccaacaggatttacaacgcaagcctgttcagaacctgaaagacgtgctgcgcgatgtgcctggggtccagctcaccaacgaaggggataaccgcaagggcgttagcatccgcggtctgagcagcagctataccctgatcctggtcgacggcaagcgcgttaactcgcggaacgccgtcttccgccacaatgacttcgaccttaactggatcccggtggatgctattgagcgtatcgaagtggtgcgcggcccgatgtcctccctctacggctccgatgcgctcggtggggtggtcaacattattaccaaaaaaatcggccagaaatggaccgggacgctgagtgctgataccactattcaggagcaccgcgatcgcggggatacctggaacggccagttcttcaccagcggcccgctgatcgacggcgtacttggaatgaaggcctacggcagcctggcaaaacgcgccaaggacgatccgcagtcatccagtaatgccaccggcgagacgccgcgcatcgagggcttcaccagccgcgatggcaatgttgaattcgcctggacgccgaacgaaaaccacgattttaccgcaggctacggctttgaccgtcaggatcgcgattccgattcccttgaccgcaaccgccttgagcgggagaactactctctgagccataacggccgctgggatatcggcaatagcgagctcaagttctacggcgaaaaggtggataacaaaaatccagggcagagcgggactattacctcggaaagcaatgccatcgacggcaagtatgtcctgccgctgggcatgattaaccagctggtgaccttcggcggcgaatggcgccacgacaaacttaaagatccggtcaacctgagcagcggcggccagtcaacgtcggccagccagtacgccctgtttatcgaagacgaatggcgcatcatcgagccgctggcgctgaccaccggcattcgtatggacgaccatcagacctatggcgatcactggagcccgcgcgcctatctggtgtataacgccaccgataccgtcaccgtcaaaggcggctgggcgacggcgtttaaagccccgtcgctgctgcagcttaaccccgactggaccaccaactcctgccgcggctcgtgcagcatcgtcggtaacccggatctgaaaccggaaaccagcgaaagcttcgagctcggtctctactaccgcggggaagagggctggcttgaaaatgtcgaaggcagcatcaccaccttccagaataatgtcgacgacatgatcgacgttctgcgcacctccagcgccagcgaagcgccgggctacccgaactttgtcggctggaaaactgtcaacggcaagcgcgtgccgatcttccgctatttcaacgtcaacaaagcccgcatcaaaggggtggagacggaggtgaagatcccgtttggcgatgagtggaagctgacggtgaactacacctacaacgatggtcgcgatctgagcaatggcggcgacaaaccgctgcagacgctgccgttccataccgccaacggcacgctcgactggaaaccgctggacgactggtccttctacgtgacggccaactataccggccagcagcgcgcggtgagcgccaccggcaaaacgccgggcggctacaccctgtttgacgttggcgcggcatggcaggtgaccaaaaacgtgaaactgcgctccggggtgcagaacgtgggtgataaagatctgagccgggacgactacagctataccgaagaaggccgtcgctactttatggcggtggattatcgcttctga

SEQ ID NO: 51 - DNA, 2028 bp, Klebsiella pneumoniae
atgaacagagccgccacgctgaccctcaacgcgcccctgctgatgctcgtcgctgcgctggcgctttcaacccctttcaccgccggcgccgcgccggcctttcttgattacgcccaacagcaaacccagcaatctcaggcgcaagaaaaaaacgatgccgcaagcgcaaaacaaacacaagaaagccgccagagcgcagataataaaaaaaccggtaccagcacctcacaattacaaaaaagaatcaccagccagcaggcggcgattgcacaaaaagataagcttatacagcaattaaaaaaacagcttgccgctacgccgcaaacggatactgccggagcgaatgagcaagcggcgttgaataagagaattaatgaattacaggtcgccttaagcgccgctactgcagaaaaagaggcattaataaaaaaagcaggcgttgtgcagaataataatctacagcaaagccaggccgcggcgcgtcagcagatccagcaattaacgacgcagattcagcaagccgaagctgaaaataaacgcctcagcgccagctttaccacgcttaataaagataaacacgcgctaatgacccaactggccgcaacggaaaaagagaaacaggccgctcttgagcaggtcaaagcgcttaacgctgacaaacagccgctgacgacccggctggccgccgcggaaaaagagaaacaggccgtcctcgagcaggttaaggcccttaacgccgataaacagtcgctgactattcgcctcgccgctgcggagaaagcgcagcaggccgctgttgaccaggctaaagcgcttaacgctgacaaacagccgctggctacccgactggccgccgcggaaaaagagaaacaggccgtcctcgagcaggttaaggcccttagcgccgataagcagtcgctgactattcgcctcgccgctgcggagaaggcgcagcaggccgctcttgaccaggctaaagcgcttaacgctgacaaacagccgctggcgacccggctggccgccgcggaaaaagagaaacaggccgtcctcgagcaggttaaagcccttaacgccgataagcagtcgctgactattcgcctcgccgctgcggaaaagacgcagcaggctgccctcgatcaggtcaaagcccttaacgccgataaacaatcgctgtccacccggctggccgccgcggataaagcgccgcatggccccgctaacgacgccgctgcgccaaaaaatgagccaccagagatggcggccatagtggcagcctatcgcctgcaggcggataaagacaacgcccagctacggatgaaagaagatgaaatcgaactgctgagaacgcagctttctgtacagtccaaaacgcgcagcggcgagagcgccgccgccaaactcagcgcatcgggagaacagcaggcttatgcgatcggcgcctcgatgggaagcgaggcgctcaacgtccttaccacccgtcgtactcagggagttaccgtcgacgcaggcctggtgctgcagggcatcgaagatgcctttcgcggccagcttcgtctcggagagcaggaacgtaacaaggcgctgtttgatgtgtcgcagcaggtttttcagaacctgaataaaatagagcagaaaaacatcagtgccggcaagaaatatcagcaggcgtttgcgcgcaaaaaagatgtggtctttaaagagggcgtctacagccgcgtcgattacctgggtaaaggaaaaataagcggtaatgacctggttaccgtggtgatcaaagagatgctgacggacgggacggtgatcaacgatatggaagcgaaagatcaggcgcttacgcaaaagctggatgcctatcccccggtgtttcgcgaaccgctgaagcgtctacagaaccacggctccgtgacgctcgtcgtcccgcctgaaaaggcctatggcagtaaaggattaccgccaaaaatcccgccaggcgccaccatggtttattccgtgcggatagtagatagccaacccgagccggcaaaatag

SEQ ID NO: 52 - DNA, 2106 bp, Klebsiella pneumoniae
atgaaaatcctgtccgtgcgtcacgccgccctcccggccctgctcttgccgctcattgcggcagcccaggccgctgatgaacaaaccatggtggtgaccgccgcgccaaccacggtttctgaactggatacccccgccgccgtcagcgtggtgaatggggatgagatgcgccaggccgcgccgcgcgtcaatctctctgaatcgctgggcgccgtgccgggcctgcaggtgcagaaccggcaaaactatgcccaggatctgcagctgtcgattcgcggctttggctcgcgctcaacctatggcgtgcgcggactgcgcatctatgtggatggcattccggccaccatgcccgacggccaggggcagacctcaaatattgatatcggcagcgttgacaccattgaggtgctgcgcggccccttctctgccctgtacggtaactcgtccggcggggtgatcaacgtcaccagccagaccggcacccagccgcccaccgtggaagccagcagctactatggcagcttcggcacctggcactacgggatgaaagccactggcgccgttggcgacggcagccacgcaggcgatgtggattacacggtctcaaccaatcgcttcaccacccatggctatcgcgatcacagcggcgcgcgcaaaaatctggcgaacgcccggctgggggtgcgcatcaacgacgtcagtaagctgactctgctgctgaatagcgtggatatcaaagccaatgacgccggtggcctgaccgccgatgaatggcgcgataacccgcgccagtcgccgcgcggcgaccagtataatacccgcaagaatacccgacagacccaggccggcctgcgctatgagcgccagctcagtgcccaggacgatctcagcgttatgatgtacgctggagaacgtgaaaccactcagttccagtcgatcccgcgcgcgccgcagctgaagccgagccatgccggcggggtgatcgaccttacccgtcactaccaggggatcgatacccggctgacccatcgcggagagctgctggtgcccgtcacgctcaccgccggtctcgactacgaaaacatgagcgagcggcgcaaagggtatgaaaactttgtgatggtcaacggcgcgccgcagtatggcgaacagggcgcgctgcgccgtaacgaacgcaacctgatgtggaacgtcgacccctacctgcagacccagtggcagctcactgacaaactctcgctcgatgccggggttcgctacagctcggtatggttcgactcgaacgactactacatcaccccaggcaatggcgatgacagcggtgatgccagctatcacaaatggctgcccgcgggctcgctgaaatatgccctgaccgacgcgtggaacgtctatctttccgccggccgcggcttcgagacgccaaccattaacgaactctcctaccgctccgataaccagagcggcctcaacttcggcctgaaaccctccaccaacgacacggtggagatcggcagcaagacgcggatcggcaatgggctgttcaccgccgccctgttccagaccaataccgataatgagattgtggtcgacagcagcagcggcgggcgcaccagttataaaaacgccggcaagacccgccgtcaggggatggagctggggctggatcagcagtttggcgagagctggcgtctgaaggcggcctggacctggctggacgcgacctatcgcactaacgtctgcgacgacgccagctgcaatggcaatcgcattccggggatcgcgcgcaatatgggctacgcctcctttggctatcagccggagcaaggttggtacgccgggagcgatattcgctatatgagcgatatcatggccaatgacgaaaacaccgccaaagcgccctcctggacggtggttggcctgacgactggctataaatggagctacggcaggatggatatggatctgttcggtcgcatcgacaacctgttcgaccgggagtacgtcgggtctgtcatcgttaacgagtctaacggacgttactacgagcctgccccgggacgtaactacggcatcggcctgaacctcgcctggcgcttcgaataa

SEQ ID NO: 53 - DNA, 2259 bp, Klebsiella pneumoniae
atgaaatacacgtctcacttcccgctggggatcgtcattcctctgctcgcctgtagcgtgccgctgcaggcggcagagaacatgaccgaacaatcgacgcctgacgagagcgccgccactgccgaaaatcacgaggagacgatggtcataaccgccgccaggcagaacctgcaggcgccgggcgtgtcgaccatcaccgcagaagagatccgcaaacatccccccgcccgcgatgtgtcggagttaattcgtacgcagcccggggtaaacctgaccggcaactccaccagcgggcagcgcggcaacaaccggcaaattgatatccgtggcatggggcccgagaatacgctggtgctggtcgatggtaaaccggtgaccagccgtaactcggtgcggtatggctggcgcggcgatcgtgactcccgcggcgataccagttgggtgccagcggagatgatcgatcatatcgatgtgatccgcggcccggcggcggcgcgctatggtaatggcgcgatgggcggggtcgtcaacatcgtgaccaaaccgaccacgcgagaatggcacgggtcgtggaatacctatatgaatgctccgcagcaccgtaaagaaggggcgacgaaacgtactaactttagcctcaatggtccgctgtcggacagtgtcagcttcaatctctggggtaatctgagtaaaacccaggccgatgcacaggatattaacgccgggcatgaagcggaacgtaccggttcctacgccggttcttatcccgccggacgtgaaggggtggtgaacaaagatattcacagtaagctgcgctgggagtttgccccgatgcaggccctggagtttgaggccggttacagccgccagggtaatctctatgccggcgacacacaaaacaccaataccagtacgctggtgaagagtatgtacgggaaagagaccaaccgtctctaccggcaaacttacggcgtaacatggaccggcggctgggataatggcgtgaccagcaacagctatgcccagtacgaacacacccgtaactcgcgaatggatgaagggctggcgggcggtacggaagggatcttctccagtagcgagttttcagatatcgatctggccgatgtcctgctacatagtgaagtgaatattccgtttacgctgggggtcgatcagaatctgacgctgggggcagaatggaatcagcagcggatgaaagatggcgtatcgacaacccaggcgctctcttatggcactatcgatggcgtatcggctaccggtcgtagcccgtactccagtgccgagatcttctcgctgtttaccgaagataatatggcgctaacggacagcaccatgctgacacccgctctgcgcttcgatcaccacagcatcgtcggcaataactggagcccctcactgaacctgtctcaggagctgacggacgactggacgctgaagctgggcattgcccgtgcttacaaggcgcctaacctctaccagttgaacccgaactatattctctacagcaacggtcaaggctgttacgccagtagttccgcctgctatctgatggggaatagcgatctgaaagcggagaccagcgttaataaagagattggtcttgagtacaagcatgatggctatcaggcggggatcacctggttccgtaacgactatcacaataagattgagtcagggtatgcggcggtgggtaccgccagcaacggcaccaccaatatctatcagtgggaaaacgtaccaaaggcgttagtggaaggcctggaaggaacgctgaatctgccggtgggggaggcggttaactggagcaataacctgacctggatgctgcagagcaagaataagacgaccggcgaccggctgtcagtgatcccgcagtttaccctgaactcgactttgagctggcaggttcgtgaagatctctccctgcagagcacctttacctggtatggccgacagaaaccaaaacgcttcaattataagggcgaggcggtcagcggcagcgaactaaacgaagtcagcccatacagcattgtcggcctcagtgcgacctgggatgtgaacaaaaatctgagcttcaccagcgggatagataacctgtttgatattcgccactaccgggcagggaatgcgcaaacgaccggcaacgcgacgacgggagcttatctgtatggcgcgggtgccgagacctataacgaatcggggcggaccttctttatgagcgttaatactcatttctga

SEQ ID NO: 54 - DNA, 2286 bp, Klebsiella pneumoniae
atggaaaaaaacgcttctctgcctttcggcagtttcaactcattggcattgtttacaggtctgtgtctgggagcctcgccggcagcaggcatcgcagcggaaaattcggtcaaaaatagtgaagagacgctggtagtggaagccgctccgccttcactctactcccccggcgcttccgccgatcccaagttcaataaaccgctggtcgataccacccgcaccatcaccgtgatcccggaacaggtgattaaagatcagggcgtcaccaacctgactgacgccctcaaaaacgttcccggcgtcggggcgttttatgccggggagaatggcagctcaaccaccggggatgccatctttatgcgcggcgtggatacctctaacagcatctatgtggacggcattcgcgacatcggtagcgtgacgcgcgataccttcaatacccagcaggtggaagtcatcaaagggcccgccggcacggactatggccgcagcgcgccctccggctcgatcaatatgatcagcaagcagccgcgccttgactccgggatcgacggctcggccagcatcggcagcgcctggtcgcgccggggcactctcgacctgaaccaggcgtttagcgacaacgctgcgttccgtctgaacctgatgggggaaaaaacgcatgacgctggtcgggaccgcattgaaaacgaacgctatggcatcgcaccgtcgctggccttcggccttgataccccaactcgtctgtatctgaactatctgcacgtccggcagaacaacaccccggatggcgggatccctaccgtcggcctgccgggctattcggcgccttcgccgaagtatgccgcactcaactccgccgggaaggtcgataccagcaatttctatggcaccgactccgattacgataaatctactaccgacagcggtaccctgcgcttcgaacacgatctgacggagaataccaccgtgcgcaataccacccgctggtcgcgagtgaaacaggagtatcttttgaccgcggtgatgggcggcgcgaacaatatcaccgcccccgatatcaatgacgtcaacacctggagctggtcgcgtctggttaataccaaagatgtcagcaaccgtattctgaccaaccagaccaatatcacctcgactttcaatactggctcgataggccatgacgtcagcgccggcgtggagtttacccgggaaaaccagaccaactatggcgttaacgccaggaccgcgccggcggtgaatctctaccatccggtgagcaacctgtcgattggcgggctggacagaaacggggcgaacgccaacggccagaccgataccttcgggatttatgcctttgatacgctgacgctgaccgagcggattgagatcaacggcgggctgcgtctcgacaattaccataccaaatatgacagcgccaccgcctgcggcggcagcggacgcggggctatcgcctgcccgcccggacagtcgaccggcagcccggtcaccactgtcgataccgctaaatccggcaatctggttaactggaaagccggggcgctgtaccgcttaaccgagcagggcaatgtctacgtcaactacgccatctcacagcagccgccgggaggcagcagcttcgccctggccgccagcggcagcggcaacagcgctaaccggaccgactttaagccacagaaggcgaaatccagcgagctgggcaccaagtggcaaatcttcgacaaccgtctgctgctcagcgcggcgttattccgcaccgatattgaaaacgaagtggccgccaacgatgacggaacctggtcgcagtacggcaaaaagcgcgtggaggggtatgaactctccgcgaccggaaacctgaccccggactggacgattatcgccggctacactcagcagcatgcgacagtgacggagggacagaacgttgcacaggatggatcttccgccctggcctacaccccgaaacatgcctttacgctgtggacgcagtatcaggccaccagcgatctgtccgtcggcggcggtgtgcgctatgtcggaagcctgcgccggggcagcgatggtgcagtcggtaccccggatcacaccgagggctactgggttgccgacgccaaactgggctatcgggtcaacagcaacctcgatctgcagctcaatatgtataacctgtttgataccgattacgtggcctccatcaacaagagcggctatcgctatcatccgggcgaaccccggacctttatgctgacggcgaacgtccatttctga

SEQ ID NO: 55 - DNA, 2373 bp, Klebsiella pneumoniae
atggcgactatgtacaaatcgactccgtcagcagcatggtgtaaaaaacgcctgctggtgacctctttgtttgcagcaatttatcagacttctgccatcgcagcagatacttccgccgttagcggcgaggcggtggatgacacctcggaacaaatgaccgtcaccgcccccgcgccggtgcagaaagccggtagcgaacacagcatcagcgcccgggagctggagaataaaggcgctaacgatttcggctcaatcatgcgctatgagccgctcatcagcgccaccggggccagcggcggctccggcaacggcaaaagcggcttcgaccgcggaggttacaccggctacaacattcgcggtatggagagcaaccgcgtaggcatcgacgtggacggtatcgcgcaacccaacgccaccggccgcggctacgtcggccgcgccgggctcaacaccttcggcatcggccgcgattatatcgacccgtatatgtacggcagcgttgatatccagtccggcgccacctcgacggaaacggccaacagcgctatcggggggaatgtctccttccgcccgaaatcagcggatgattacctgcgcccgggcaagaccagcgccttcggctaccgcagcggttacgactctgcggatcgcagctggcacaacggggtgaccgtcgccggcggcgatgagttcctgcgcgggattttggtctatagccgccgtgacggccaggaaactgaaaacaacagcggcaccgtcgacgcctacccggcgaactggcactccgatgcttttctggcctccgggatctggcagcctaacgatgagcacaagctgaccagcaccttcgactattaccataaaaccaaccacacccactacgatacctgggactccagcggcaacagcaccatcggcaccgccaaccagaccagccagacccggcgctggggcctgagcctgaaggatgactggacgccgatgaacgactacctcgacagcgtctccacaaaaatctactaccagcataccgaagcccatgactggacttatatgccggacagcgtcacccgcaaaatgcagacggtgaactctaactacgataccgacacctggggcctgcagaccgcgctggcgaaaaccctgggccgccacgatctgagcgccggtttcaacgccagcaccagcaaaacccagcggccgttcagccagtcgccgatccccagcgtttacagcgagatcatgcagccggaggcagacagccgcagctacaccctcggcggctttgtccaggataagatcaacttcgatctcgacagccacaacttcgccgttattcccggcgtgcgcgtggtgcatcaatcgactaagccggaaaatctgtccgatctcgccgccaacagcagcgtgctgagcgaatcgtcggtggcgaatctgtacggcaaaaacagcgatacccaggttctgccgtcgttgaccttccagtacgacctcaccccgcgcctgatgacctacctgcagtaccagcgcggggcgcagttccccaacgccagccagctgtatggctcctggaacctcggctccagctacgccggcagccagcagtatgccctgatcggcaataccgatctgaagacggaaaccagcgataatctcgagtgggggctgaaaggggaagttaccgaaggcatcaccctgcgcacggcgctgttctacaacagctataagaactttatcgcctatacccgctatacccgcgccaacaatccgggccagttcacgaatgtgccgtcgaacatctacaccatttatcaggcggaaaaccgcgataaagcctatatctacggcggtgagattagcaccaaatttaactttggcacctggtttgagcaggtggacggcctgagcgccaccctcgccctcggctatagcgaagggaaatcgaaatccagctacagcggcgataaatacgtcgacctcgacagcgtggcgccaatgaaagccatcgtcggcgtggcgtgggacgatccggcgaaacgctacggcaccgccctgacggcgacctttgtcaaagggaaacaggcgaccgccaccaaccgcgaaagctacagcaacagcggatccgccatcaccgatgccagcagcgactatatgcgcgtgccgggctacggcatgctggactggaccgcgtactggcaggtggcgaaaaacgtgcgcctcaatggcggggtctacaacctcaccgatcgtaaatactgggattacctgagcagccgcaatatcgagaccggcaccaaccaggacgccaacgataaagcgctggcggtgatgccgggccgcacctggcagctgggcgtcaacgtcgacttctga

SEQ ID NO: 56 - DNA, 2430 bp, Klebsiella pneumoniae
atggcgatgaaaaagttgctcatagcgtcgctgctgtttagcagcgcgactgtatacggtgctgaagggttcgtggtgaaggacattcatttcgaaggcttgcagcgtgtcgctgttggtgcggccctcctcagtatgccagtgcgtcctggcgatacggtgaccgacgatgatatcagtaacactattcgcgcgctgtttgccactggcaacttcgaggacgtccgcgtcctgcgcgatggtgataccctgctggttcaggtgaaagagcgtccgacgatcgccagcatcactttctccggcaacaagtcggtgaaagatgacatgctcaagcagaaccttgaggcctcaggcgttcgggtgggcgagtcgcttgaccgcacgaccatcgcggatatcgagaagggtcttgaagacttctactacagcgtcggtaaatacagcgccagcgtcaaagcagtcgttacgccgctgccgcgtaaccgtgtcgatttgaagctggtcttccaggaaggcgtctccgcaaaaattcaacagatcaacatcgtcggcaaccatgcgttttcgaccgatgagctgatctcccacttccagctgcgcgatgaggtgccgtggtggaacgtggtcggcgaccgtaaataccagaagcagaagctagcgggcgaccttgaaaccctgcgcagctactacctggatcgcggctatgcccgtttcaacatcgattctacccaggtcagcctgacgccggataagaaagggatctacatcaccgtcaacatcaccgaaggcgatcagtacaagttttccggagtgcaggtgacgggcaacctcgctggccattccgcggaaatcgaagcgctgactaaagttgagccaggcgaactgtacaacggcgcgaaagtgaccaagatggaaaacgacatcaagaaactgttgggtcgttatggttacgcctatccgcgcgtgcagtcgcagccggagatcaacgacagcgataaaaccgttaagctgcacgttaacgtcgacgcaggcaaccgttattacgtgcgtaaaattcgcttcgaaggcaacgacacctctaaagatgccgtactgcgccgcgaaatgcgccagatggaaggcgcatggctgggcagcgacctcgtcgatcagggtaaagaccgtctcaatcgtttaggtttctttgaaacggtggatactgatacccagcgcgtgccgggcagcccggaccaggtcgacgttgtctacaaggtgaaagagcgtaacaccggtagcttcaacttcggtatcggctacggcaccgagagcggcgtcagcttccaggcgggcgttcagcaggataactggttaggtactggctatgctgtcgggatcaacggtaccaaaaacgactaccagacctataccgagctgtcggtgaccaacccgtacttcaccgtagacggtgtaagcctcggcggtcgtgtcttctataatgactttgatgcgaacgatgcggatctgtctgactataccaacaaaagctatggtacagacattacgctgggcttcccggtcaacgaatacaacacgctgcgcgccggcgtcggttatgtgcataactccctgtccaatatgcagccgcaggtggcaatgtggcgttaccttaactcgatgggccagtatccggacaacaccaacgaccggaactcgttcagtgcgaatgacttcaccttcaactacggttggacctataacaagcttgaccgcggcttcttcccaacggaaggttcgcgcgtcaacctgaacggtaaggtgaccattccgggctcagacaacgagtactacaaagcgacgctggataccgcgacctacgtgccgatcgacaacgatcatcagtgggtagtactgggtcgtacgcgctttggttatggcgatggtatcggcggcaaagagatgccgttctatgagaacttctatgccggtggttccagcaccgtgcgtggcttccagtcgaacaccattggtccgaaggcggtgtacttcccggcaagcagtcgtcatgatgatgacgatagttacgataatgaatgtaagagcaccgaatccgcaccgtgtaaatccgatgatgcggtgggcggtaacgcgatggcggtggccagccttgagctgattaccccgacgccgtttattagtgacaaatatgcgaactcggtccgtacttccgtcttctgggatatgggtaccgtatgggatactcactgggattcgagcgcgtacgctggttatccggattacagcgatccgagcaacatccgtatgtctgcgggtattgccgtgcagtggatgtcgccgttggggccgttggtcttctcctacgcccaaccgttcaaaaagtacgatggagacaaagccgaacagttccagtttaacattggtaaaacctggtaa

SEQ ID NO: 57 - DNA, 2691 bp, Klebsiella pneumoniae
atgacagatgtgactattaaagcgctggcctcagagattcagacctctgtggatcgcctgatacagcaatttgctgacgcaggcatccgcaaatcggctgatgattctgtgacctcgcaagagaaacaaactttgttgacgcacctgaaccgtgaacacggctcggcgccagacaagctgacgttacagcgtaagacgcgcagtacgttaaatattccaggtaccggtggaaagagtaaatcggtacaaatcgaagtccgcaagaaacgcacctttgtgaaacgcgatccgcaagaggctgaacgcctggccgcggaagagcaggcgcagcgtgaagcggaagagcaggcccgtcgtgaagctgaagaagcagcgaaacgcgaggcgcaattaaaagctgaacgtgaggccgcagaacaagctaaacgtgaagtcgctgataaagcgaaacgtgaagctgcggaaaaagacaaagtgagcaatcaacataccgacgaaatgaccaaaaccgcccaggctgaaaagatccgtcgcgagaacgaagccgcggaattgaagcgcaaatcggaagaagaagcacgccgcaaacttgaagaagaagcgcgccgtgtagcggaagaagcacgccgtatggctgaagaaaacgaaaaaaattggtctgaaacctcagacagcccggaagatagcagcgactatcacgtcaccacatcacagcatgctcgtcaggctgaagatgataacgatcgtgaagtcgaaggcggtcgcggccgtagccgtagcagcaaagcggctcgtccggcgaagaaaggcaacaaacacgctgaatcgaaagctgatcgtgaagaagcccgcgcggccgtgcgcggcggtaaaggcggtaagcaccgtaaaggttccgctctgcagcagggcttccagaagccagcgcaggccgttaaccgtgacgtcgtaatcggcgaaaccatcaccgttggcgaactggctaacaagatggcggtgaaaggttctcaggtcatcaaagcgatgatgaagctgggcgccatggcgaccatcaaccaggtcatcgaccaggaaaccgcacagctggttgccgaagagatgggccacaaagttatcctgcgtcgtgaaaacgaactggaagaagccgtaatgagcgaccgtgacaccggcgcggcggctgaaccgcgcgcaccggtcgtgaccattatgggtcacgttgaccacggtaaaacctcgctgctggactacattcgttctaccaaggttgcctccggcgaagcgggtggtattacccagcacatcggtgcttaccacgtcgaaaccgacaacggcatgatcaccttcctggataccccgggccacgccgcgtttacctccatgcgtgctcgtggcgcgcaggcgacggatatcgtggttctggtggtggcggcagacgacggcgtgatgccgcagactatcgaagctatccagcacgctaaagcggcgcaggtaccggtggtagtggcggtgaacaagatcgataagccagaagccgatccggatcgcgtgaagaacgaactgtcccagtacggcatcctgccggaagagtggggcggcgagagccagttcgtccacgtttccgcgaaagcgggtaccggcatcgacgacctgctggacgcgatcctgctgcaggctgaagttcttgagctgaaagcggtccgcaacggtatggcgagcggcgcggtcatcgaatccttccttgataaaggtcgtggtccggtagctaccgttctggttcgcgaaggtactctgcacaagggcgacattgttctgtgcggcttcgaatatggccgtgtgcgcgcgatgcgtgacgaactgggtcgcgaagtgctggaagcgggtccgtccattccggtggaaatcctcggcctgtccggtgtgccggctgccggtgatgaagtgaccgtagtgcgtgacgagaaaaaagcgcgtgaagtggcgctgtatcgtcagggcaaattccgtgaagttaagctggcgcgtcagcagaaatctaaactggaaaacatgttcgctaacatgaccgaaggcgaagttcacgaagtgaacatcgtactgaaagcggacgtacagggttctgtcgaagcgatttccgattccttactgaaactgtctaccgacgaagtgaaagtgaagatcatcggttccggcgtaggtggtatcaccgaaaccgacgctaccctggcagcagcatccaacgcgattctggttggcttcaacgttcgtgccgatgcctctgcgcgtaaagttatcgaagcggaaagcctggatctgcgttactactccgtcatctataacctgatcgacgaagtgaaagcggcgatgagcggcatgctgtctccggaactgaaacagcagatcatcggtctggctgaagtgcgtgatgtcttcaaatcgccgaaattcggcgccatcgcgggctgtatggttaccgaagggacgatcaaacgtcacaacccaatccgcgttctgcgtgacaacgtggttatctatgaaggcgagctggaatccctgcgccgcttcaaagatgacgttaacgaagtccgtaacggcatggaatgtggtatcggcgtgaagaactacaacgacgttcgcgttggcgatatgatcgaagtgttcgaaatcatcgaaatccagcgtagcatcgattaa

SEQ ID NO: 58 - DNA, 3234 bp, Klebsiella pneumoniae
atgaaaagaatgttaatcaacgcaactcagcaggaagagttgcgcgtcgcccttgttgatgggcagcgcctgtacgacctggatatcgaaagccccgggcacgaacagaaaaaagcgaacatctacaaaggcaaaatcacccgcattgaacccagccttgaagccgcgtttgttgattacggcgccgagcgtcatggtttcctccccctcaaagaaatcgcccgcgaatacttccccgccaactacaatgcgcatggtcgtcctaatatcaaagacgtactgcgggaaggtcaggaagttatcgtgcagattgataaagaagaacgcggcaacaaaggcgctgcgctcaccacctttatcagcctcgcgggcagctatctggtactgatgccgaacaacccgcgcgccgggggaatttcccgccgtatcgagggcgacgaccgtaccgaactgaaagaagcgctggcgagcctggagcttccggacggcatgggcctgatcgttcgcaccgctggcgtcggcaaatccgccgaagccctgcagtgggacctgagcttccgcctgaagcactgggaagcgattcagaaagccgcggaaagccgtccggcgccgttcctgatccaccaggaaagcaacgtcattgtccgcgccttccgtgactacctgcgccaggacatcggcgaaatcctgatcgataacccgaaagtgcttgagctggcgcgccagcatatcgccgcgctgggtcgtccggatttcagcagcaaaataaaactgtacaccggtgaaatcccgctgttcagccattatcagatcgaatcgcaaattgagtccgccttccagcgcgaagtgcgcctgccttccggcgggtctatcgttatcgatagcaccgaagcgctgaccgcgatcgatatcaactccgcccgcgccacccgcggcggcgatatcgaagagacagccttcaataccaacctcgaagcggctgacgaaattgcccgccagctgcgtctgcgcgacctcggcggcctgatcgttatcgacttcatcgatatgaccccggttcgccaccagcgcgccgtggagaatcgtctgcgcgaagccgtccgtcaggaccgtgcgcgcattcagatcagccatatttcgcgcttcggcctgctggagatgtcccgtcagcgcctgagcccgtcgctgggcgagtccagccaccacgtctgcccgcgctgctccggcaccggcaccgtgcgtgataacgaatcgctgtcgctctctattctgcgtctgatcgaagaagaagcgctgaaagagaataccaaagaagtccacgccattgttccggtaccgatcgcctcctatctgctgaacgaaaaacgtgccgcagtgagcgctatcgaatcccgtcagggcgatgtgcgcgttattatcgtgccaaacgacgaaatgcaaacgccgcactactccgtcctgcgcgtgcgcaaaggtgaagaaacctcaacgctgagctatctgctgccgaagctgcatgaagaagaaatggcgctgccaggcgacgatgagccggcggagcggaaacgtccggaacagccggccctggccgcttttgtcatgccagatgcgccgccagccccgatgctcgaagagcctgccgccgcgcctgtcgccgcagcggcaccggtcgcggccgccgcaccggcgcagcctggcctgctctcacgcttcttcagcgcgctgaagaatatcttctctggcgccgaagaggccaaaccggctgaagttcaggtcgagaagaaagcggaagaaaaaccggagcgtcagcaggagcgtcgtaaaccgcgcgccaacaaccgccgcgaccgcaacgaccgccgtgataaccgcgacaatcgtgacaaccgcgataaccgtgacaatcgcgacacccgtgcggacaatgccgagggccgtgaaccgcgcgaatcgcgtgaagagaaccgtcgcaaccgtcgcgagaagccgtcgcagaacgtggaagcccgtgatgttcgccaaacctcaggcgacgacgcggagaaagcgaaatcccgtgacgagcagcagccgcgccgcgaacgcacccgccgccgcagtgacgacaaacgtcaggcgcagcaggaagccaaagcgcagactcgcgaagagccggttgtgcaggagacggagcaggaagagcgtgtacaaactctgccgcgtcgtaaaccgcgccagctggcacagaaagtgcgcgttgagtccgctgtcgtcgagccagttgccgagatcgtgccagaagccgtagtggctgaagttatcgctccgcacagcgagccggtgaaagccgagctgccggcaggggtggagagcgtggcggaccaggacgaaaatggcgaatcccgtgaagcgaacggtatgccgcgtcgctcacgtcgctccccgcgtcacctgcgcgtcagcggtcagcgtcgtcgtcgctatcgtgacgaacgctatccgacccagtcgcctatgccgctgaccgtagcctgcgcatcgccggagatggcttccggtaaagtctggatccgctacccggtggttcgtccgcaggatcagcagccggaagaggttcaggttcaggacgccagcgtcgcgaaaactgtcgaggccgtagcggccccggtcgccgtcgttgaaaccgttaccgctgcgccggtcaccgtcgagccggctaccatggaaccagtaaccgctgagccggtagtcgtcgagccggtagcggccgccgagccgctggtcgttgatgctgcggaagttgtcgcgccagcagccgtcgagccagcgcctcaggagccggtcaccgaagcaccggctgtcgaagcgcctcaggctatcgcgccagtgacgctcgacgccgagccggtggtggtagaacctgaagcggtggaaacgacgcctgtcgttgcagcgccagtggaaactatcgccccggtcgcagaaaccgtggagcaagcgccagtgaccgaagcggcccctgccgaaccggtcaaagccgagcccccggtgagcaagccggtcgtagtggcgggtcatcgccatgccaccgcgccaatgacccgtgcgccagctccggactatgtcccggaagcaccgcgtcatagcacctgggtgcgcccgccgttcgcctttgaaggtaaaggcgccgccggtggtcatagcgcgacccataaagccaccgctgaaccgactcgcccacagcccgtcgagtaa

SEQ ID NO: 59 - DNA, 3480 bp, Klebsiella pneumoniae
atgcgcaagctctcactaagtttactcacgctgtccctcggcgttgcgctgctgccgttagcgcaggcggcgacgacgcctgcccaggagcatctgctggagcaggtccgcctcggcgaggccagcaatcgtgaagacctggtgcgccagtcgctgtaccgtctggagctgattgatcccaacaacccggagctgattgccgcgcggatgcgctatctgctgcgtcagggggatgccgccggggcgcaaaaagagctggaacgactgacgaagcaggcgccggactccccggagctgaaggcgtcgcgcaatgagatgaaaagcaacaccggcgagggccgccaggcgctgcagcaggcgcgactgctgggcgtggccgggaaggtcgatgaagccatcgccgcctatgaaaaactgtacggcggggtgccggatgacgttgacgtcgccattgagtactggacgctggtggcgcgcctgccggcccgccatagcgaaggcgtcagccagttgaaaaaactgaacgccagcgcgccgggcaacgtcagcctgctgacttcgctggcgaagcagatgttcgccgataacaaaccgcaggaggggttcgcctatctggcggagatggcccgatcggcctcgggacgcggtatcgccgccgatatgtggttcagtgaggtgaaaagcatgccggtgagtaaggccagcgtgcaggcgttgcagcaatttcttctgcagtttcccaccggctcggtggcggcgaacgcccgcgttctgctcgaccaacagcaggcgcagctgcaggatccgactttccgcgcccgctcggaagggctggcggcggtcaagtccgggaataccacgcaggcggtcgcggatctgcagaaagccgttcaggccgacagccgcgacagcgacgcggtgggcgctctcggccaggcctattcccagcgcggcgaccgcgcgcgggcagtggcgcagctcagtaaagcgattgctatggaccctgacagcccgaaccgcggcaagtgggacagcctgctgcaaactaaccgctactggctgctgataaagcagggggataacgccctgaaagccggccagctttcgcaggcgcagaactattatgcccaggcgcagcgggtcgatcgcaccgacagctatgccgtgctggggctgggggacgtcgcggcggcgcgcaaagaggcggcggcggcggagcgctattaccagcaggcgttgcgcctggatcgcggcaataacctggcggtgcgcggcctggccaacctctatcgcgccgaatcgccggagaaagccagcgcctggatcgccggcctccctcccgctcagcggcggagcatcgatgatattgagcgcagcctgactaacgaccggctggagaaacaggcgcaggctctggagagccagggcaactgggcgcaggcggcggaagttcagcgtcggcgcctggcgctggatccggacagcgtctggataacctaccgtctggcgcgggatctggtcagcgccggcgaacgccaggaggccgacgcgctgatgcggacgatggtcaaccgccagccgcaggacgccgaacgggtctacgcctcgggactctacctgtcggggaacgaccaggacgatctggctctggcgcaaatcgccgctctgccgcgcagcgcgtggacggataacattcgtgagctcgaagcgcgtttgcaaagcgaccgggtgctgcgccaggccaaccagctgcgcgacagcggtaacgaagcgcaggcgatcgcccttatccgacagcagcccgcctcggtgcgctatgacctgacgctcgccgactgggcgcagcagcgcggcgacagccagacggcgattgccaactatcagcgggtgctgcgccaggaggccgacaacggcgatgcgcgcctcggccttgcggaagtctacctggccgagggcgataaaccggccgcccgggcgcaggtcatgcagctgaaaggcgcagagaccgaatccatgaacatgcagcggcgggtggcgctggcgcgagctggccttggcgataccgctgacgcgcaacggatttttaatcagattgtgccgcaggcgaaggcgcagccgccctcgatggagagcgcgctggtgctgcgcgatgccgcgcgctttgccacccagagcggggcgccgcagcaggcgctgacgcactaccgggaagctatggtggcctccggcattacccccgcgcagccgcaggataacgatacttttacgcggctgacgcgcaacgacagccatgatgactggctgaagcgcgggatccgcagcgatgccgccgacctttatcgtcagcaggatctgaacgtcaccctggaacatgacttctggggttccagcggcaccggcggctattccgacctgaaggcgcataccaccatgctgcagatggatgctccgctggcggatggccggatgttcttccgcaccgacctggtcaatatggatgccggcagcttttccacccacagcgacgggagctactcgcccagctggggcacctgcggggagatcgcctgtaccagcggcagtaaaaatcagaccgacagcggggccagcgtggcggtcggctggaagaatgacacctggagcggggatatcggcaccacgccgatgggcttcaatgtcgtcgatgtggtgggggggctgagctacagcagcgacgtcgggccggtggggtacacggtcaacgtccaccggcggcctatctccagctcgctgctctcctttggcgggcagaaggacagcagcagccataccggcgccacctggggcggcgtccgcgccgacggcggcggcctgagcctgagctacgatcgcggggaggctcacggcatctggtcctcgctgggcgccgactcgctgaccggtaaaaacgtggcggataactggcgcgtgcgctggatgaccgggtactactacaaggtcatcaacgagaataatcgtcgcgtcaccgtcggcctcaacaatatgatctggcactacgacaaagatctcagcggctacaccctcggccagggcggctattacagcccacaggagtatctctcgttcgccgtgccggtgacctggcgtcagcgcaccgagaactggtcctgggagctcggcgggtcggtgtcatggtcccattcgcgcacccagacgcaagcccgctatccgctgctgaacctgatcccgtccgactaccggcagcgcgccagcgagctgacggaggaggggagcagcagccatggattcggttacaccgccagagcgctggtggagcggcgggtgaccagcaactggttcgtcggcgccgcggtcgatattcagcaggcgaaggattacaccccgagccatgcgctgctttacgtccgctactcggcggccggctggcagggggatctggatatgccgccccagccgctggtgccctacgccgactggtag

SEQ ID NO: 60 - DNA, 4236 bp, Klebsiella pneumoniae
atgagccaggaatacaccgaagacaaagaagtcaaactaaccaaactcagcagcgggcgccgactccttgaggcgatgctcatcctttgctccctcttcgccatctggctgatggcggcactactgagctttaacccctcggaccccagctggtcgcaaacggcatggcatgagcctattcataatttaggcggcgcccccggcgcgtggcttgccgataccctctttttcatttttggcgtcatggcctacaccatcccggtgatcatcatcggcggatgctggtttgcctggcggcatcaggaaaacgacgaatacattgattattttgccgtttcccttcgcctcatcggtgcgttagccctgatcctgacctcctgtggtctggcggcgattaacgccgatgatatctggtacttcgcctccggcggggtgatcggcagcctgctgagcaccacgctgcaacccctgctgcacagcagcggcggcaccatcgccctgttgtgtatctgggcggccgggctgacgctgttcaccggctggtcgtgggtcagcattgcggaaaagctgggcggcggcatcctgtccgttctcacctttgccagcaaccgtacccgtcgggatgatacctgggtcgatgaaggcgaatatgaagacgacgaggaagagtacgacgacgaagaggcggccaggccgcaggaatcgcgtcgcgcccgtatcttacgcagcgcgctggcgcggcgtaagcgtctggccgagaagtttaccaaccctatggggcgtaaaaccgacgctgcgcttttctccggcaaacggatggatgacggcgaagaggtggtgcaatacagcgccagcggggcgcctgttgccgccgacgatgtactgttttccggcgccagcgccgcgcgtcccgcagaggatgatgtgctgttctccggcgccagcgccgtgcgcccgggcgatttcgacccttacgatccgttgttgaatggccacagtatcgctgagccggtaagcgcagcggcggcggctacagccgcgccgcaggcgtgggcagaatcaccggtgggccatcacggcgctgcgccagcttatcagccggaagccagctatccgccgcagcaggcctatcagcctgaacccgctccgttccagcaggcctatcagcctgaacccgctccgttccagcaggctgcttatcagccgccagcggggcaaaccgcaccgcaggcgtatcagcctgagccagcgccgtatcaacagccggtttacgatccgcgtgccggtcaacctgcgccgcaggcctatcagcctgagccagcgccgtatcagcagccggcttacgatccgtatgccggtcaacctgcgccgcaggcctatcagcctgaacctgcgccgtatcagcagccggcttacgatccgcatgccggtcaacctgcaccgcaggcctatcagcctgagccagcgccgtatcagcagccggcttacgatccctatgccggtcaacctgcgccgcaggcctatcagccggagccagcgccgtatcagcagccaacttacgatccctatgccggtcagcctgcgcctcagacctatcagcagccggcttacgatccgaatgccggtcagcccgcgccgcagccgtatcagccggagccagcggcgtatcagccgcaaagcgcgccagttcccccaccggagccagagcccgaggtcgtgcaggaggaagtgaaacgtccgccgctctattatttcgaggaagtggaagagaagcgggcgcgcgaacgcgagctgttggcctcctggtatcagccaattcctgagccggaaagtccgattgccactaaaccgctgacgccgccgaccactgcgtccaaaccgccagtggagacaaccgtagtctctgcggtagcggctggggtgcatcaggctaccgccgccagcggcggcgcggcggcagcaacctcgtccactgccgcatccgctgcggctacgccattgttcagcccggcgtccagcggcccaagggttcaggtgaaagagggcatcggtccaaaactaccgcggcccaatcgcgtgcgtgttcctacgcgtcgggaactggcctcctacggcatcaagctaccgtcgcagcgggaggcggaacagcgcgcgcggcaggcggagcgcgatccgcattatgatgatgagctgctctcggatgaggaagcggatgctatggagcaggatgaactggctcgccagttcgccgccacccagcagcagcgctacggtcatcgctgggaagacgataacgcgactgatgacgatgaggccgacgccgcggcggaagcggagctggcgcgtcagtttgccgctacccagcagcagcggtacgctaccgagcagccgccgggcgccaacccgttctcgccggcagattatgaattctcgccgatgaaaacgttggtcaatgacggcccgagcgaaccgctgtttacgccgacgccggaagtccagccgcagcagccggcccagcgctatcaacaaccggcggccgctccgcagcagggttatcaacctgcgcagcatcagccgatacaccatcagcctgtgccgccacagccgcagtcctatccgactgcgtcgcagcccgtacagccgcaacaaccggttgccccgcaggggcatcagcctgccgcccctgcgccgcaggagagcctgatccacccgctgctgatgcgcaatggcgatagtcgaccgctgcaaaagccgaccacgccactgccgtcgctggatctgcttaccccgccgccgagtgaagtcgagccggtggatacctttgctctcgagcagatggcacgcctggtggaagcgcgactcgctgatttccgcattaaagcggatgtggtgaactactcaccggggccggtgatcacccgcttcgaactgaatctggcgcctggcgttaaggccgcacggatctctaacctgtcacgggacctggcgcgatcgctgtcaacggtcgccgtgcgcgtggtggaggtgatcccgggcaaaccgtatgtcgggcttgagctgccgaataaaaaacgccagaccgtctacctgcgtgaagtgctcgacaacgccaagttccgtgataacccatctccgctcaccgtggtgttgggtaaagacatcgctggcgatccggtagtagccgatctggcgaaaatgccgcatctgctggtggccggtaccaccggttccggtaagtctgttggcgtcaacgccatgatcctcagcatgctctacaaggcgcagccggaagatgtgcgtttcattatgatcgacccgaaaatgctcgagctgtcggtctacgaaggaattccgcacctgctgacggaagtggtcaccgacatgaaagacgccgccaatgcgctgcgctggagcgtcaatgagatggagcgccgctacaagctgatgtcggcgctgggcgtgcgtaacctcgcgggctacaacgagaagatcgccgaagccgcgcgcatgggacgtccgatcccggatccgtactggaagcctggcgacagcatggacgccgtacatccggtgctggaaaaactgccgtacatcgtggtgctggtggatgaattcgccgatctgatgatgaccgtcggcaaaaaggtggaagagctgatcgctcgcctggcgcagaaagcgcgcgcggcggggatccacctggtgctggcgacacagcgtccgtcggtagatgttattaccggcctgattaaggccaacatcccgacgcgcatcgcctttaccgtgtcgagtaaaattgactcacgtaccattctcgatcagggcggcgcggaatcgctgctgggtatgggggatatgctttactccgggccgaactctaccacgccggtgcgtgtccacggggcgtttgtgcgcgaccaggaagtccacgccgtggttcaggactggaaagcccgcggtcgcccgcaatatgtggatggcattacctccgacagcgaaagcgaaggcggcggtggcggcttcgacggcggggaagagttggatccgttgttcgatcaggcagtcaactttgtgaccgagaagcgcaaagcgtcgatttccggggttcagcgtcagttccgcatcggctataaccgtgccgcgcgtattatcgaacagatggaagcgcagggtatcgtcagcgagcagggccataacggtaaccgcgaagtgctggcgccgccgccctttgaatga

SEQ ID NO: 61 - RNA, 285 nt, Klebsiella pneumoniae
augaagaaguuagcuuuacucuccgccguaaugacgcuuggaaugucgucaugggcuuuugcugccgacaacccgccgccgccgccggaaaaaggcgcgcagcaucaggguaaaccgccggugaaaaacggccaacacgaagguaagcaagcgcaauacaacagaaaacagccacaacgagacggcaaacagccgcagcacgacgguaaacagccgcagcacaacggcaagcagccgccaaaagggagcgagcacagcgggaaaccgcugccgccgaaagcguaa

SEQ ID NO: 62 - RNA, 354 nt, Klebsiella pneumoniae
augaaacguuacgcaaccgcacugcucuuuugcacucugucgcugaccagccuggccgcucgcgccgauauuaucgaugacgcgaucggcaauauucagcaagccauuaacgacgccuauaaccccggcagcagucgcuccgaugacgacgacagauacgaugacgauggccgguaugaugacgggcgcuaucaggggagccgucagcagagccgugacagucagcgccaguaugacgagcggcaacgccagcuggacgagcgccgccgccagcuggaugaacgccagcgucagcucgaccgcgaucgucgucaguuagaaagcgaccagcgucgucuggaugauagcuacuga

SEQ ID NO: 63 - RNA, 360 nt, Klebsiella pneumoniae
auguucaggucacugauucuggcagcaguacugcuggccgcagggccacuggucgcuaacgcuggugaaaucacccugcugccaucgguaaaauuacaaauaggcgaucgugacaauuacgguaacuacugggacgguggcagcuggcgcgaccgugauuacuggcgucgucacuaugaauggcgugauaaccguuggcaucgucaugacaacggcuggcacaaaggcugguacaaaggcagagauaaagccugggagcgcggcuaucgugcuggcuggaacgaccgcgaugaccaccgcggcggcuggggucgcggcccgggcgggcgcggucacggucauggacauggccaucacuaa

SEQ ID NO: 64 - RNA, 363 nt, Klebsiella pneumoniae
augaaggaaaucggcuuaccguuauugcuacugaccgcgcuggccaguccggcuuuugcugcagacugucagccaaacggcauuggcggcucguuuugcauuaacgaugacgguacgacuaccgacacggugccuaacgaagucaacggcauggauacguacucgaauaauggcggcuauaccaguucccugcccgaucggucaggggcggaugaagcacuggaagguucaucgcugucgacgcagcaaggcgucggcagcggacagagcgacagugcgcuggcgggucgcgacuggcauucgcccgccaaucugaaugauggcgccgccaccuccaguaugagccugcuggauaaacccuga

SEQ ID NO: 65 - RNA, 366 nt, Klebsiella pneumoniae
augaauaugaaaaaacugacgacccuuuugcucaccgccaccuuaggucuugccagcggcgcggcccuggcggcagacaccggcgcccaguccaauaauggccaggccaacucuuccgcggaugccggucagguggcgccggaugcccgugagaacguggcgccgaacaacguggacaauagucagaucaacucuggcucugggggcaccacgggcucgacgaugacccaggauaauaugucgagcaaugagguacauaaaaacucgauguguaaagacggccgcuguccggacaccgguaaaaaacuggacaacgguggcaauacgacccaagacaacagcaaaaccgacggcaccacccaguaa

SEQ ID NO: 66 - RNA, 369 nt, Klebsiella pneumoniae
augaaacaccgcaucgcucugcuucugguccugacuucacuuagcgccagcgcccuagccgccucucccugccaggaaaaagagcaggauauucaacgagagaucagcuacgccgaaaagcaucauaaucaaagucgcauugaugggcuaaauaccgcgcuacgucagguucgggaaaacuguagcgacaguaaacucaaagccgaucaucagcaaaaaauugccaaacagcgggaagagaucgcugaacgucagcgcgaucugcaggaagcccggaagaaaggcgaugcggacaaaauuaacaaacgccagcauaaacucaaugaagcgcaacaggaguuaaaaacgcuggagucucgggauuacuaa

SEQ ID NO: 67 - RNA, 426 nt, Klebsiella pneumoniae
augcgacucauaacacgacacgugagagaggauauuaugaaaaaagcaaugauugcguuaucggcuauucugguugcggcuccgguuuuugcugcgacaacacaugcaacagaugauaccgucgcggcggcgaaugccaacgccaacaccgcuaaagagaagcugcaucaggcccagcacgagggcgaagagcagcagcugaaggcgaaacacgccgccgaaggcaagcaggacagcgucggcagccaggugagcgaaggcgcgcagaaaaccuggaacaagaccaaagaaggcaccgagaaggggugggauaagaccaaagaggucagugaaaaaggcuggaacgccaccaaauccggugcggaaaagggcugggauaaaaccaaaaccggcgccgaagaguuaaaaaauaaagugacugaauaa

SEQ ID NO: 68 - RNA, 456 nt, Klebsiella pneumoniae
augaaaaagaugauuucucuggcaguaauuuuauccugugugcugagcgucccggccuuugccgauggcccgaacgacggccaucgcccggagcagcccacgguguggcagaacgguccggaccaugacgggcaugcaccgcagggcggaccugacgcgcaucaucagggcgaccaugaccagcguggcccggaucgcgacggccaugacaaacgcgaucuggcacgucaugagcaggaccauuucgccuggcgcgggaacgauuuccgcaaaggccacccggcuccggcgccguuccguggcgaugaauaucgcguccgcgacuggagcgaccgcggccugccgcccccgccggaaggccaucacugguccuauaucgacgguaacuaugugcugaucgccgcggcgaccgggaucaucaccucgauucuggugagcggcgcccucggccacuaa

SEQ ID NO: 69 - RNA, 507 nt, Klebsiella pneumoniae
augaaaaaaccgacauccgccacccguggcaaauccggccgcaagucgcgugaagaguuaaaucaggaagcucgcgaucgcaaacggcagaagaaacaucguggccacgcggcaggcagucgcgcgaacggcggcgaugcggcuucagcggguaaaaaacagcgucaggcgcaagauccgcgcguggguagcaaaaaaccgaucccgcugggcgugagcgaaagcagcguuccagcucccaagcagcauaaaccaaagagcgagaaaccuaugcuuucaccgcaggcugagcuggaguugcuggagaaugaugagcgccuggacgcgcugcuggaacgucuggaagagggcggcacccugaaugcugaagagcagagcuggguggacgccaaacuggaucgcauugaugagcugaugcagcagcucggccucucuuacgaugaugaagaugaagaagaggaagagcgucaggaagauaugaugcgucugcugaaggguggaaacuaa

SEQ ID NO: 70 - RNA, 690 nt, Klebsiella pneumoniae
auggcgaguaaguuucagaaccguuuagucgggacaaucgugcugguggcgcugggggugauuauccugccagggcugcuggacgggcagaaaaagcauuaccaggaugaguuugccgcgaucccgcugguaccgaaaccaggcgaucgcgaugaaccggauauguugccggcggcaacccaggcguugccuucgcaaccgccggaaggggcggcggaagaggugcgggcgggcgaugccgccgcgccaucguuagauccaucgcguauuccggugaacagcaacagcuucgaugacguucaggagccggugguggccgcgaaaccgcagcccaagccgcagccgaaaccgcagccgcaacagcaggccucgacgccaacgccgccgccggcuaagccacagcagcaacagccaccgcagcagcaggcggcccugccggcgccgaccggcaaagccuaugugguucagcugggcgcguugaagaacgccgauaaggugaaugagauugucgguaaacugcgggccucggguuucaaagucuauacgucgccuucgacgccgguacaggguaaaauuacccgcauccucgucggcccggaugcgucaaaagacaagcugaaaggccagcugggcgaucugcagcagaucuccgggcuuagcgggguggugaugggcuucaccccgaacuga

SEQ ID NO: 71 - RNA, 969 nt, Klebsiella pneumoniae
auggcacaacgagauuauguacgccgcagccaaccggcuucuucgcggcgcaaaaagagcacgacccgaagcucaaggaauaagcaaagcagccuuccggcgauuucaccggcgaugguggcgaucgcggcggcugugcugguggccuuuaucgguggccucuauuucauuacgcaucauaagaaagaagaagcggaagcgaugcaaaaucgccaggccgccggcaacggcuugccgcccaaaccggaagagcgcuggcgcuauauuaaagagcuggaaagccgccagccuggcguccgcgcgccgaccgaaccgaccgccgguggcgaagucaugaaaccggaacagcugaccgacgagcagcgccagcugcucgcccagaugcaggccgauaugcgccagcagccgacccagcugaccgaagugccguggaacgaacaaacgccggcgcagcgccagcagacgcuucagcgucagcguuuagcgcagcaacagcagcaggcgcagcagcaacagugggcgcagacucaggcgcagaccguccaacagcagccgccgcgcguucagcagccgaagccgguucagcagcaacagccgaagcagaccgcgucaaaccagcagccguaccaggaucugcugcagacgccagcgcauaccaauaccacgcagccgcguacccaggccgcggcgccgguaacucggguggaagaagcgccgaaaaccaccgccgagaagaaagacgaucguagcuggaugauccagugcggcucuuuuaaaggcgccgagcaggccgaaaccguccgcgcucagcuggcuuucgaaggguuugcuucgcacauuaccacuaacaacggcuggaaccgcgugguuauuggcccguugaaaggcaaagaaagcgccaacgagaugaucacccgccugaagauggcuggacacgcgaacugcauucgucucgccgccagggguuga

SEQ ID NO: 72 - RNA, 1131 nt, Klebsiella pneumoniae
augagcgcgggaagcaccaaauuuaccgucagccguauugcggcucuuucacugguuucacucuggcuggccggguguaccaacaccaauaauccgccugcgccgguuagcucugccggcggcgccgccucuuccagcaccaacuccggcaugcugauuacgccgccacccuccggcgucaaguccgcuccucaggcgcagccgauucagccgaugcagacccagaccauucagccggcgccgguggcgcaggagccgguacagacgguaaauggccggaucguuuacaaccgcaaauauggcgauauuccgaaagguagcuauaccggcggcaguaccuauacgguaaaacgcggcgacacgcuauucuauaucgccugggucaccggcaacgauuuccgcgaccuggcgcaacguaacaauaucccggccccguacgcgcugaacguggggcagguacugcaggucgguaacgccucaggccagccgaucaccggcgaaaacgccguuucucaggccagcgcaagagcgagcggcggugcgacgaccagcacaacuucugcacaaaaaucgaccgcggugguugcuucacaaccgacuauuacguauucugaaucuucaggugaacagagugcuaccaagauguugccuaauaauaaaccagcgaccacaaccacaacgguugucgcgccggugacggcaccaacaacggugagcacaacccagccgacugcaagcaguacgucaaccaguucgccgaucucagcauggcgcuggccgacugauggcaagguuaucgagaacuuuagcggcgcggaaggcggcaauaaaggcaucgauauugcaggcaguaagggacaggcuauugucgcgaccgccgaugggcgcgucgucuaugccgguaacgcacugcgcggcuacgguaaucuuauuaucaucaaacacaacgaugauuaccugagugccuacgcucauaacgauaccaugcugguucgggagcaacaggaagucaaagcggggcagaaaaucgcuaccauggguagcaccggaaccagcucaacaagauuacauuuugaaauucguuacaaggggaaauccgucaacccgcugcaguacuuaccgcagcgauaa

SEQ ID NO: 73 - RNA, 1149 nt, Klebsiella pneumoniae
augcguaagcaauggcuggggaucugcauagcagcggggcugcuggcggcauguucgagugaugacgugcaacaaaaaacggucaguacuccacagccggccgucuguaauggcccgacgguugagaucagcggcgccgauccgcaguaugaaacgccgaacgccacggcgaaucaggauuaugagcgcgacgguaaaagcuacaaaaucguucaggauccggccaacuuuacucaggccgguuucgcggcgaucuaugacgcagaacccaacagcaaccugaccgccagcggcgaagccuucgauccgacucaguugaccgcagcgcacccgacgcugccgaucccgagcuacgcgcggaucacuaaccuugccaacggacggaugaucgucgugcggauuaacgaucgcggucccuauggcaacgaucgggucaucucgcuuucccgcgcauccgcugaccgccugaacaccuccaacaacaccaaagugcgcaucgaccccaucaucgucgcgccugacgguucgcuuuccggcccggggauggccuguaccaccgucgccaaacagacuuacgcccugcccgcccguccgaaucuggacgguggggacgccgcuggcaugagccagcccgcgcccacugacguucgcccgaucagcaacagcacgcugacgccggcagacagcgugggcgcgccggugaacagcggcgguuuccucggcgcgccgacgccccugaacaacggcgugcuggagaguagcgaaccagcggcagccgccgcgacggcuccugccgccggcgccacgccaacagcgccagugaccgcgccuggcuccauucaggguaauguggugcccgcugcggccaccgccgcagccgcuggcgccguggcggccucguccuccgcgaccuccagcgccagcgguaauuuuguuguccaggugggcgcaguaagcgaccagacgcgggcgcagcaguaucagcagcgccugagccagcaguuuucugugccaggccgggucaugcaaaacggcgcggucuggcguauucagcugggucccuuugcugauaaagcacaggccagcgccgugcagcagcgccugcaaagcgaagcgcagcugcaguccuuuauuacucgcgccaacuaa

SEQ ID NO: 74 - RNA, 1287 nt, Klebsiella pneumoniae
auggaugauuucaaaccagaagacgauaugaaagccgaucgcaacgaucgucgugcuggucguucccgucagucuuccgagcgugaugccgauccgcagaucaauuuugacgauguugaucuugaugccgaugaaggccguccgacgcgcgcugguaaggcccgucgcgagcgugaagaggaagaguucgaagaagaacuggaugcgcaagacgaggagaugcucgaagagcagccuguagagcgucguccgcgcaagcguaaaaaagcgccggccaaaccggccucccgccaguacaucaugauggguguggggauucuggugcugcugcuguugaucguggguaucgguuccgcacugaaaucgccaucaucuuccagccagcagaccgcuuccggcgagaagagcauuaaucugucugacgaccaguccgccagcaugccugcugccggccaggaccagacugccgccgcuaacagcaccucacagcaggacguaacgguaccgccuauugccgcgaacccgacgcagggccaggcagcgguugcgccgcagggccagcagcguaucgaaguucagggcgaucugaacaaugccuugacccagcagcagggccaacuggacggcgccguggcuaacucgacgcugccgacugaaccggcuaccgucgcgccaauccggaauggcgccaauggcaccgcggcgccgcgccaggcgaccgagcgucagacagcagcgaccccgcguccggcugaacguaagcauaccguuaucgaagcgaagccgcagucgaagccacaggccguggcgaaaacgccgguagaaucgaagccgguccagccgaagcauguugaaagcacggcgaccaccgcuccggcgaaaacguccgucagcgaaagcaaaccgguggccaccgcucagagcaaaccgaccacgacgaccgcagcgccagcggcaacggcagcugcggcagcgccggcagcgaagaccgggaagacggcaggugacgucagcucaaugaaaacugcgccgucgggucacuauacucugcagcucagcagcuccucuaacuacgacaaccucaacaacugggcgaagaaagagaagcuggauaaauauguugucuaugaaacgucgcguaacggccaaccaugguacgugcuggugagcgguaucuaugcaucgaaagaugaagcgaaacgugcugucaccucgcugccggcggacgugcaggcgaaaaauccaugggcaaaaccgcugcaucagguucaggcugaccugaaauaa

SEQ ID NO: 75 - RNA, 1326 nt, Klebsiella pneumoniae
augucaaaggcaaccgaacaaaacgacaagcuuaaacgagcgaucaucauuucagucgcgcugcacaucauucugaucgcgcugcugaucuggaguucguuugacgagcaucuggaugccucugccggcggcggcggcggaucgucgauugaugccgucauggucgauccgggggcggugguaaauaacuauaaccgucagcaacagcagcaggccagcgcacgucgcgccgcugaacagcgugaaaaacaggcgcagcagcaggcggaagaguuacgugagaaacaggcggcggaacaggaacggcugaaacagcucgaacaggagcggcugcaggcgcaggaagcggcgaaagaagcgaaggagcagcagaagcaggcugaagaagcggcugccaaggccgccgcggcggcaaaagccaaagcggacgcacaggcaaaagaagcgcaggaagccgcugccaaagcggccgccgaggcgaaagcgaaggcggaugcccaggcgaaagcggcagaacaggcggcggccaaggcggcugcugacgcgaaaaagcaggccgaagccgcugcagcgaaagccgcugccgaggcgaagaaacaggcggaagcugaagcggcgaaagcugcggccgaggcgcagaagaaagcggaagcggcggcugcgaagaaagcgcaacaggaagcggagaaaaaagcccagcaggaagcggcuaagcaggcggcagcugaaaaagcggcugccgaaaaagccgcugagaaagccgccgcgcaaaaagcggccgcugagaaggccgccgccgagaaagccgcagccgcugaaaaagcggcggcagcgaaagcggcugcagcagagaaggcugcagcugauaaagcggccaaagcggcagcagcaaaagccgcggcggcgaagaaagcggcggcugcgaaagaagcggacggcguugacaaccugcucggcgaucugaguucugguaagaaugcgccuaaaacaggcgguggggccaaaggaaacaaugccuccgcugccgggagugguaauacuaaaaacagugccucaggggcugauaucaacaacuaugccggacagauaaaaucggcgauugaaaguaaguuuuaugacgcaucguccuaugcgggcaaaacauguaccuugcguaucaaacuugcuccugacggccuguuguuaaauauacaguccgaagguggugauccugcucugugccaggccgcucuugccgcagcccgacaggcuaaguuuccgaaaccaccuagccaggcaguauaugaagucuucaaaaaugcgccacuggacuucaaaccucaguga

SEQ ID NO: 76 - RNA, 1455 nt, Klebsiella pneumoniae
auguuuuuuuuaaguauuuuuuacauggagaugacaaaagugaaauuaagcgcucuguuuauugcccugauuccucuacugggcucgccgguuauucaugcagaaacuacugcugcgccgguucuggaaaaucgcgcugcgcagggagauaucaccacuccuggcggcgcgcgucguuuaacaggcgaucaaaccgaagcgcugcgcgccucguuaaucaauaagccagcuaaaaacguuauuuugcugauuggcgauggcaugggugauucggaaauuaccgcugcgcgaaacuaugccgagggggcgggcgguuucuuuaaaggaauugaugcucugccguuaaccgggcaguacacgcauuauucgcuggauaaaaaaaccgggaaaccggacuacgugaccgacucggcggccuccgccaccgccuggaccaccggcgugaagacuuauaacggcgcgcugggcgucgauauucaugagaaugcgcaucagaccauccucgagcuggcgaaagcggcggggcuggccaccggcaacguuuccaccgccgagcugcaggacgccacccccgcggcguugguagcgcaugugacaucgcguaaaugcuacggcccgacggucaccagcgaaaaaugccccagcaaugcgcuggaaaaagggggcaaaggcuccauuaccgaacagcugcugaacgcccgaccggaugucaccuugggcggcggcgcgaagaccuuuaccgaaacggcgacggcgggcgaguggcagggcaaaacccugcgcgagcaggcgcaagcgcgcggcuaccagauugugaccgacgcggcuucucuugccgccgcgacggaagccagucaggauaaaccgcugcugggacucuuugccgauggcaauaugccgguacgcugggaagggccgaaggcgucuuaucacgguaauaucgauaagccgccggugaccuguacgccaaacccgaagcgugacgccucggugccgacgcuggcgcagaugacggagaaagcgauugaccugcucagucgcaacgagaaagguuucuuccugcaagucgaaggcgcuuccaucgauaagcaggaccaugcggcgaauccgugcggccagaucggcgaaacgguugaucuugacgaagcggugcagaaggcgcuggaauucgcgcgaaaagacgguaauacccuggugaucgucaccgccgaccaugcgcaugccagccagaucaucccggcggauagcaaagccccggggcugacccaggcucugaacacgcacgauggcgcggugauggugaugagcuacggcaacucugaggaagagucgauggagcacaccggcacccaacugcgcauugcggccuacgguccgcaugcggcuaacgucguaggccugaccgaucagaccgaccuguucacgaccaugaaagcugcccugagucucaaauaa

SEQ ID NO: 77 - RNA, 1608 nt, Klebsiella pneumoniae
augucacugccguucaaaccccauauuaucgcccugcucuguagcgcuggcuuacucgcggcggcaggaacacucuaugugcaaagccgaaccccagcgacgaucgcugaaccgccugcgcagcaagcgccagcgcccgcagcgucgacgacacagccgguggccgccacuuacacccaggcgcaaauugaucagugggucgccccuaucgcgcucuacccggacagccugcugucgcagguguugauggccuccacuuaucccgacaacguccugcaggcgguccaguggucccaggauaaccccgcgaugaaaggggaugcggccgugcaggcgguugccagccagccgugggacccuagcgucaaaucucuugucgcuuucccugcccugcuggcgaugaugggcgagaauccgcccuggguggaaaaucuuggcaaugcguuuuuggcccagccgcaugaugugauggauucagugcagcgccugcgcgccauugcccaacaaaccgggacgcugaaauccacaccgcagcagaaagugauugucaccccugccgcaccgguuucagccagcagcagcacggcagcaaccgcaaccgcccacacagcggcgccugcgcccacgcaggucauuaaaauagagccgaccaauccacagguggucuauguucccagcuauaaccccuccaccgucuaugguaccuggccgaacagcgccuauccgccggucuaucugccgcccccucccggggagcaguuuaccgauagcuucgucaaaggcuucggguacagccucggcguggccaccaccugggcgcuguucagcaguaucgacugggaugaugaugaccaucaccaucacgaugacgacuaccaccacggcgauuacucgcauaauggcgauaacaucaauauuaauguaaauaauuucaaucauauaacaggagaaaaccugccgggaaaccacguuaacuggcagcacaauccugccuaucgcggacacacaccguaucccgauaauacgguagcucagcgcuuccaucagaccaacguuuccggcggacugagcgcgacccaacaugcgccagucgaucgcgaagcgcagcgccaggcagcgaugacccagcugcagcauaacguaccgacggccacagcgggcaaccuggcggcaaacaacgccucacgcgacgcccagcgucaggcggccucggcgcagcugaagcaagccacccaacgcaguaauuaccgcgguuacgacaguacgccgacccaacagcagcgucgcgaggcggcaaaaacgcagcugaaaaaccccacgccgcagcaacagcagcgucgagaagccgccaggagccacgagcagaaccgcacaccucagcagcagcagcgccggcagcaguuccaguccgccacgccagcccagcgucagcagacgcucagccaucugcgcgccaacgcccuuagcggcaacgaaagccgcgcccccuccuggcaagcgcagcaggaacgaggacugcagagccgccaguuuuccggcguaaaccgcgaguuacgcgauggcaccagagaacgucuuuccgaacaccaugaacugcgucgccgcuaa

SEQ ID NO: 78 - RNA, 1794 nt, Klebsiella pneumoniae
auguuuaaguuuaaggcuucuuaugucgcacuggcggcaguauuaaccucgucgguaguuuaugccgaccccacaagcuauacgcacucuuccggcgccacgguuaucgauauugaaaagccgaacgccgccggugucucccauaaccuguaccgcgacuucaacgucggcgccaauggcaccauccucaauaacagcggcgaugaugucagccacagcacauuuggcaauaucgcccgcaacaauaaucugaccgccggcagcgcuucggugauuuugaacgaggugaccuccaaaaacgccaguagccugaagggcuuuaucgaagucaacggucagaaagcggaugugguaaucgccaacccgaacggcaucaccuguuccggcuguagcuuuguuaauaccaacaaggcuauccugaccaccggcaagguuaauaugaccgacgauggcgcuaucggcagcuauaccguaacgggcggcacccucaccaucggcgaaaauggcaugaacgccgccaacggcuaugcgguucugcucgccgacgcgaucaauaucaacgguaaagugcaggccaacaacgcccuggucagcgcgggcaacuucaccauggauaacagcucuggcucggugaccuccgcugguaaaaaggccacccugauccagaugacgguuaacccgcaguacagcaucgacgucagcagccuuggcggcauugaggccaacagcaucagcauggucggcaauaacaucggcuuuggcguacguaauaaaggcucuaucgucgcgaauaguucgcugcagcucaccagcaacgguaaucugcugaacaaaggcacgaucaaaagcaacggucugcugagucaggucgccaccgccucgggcaucaccaaugacgguagcaucgccggcgccuauuauuuaaugcucuccaguggcgauuauaucguuaacaccgguucucucuccggcggccagcugauugccaccgcuaacggcaacaucaccaacggcgacucaggcacgaugaccggcaccaguggauuaagccugaccagcggcgggaaaauccgcaacgaagaaaaagccucccugcugucaaauaaccagauugccgccacggcaaucggugauuuccucaaugaaggcaaaaucagcgccaaacacaccagccugacguuugucggcgacagcuuuaaaaacacuggcaauauuaacucuacuggccaaaccaccauucagucgcuuaaacaggacggcagcgccaauacgggcgagaucuauaaccucggcaauaucaccggcgaaaauaucaaucugcagaccaauggcacgcuggcgcaaagcagcaguggucguauugaggcaaccaacgccauuaccgcccacagcuacuggcugaaccaaaaugguuauaugaaugccgccgauaucaccaccgaucacggcguagugaauaauuauggcaauauuacugccaaaaauauuucaaucacgaccuacucagauaucaccaacgaagggcagaucagcagcaccggcgaccugaccuuaaauaccaaaaauaaaggcgcgaucuacaauuauucaacccucagcgcgggcggcaacaugacguuaaccgccaccaaaguggucaauggugguaaaaguugcggcauacugggccuggcgaaaugcggcgucgggacguuaacugcugacaagcugguacugaacucaucgcagaaauauguuagcgacauggguggaaaacaguauuucaagagcaccgaagucaacacggugaaauaa

SEQ ID NO: 79 - RNA, 1875 nt, Klebsiella pneumoniae
augauggacaaccuacgcacggccgccaacagcgucgugcucaagauuauuuucgguaucauuaucgucucguucauuuugaccggggugagugguuaccugauuggcgguggcaaaaacuaugccgcaaaagugaauggccaggagauuggccgugggcaguuugaaaacgccgucgccagcgaacguaaccguaugcagcagcagcuuggcgaucaauucuccgagcuggcggcgaacgaaaacuacaugaaaaccaugcgccagcaggugcugaaccgccugaucgaugagucgcuucuggaucaguaugcccgcgagcugggccucagcaucagcgaugagcaggugaagcaggcgaucuuccagacccaggcguuccagacgaacgguaaguucgacaaccagcguuucagugguauugucgcccagauggggaugaccaccgaucaguacgcccaggcgcugcguaaccagcugaccacgcagcagcugauuaacgccauugcggguaccgacuucaugcugccgggcgaguccgaucagcuggcggcgcugguaucucaacagcgggugguccgcgaagcgaccaucaacguaaaugcccuggcggcaaaacagaccgccagcgaugaggaaaucaacgccuucuggcagcagaaucaggcccguuuuauggcgccggagcaguuccgcgucagcuacaucaaaauggaugccgccagcaugcaggagagcgccucugacgaagagauucagucaugguacgaccagcacaaggaucaguucacucagccgcagcgcaaccgcuacagcgugauucagaccaaaacugaagccgaugcgaaagcgguacuggccgagcugcaaaaaggagcggacuucgccacgcuggcgaaagaaaaaucgaccgauauuaucucugcccgcaacgguggcgauaugggguggauggaagaugccucuaccgugccugagcugaaagaugccgggcugaaagagaaaggccagcugucuggcgugaucaaauccucgguuggcuuccugguagcucgucuggacgacguccagccggcgcaggugaagccgcuggcugacgugcguaaugacauugcggcgaaagugaagcaggaaaaagcguuggaugcuuacuacgcgcugcagcagaaggugagcgaugcggccagcaacgauaaugaaucgcuggcgagcgcagcgcaggucgccgggcugaaggucguagaaaccggcugguuuggccgcgauaaccugccggaggagcugaacuuuaaaccggucgcugacgcuauuuucaacggcggucuggugggugagaacggcgcgccgggcagcaacuccgauaucauuaccguugacggcgaucgcgcuuuuguucugcgcauuagcgaacacaaagccgaggcggugaagccgcuggccgaagugaaggcacagguuagcgauaucguuaagcacaauaaagcggaacagcaggcgaaacuggaggccgacaagcugcuggcggcgcugaaagacggcaaaggcgaugaagcgaugaaggcggcuggccugagcuuuggcgcgccgcagacgcuuucucguaccggccaggauccgcugagccagcuggcauuuacccugccgcugccgcagcaggguaaaccggucuacggcgugggcagcaauaugcaaggcgauguggugcugguagcgcuggaugaggugaaagccggcagcaugccggaagagcagaagaaggccaugguucaggggaucacccagaacaaugcccaaaucgcuuucgaagcgcugaugagcaaccugcgcaaggcggcgaaaauuaagcucggcgacagcaucgaccagcagcaguaa

SEQ ID NO: 80 - RNA, 1974 nt, Klebsiella pneumoniae
auguucagguuaaacccuuuuauccgggcgggauugucugcguccgucguaucguuggcguuuccggcucuggccgaugugaaugaagaaacgcugguggugaccgccucggccacugaacagaaugucaaagacgcgccggcgagcaucagcgucaucacccaacaggauuuacaacgcaagccuguucagaaccugaaagacgugcugcgcgaugugccugggguccagcucaccaacgaaggggauaaccgcaagggcguuagcauccgcggucugagcagcagcuauacccugauccuggucgacggcaagcgcguuaacucgcggaacgccgucuuccgccacaaugacuucgaccuuaacuggaucccgguggaugcuauugagcguaucgaaguggugcgcggcccgauguccucccucuacggcuccgaugcgcucggugggguggucaacauuauuaccaaaaaaaucggccagaaauggaccgggacgcugagugcugauaccacuauucaggagcaccgcgaucgcggggauaccuggaacggccaguucuucaccagcggcccgcugaucgacggcguacuuggaaugaaggccuacggcagccuggcaaaacgcgccaaggacgauccgcagucauccaguaaugccaccggcgagacgccgcgcaucgagggcuucaccagccgcgauggcaauguugaauucgccuggacgccgaacgaaaaccacgauuuuaccgcaggcuacggcuuugaccgucaggaucgcgauuccgauucccuugaccgcaaccgccuugagcgggagaacuacucucugagccauaacggccgcugggauaucggcaauagcgagcucaaguucuacggcgaaaagguggauaacaaaaauccagggcagagcgggacuauuaccucggaaagcaaugccaucgacggcaaguauguccugccgcugggcaugauuaaccagcuggugaccuucggcggcgaauggcgccacgacaaacuuaaagauccggucaaccugagcagcggcggccagucaacgucggccagccaguacgcccuguuuaucgaagacgaauggcgcaucaucgagccgcuggcgcugaccaccggcauucguauggacgaccaucagaccuauggcgaucacuggagcccgcgcgccuaucugguguauaacgccaccgauaccgucaccgucaaaggcggcugggcgacggcguuuaaagccccgucgcugcugcagcuuaaccccgacuggaccaccaacuccugccgcggcucgugcagcaucgucgguaacccggaucugaaaccggaaaccagcgaaagcuucgagcucggucucuacuaccgcggggaagagggcuggcuugaaaaugucgaaggcagcaucaccaccuuccagaauaaugucgacgacaugaucgacguucugcgcaccuccagcgccagcgaagcgccgggcuacccgaacuuugucggcuggaaaacugucaacggcaagcgcgugccgaucuuccgcuauuucaacgucaacaaagcccgcaucaaagggguggagacggaggugaagaucccguuuggcgaugaguggaagcugacggugaacuacaccuacaacgauggucgcgaucugagcaauggcggcgacaaaccgcugcagacgcugccguuccauaccgccaacggcacgcucgacuggaaaccgcuggacgacugguccuucuacgugacggccaacuauaccggccagcagcgcgcggugagcgccaccggcaaaacgccgggcggcuacacccuguuugacguuggcgcggcauggcaggugaccaaaaacgugaaacugcgcuccggggugcagaacgugggugauaaagaucugagccgggacgacuacagcuauaccgaagaaggccgucgcuacuuuauggcgguggauuaucgcuucuga

SEQ ID NO: 81 - RNA, 2028 nt, Klebsiella pneumoniae
augaacagagccgccacgcugacccucaacgcgccccugcugaugcucgucgcugcgcuggcgcuuucaaccccuuucaccgccggcgccgcgccggccuuucuugauuacgcccaacagcaaacccagcaaucucaggcgcaagaaaaaaacgaugccgcaagcgcaaaacaaacacaagaaagccgccagagcgcagauaauaaaaaaaccgguaccagcaccucacaauuacaaaaaagaaucaccagccagcaggcggcgauugcacaaaaagauaagcuuauacagcaauuaaaaaaacagcuugccgcuacgccgcaaacggauacugccggagcgaaugagcaagcggcguugaauaagagaauuaaugaauuacaggucgccuuaagcgccgcuacugcagaaaaagaggcauuaauaaaaaaagcaggcguugugcagaauaauaaucuacagcaaagccaggccgcggcgcgucagcagauccagcaauuaacgacgcagauucagcaagccgaagcugaaaauaaacgccucagcgccagcuuuaccacgcuuaauaaagauaaacacgcgcuaaugacccaacuggccgcaacggaaaaagagaaacaggccgcucuugagcaggucaaagcgcuuaacgcugacaaacagccgcugacgacccggcuggccgccgcggaaaaagagaaacaggccguccucgagcagguuaaggcccuuaacgccgauaaacagucgcugacuauucgccucgccgcugcggagaaagcgcagcaggccgcuguugaccaggcuaaagcgcuuaacgcugacaaacagccgcuggcuacccgacuggccgccgcggaaaaagagaaacaggccguccucgagcagguuaaggcccuuagcgccgauaagcagucgcugacuauucgccucgccgcugcggagaaggcgcagcaggccgcucuugaccaggcuaaagcgcuuaacgcugacaaacagccgcuggcgacccggcuggccgccgcggaaaaagagaaacaggccguccucgagcagguuaaagcccuuaacgccgauaagcagucgcugacuauucgccucgccgcugcggaaaagacgcagcaggcugcccucgaucaggucaaagcccuuaacgccgauaaacaaucgcuguccacccggcuggccgccgcggauaaagcgccgcauggccccgcuaacgacgccgcugcgccaaaaaaugagccaccagagauggcggccauaguggcagccuaucgccugcaggcggauaaagacaacgcccagcuacggaugaaagaagaugaaaucgaacugcugagaacgcagcuuucuguacaguccaaaacgcgcagcggcgagagcgccgccgccaaacucagcgcaucgggagaacagcaggcuuaugcgaucggcgccucgaugggaagcgaggcgcucaacguccuuaccacccgucguacucagggaguuaccgucgacgcaggccuggugcugcagggcaucgaagaugccuuucgcggccagcuucgucucggagagcaggaacguaacaaggcgcuguuugaugugucgcagcagguuuuucagaaccugaauaaaauagagcagaaaaacaucagugccggcaagaaauaucagcaggcguuugcgcgcaaaaaagauguggucuuuaaagagggcgucuacagccgcgucgauuaccuggguaaaggaaaaauaagcgguaaugaccugguuaccguggugaucaaagagaugcugacggacgggacggugaucaacgauauggaagcgaaagaucaggcgcuuacgcaaaagcuggaugccuaucccccgguguuucgcgaaccgcugaagcgucuacagaaccacggcuccgugacgcucgucgucccgccugaaaaggccuauggcaguaaaggauuaccgccaaaaaucccgccaggcgccaccaugguuuauuccgugcggauaguagauagccaacccgagccggcaaaauag

SEQ ID NO: 82 - RNA, 2106 nt, Klebsiella pneumoniae
augaaaauccuguccgugcgucacgccgcccucccggcccugcucuugccgcucauugcggcagcccaggccgcugaugaacaaaccaugguggugaccgccgcgccaaccacgguuucugaacuggauacccccgccgccgucagcguggugaauggggaugagaugcgccaggccgcgccgcgcgucaaucucucugaaucgcugggcgccgugccgggccugcaggugcagaaccggcaaaacuaugcccaggaucugcagcugucgauucgcggcuuuggcucgcgcucaaccuauggcgugcgcggacugcgcaucuauguggauggcauuccggccaccaugcccgacggccaggggcagaccucaaauauugauaucggcagcguugacaccauugaggugcugcgcggccccuucucugcccuguacgguaacucguccggcggggugaucaacgucaccagccagaccggcacccagccgcccaccguggaagccagcagcuacuauggcagcuucggcaccuggcacuacgggaugaaagccacuggcgccguuggcgacggcagccacgcaggcgauguggauuacacggucucaaccaaucgcuucaccacccauggcuaucgcgaucacagcggcgcgcgcaaaaaucuggcgaacgcccggcugggggugcgcaucaacgacgucaguaagcugacucugcugcugaauagcguggauaucaaagccaaugacgccgguggccugaccgccgaugaauggcgcgauaacccgcgccagucgccgcgcggcgaccaguauaauacccgcaagaauacccgacagacccaggccggccugcgcuaugagcgccagcucagugcccaggacgaucucagcguuaugauguacgcuggagaacgugaaaccacucaguuccagucgaucccgcgcgcgccgcagcugaagccgagccaugccggcggggugaucgaccuuacccgucacuaccaggggaucgauacccggcugacccaucgcggagagcugcuggugcccgucacgcucaccgccggucucgacuacgaaaacaugagcgagcggcgcaaaggguaugaaaacuuugugauggucaacggcgcgccgcaguauggcgaacagggcgcgcugcgccguaacgaacgcaaccugauguggaacgucgaccccuaccugcagacccaguggcagcucacugacaaacucucgcucgaugccgggguucgcuacagcucgguaugguucgacucgaacgacuacuacaucaccccaggcaauggcgaugacagcggugaugccagcuaucacaaauggcugcccgcgggcucgcugaaauaugcccugaccgacgcguggaacgucuaucuuuccgccggccgcggcuucgagacgccaaccauuaacgaacucuccuaccgcuccgauaaccagagcggccucaacuucggccugaaacccuccaccaacgacacgguggagaucggcagcaagacgcggaucggcaaugggcuguucaccgccgcccuguuccagaccaauaccgauaaugagauuguggucgacagcagcagcggcgggcgcaccaguuauaaaaacgccggcaagacccgccgucaggggauggagcuggggcuggaucagcaguuuggcgagagcuggcgucugaaggcggccuggaccuggcuggacgcgaccuaucgcacuaacgucugcgacgacgccagcugcaauggcaaucgcauuccggggaucgcgcgcaauaugggcuacgccuccuuuggcuaucagccggagcaagguugguacgccgggagcgauauucgcuauaugagcgauaucauggccaaugacgaaaacaccgccaaagcgcccuccuggacggugguuggccugacgacuggcuauaaauggagcuacggcaggauggauauggaucuguucggucgcaucgacaaccuguucgaccgggaguacgucgggucugucaucguuaacgagucuaacggacguuacuacgagccugccccgggacguaacuacggcaucggccugaaccucgccuggcgcuucgaauaa

SEQ ID NO: 83 - RNA, 2259 nt, Klebsiella pneumoniae
augaaauacacgucucacuucccgcuggggaucgucauuccucugcucgccuguagcgugccgcugcaggcggcagagaacaugaccgaacaaucgacgccugacgagagcgccgccacugccgaaaaucacgaggagacgauggucauaaccgccgccaggcagaaccugcaggcgccgggcgugucgaccaucaccgcagaagagauccgcaaacauccccccgcccgcgaugugucggaguuaauucguacgcagcccgggguaaaccugaccggcaacuccaccagcgggcagcgcggcaacaaccggcaaauugauauccguggcauggggcccgagaauacgcuggugcuggucgaugguaaaccggugaccagccguaacucggugcgguauggcuggcgcggcgaucgugacucccgcggcgauaccaguugggugccagcggagaugaucgaucauaucgaugugauccgcggcccggcggcggcgcgcuaugguaauggcgcgaugggcggggucgucaacaucgugaccaaaccgaccacgcgagaauggcacgggucguggaauaccuauaugaaugcuccgcagcaccguaaagaaggggcgacgaaacguacuaacuuuagccucaaugguccgcugucggacagugucagcuucaaucucugggguaaucugaguaaaacccaggccgaugcacaggauauuaacgccgggcaugaagcggaacguaccgguuccuacgccgguucuuaucccgccggacgugaagggguggugaacaaagauauucacaguaagcugcgcugggaguuugccccgaugcaggcccuggaguuugaggccgguuacagccgccaggguaaucucuaugccggcgacacacaaaacaccaauaccaguacgcuggugaagaguauguacgggaaagagaccaaccgucucuaccggcaaacuuacggcguaacauggaccggcggcugggauaauggcgugaccagcaacagcuaugcccaguacgaacacacccguaacucgcgaauggaugaagggcuggcgggcgguacggaagggaucuucuccaguagcgaguuuucagauaucgaucuggccgauguccugcuacauagugaagugaauauuccguuuacgcugggggucgaucagaaucugacgcugggggcagaauggaaucagcagcggaugaaagauggcguaucgacaacccaggcgcucucuuauggcacuaucgauggcguaucggcuaccggucguagcccguacuccagugccgagaucuucucgcuguuuaccgaagauaauauggcgcuaacggacagcaccaugcugacacccgcucugcgcuucgaucaccacagcaucgucggcaauaacuggagccccucacugaaccugucucaggagcugacggacgacuggacgcugaagcugggcauugcccgugcuuacaaggcgccuaaccucuaccaguugaacccgaacuauauucucuacagcaacggucaaggcuguuacgccaguaguuccgccugcuaucugauggggaauagcgaucugaaagcggagaccagcguuaauaaagagauuggucuugaguacaagcaugauggcuaucaggcggggaucaccugguuccguaacgacuaucacaauaagauugagucaggguaugcggcgguggguaccgccagcaacggcaccaccaauaucuaucagugggaaaacguaccaaaggcguuaguggaaggccuggaaggaacgcugaaucugccggugggggaggcgguuaacuggagcaauaaccugaccuggaugcugcagagcaagaauaagacgaccggcgaccggcugucagugaucccgcaguuuacccugaacucgacuuugagcuggcagguucgugaagaucucucccugcagagcaccuuuaccugguauggccgacagaaaccaaaacgcuucaauuauaagggcgaggcggucagcggcagcgaacuaaacgaagucagcccauacagcauugucggccucagugcgaccugggaugugaacaaaaaucugagcuucaccagcgggauagauaaccuguuugauauucgccacuaccgggcagggaaugcgcaaacgaccggcaacgcgacgacgggagcuuaucuguauggcgcgggugccgagaccuauaacgaaucggggcggaccuucuuuaugagcguuaauacucauuucuga

SEQ ID NO: 84 - RNA, 2286 nt, Klebsiella pneumoniae
auggaaaaaaacgcuucucugccuuucggcaguuucaacucauuggcauuguuuacaggucugugucugggagccucgccggcagcaggcaucgcagcggaaaauucggucaaaaauagugaagagacgcugguaguggaagccgcuccgccuucacucuacucccccggcgcuuccgccgaucccaaguucaauaaaccgcuggucgauaccacccgcaccaucaccgugaucccggaacaggugauuaaagaucagggcgucaccaaccugacugacgcccucaaaaacguucccggcgucggggcguuuuaugccggggagaauggcagcucaaccaccggggaugccaucuuuaugcgcggcguggauaccucuaacagcaucuauguggacggcauucgcgacaucgguagcgugacgcgcgauaccuucaauacccagcagguggaagucaucaaagggcccgccggcacggacuauggccgcagcgcgcccuccggcucgaucaauaugaucagcaagcagccgcgccuugacuccgggaucgacggcucggccagcaucggcagcgccuggucgcgccggggcacucucgaccugaaccaggcguuuagcgacaacgcugcguuccgucugaaccugaugggggaaaaaacgcaugacgcuggucgggaccgcauugaaaacgaacgcuauggcaucgcaccgucgcuggccuucggccuugauaccccaacucgucuguaucugaacuaucugcacguccggcagaacaacaccccggauggcgggaucccuaccgucggccugccgggcuauucggcgccuucgccgaaguaugccgcacucaacuccgccgggaaggucgauaccagcaauuucuauggcaccgacuccgauuacgauaaaucuacuaccgacagcgguacccugcgcuucgaacacgaucugacggagaauaccaccgugcgcaauaccacccgcuggucgcgagugaaacaggaguaucuuuugaccgcggugaugggcggcgcgaacaauaucaccgcccccgauaucaaugacgucaacaccuggagcuggucgcgucugguuaauaccaaagaugucagcaaccguauucugaccaaccagaccaauaucaccucgacuuucaauacuggcucgauaggccaugacgucagcgccggcguggaguuuacccgggaaaaccagaccaacuauggcguuaacgccaggaccgcgccggcggugaaucucuaccauccggugagcaaccugucgauuggcgggcuggacagaaacggggcgaacgccaacggccagaccgauaccuucgggauuuaugccuuugauacgcugacgcugaccgagcggauugagaucaacggcgggcugcgucucgacaauuaccauaccaaauaugacagcgccaccgccugcggcggcagcggacgcggggcuaucgccugcccgcccggacagucgaccggcagcccggucaccacugucgauaccgcuaaauccggcaaucugguuaacuggaaagccggggcgcuguaccgcuuaaccgagcagggcaaugucuacgucaacuacgccaucucacagcagccgccgggaggcagcagcuucgcccuggccgccagcggcagcggcaacagcgcuaaccggaccgacuuuaagccacagaaggcgaaauccagcgagcugggcaccaaguggcaaaucuucgacaaccgucugcugcucagcgcggcguuauuccgcaccgauauugaaaacgaaguggccgccaacgaugacggaaccuggucgcaguacggcaaaaagcgcguggagggguaugaacucuccgcgaccggaaaccugaccccggacuggacgauuaucgccggcuacacucagcagcaugcgacagugacggagggacagaacguugcacaggauggaucuuccgcccuggccuacaccccgaaacaugccuuuacgcuguggacgcaguaucaggccaccagcgaucuguccgucggcggcggugugcgcuaugucggaagccugcgccggggcagcgauggugcagucgguaccccggaucacaccgagggcuacuggguugccgacgccaaacugggcuaucgggucaacagcaaccucgaucugcagcucaauauguauaaccuguuugauaccgauuacguggccuccaucaacaagagcggcuaucgcuaucauccgggcgaaccccggaccuuuaugcugacggcgaacguccauuucuga

SEQ ID NO: 85 - RNA, 2373 nt, Klebsiella pneumoniae
auggcgacuauguacaaaucgacuccgucagcagcaugguguaaaaaacgccugcuggugaccucuuuguuugcagcaauuuaucagacuucugccaucgcagcagauacuuccgccguuagcggcgaggcgguggaugacaccucggaacaaaugaccgucaccgcccccgcgccggugcagaaagccgguagcgaacacagcaucagcgcccgggagcuggagaauaaaggcgcuaacgauuucggcucaaucaugcgcuaugagccgcucaucagcgccaccggggccagcggcggcuccggcaacggcaaaagcggcuucgaccgcggagguuacaccggcuacaacauucgcgguauggagagcaaccgcguaggcaucgacguggacgguaucgcgcaacccaacgccaccggccgcggcuacgucggccgcgccgggcucaacaccuucggcaucggccgcgauuauaucgacccguauauguacggcagcguugauauccaguccggcgccaccucgacggaaacggccaacagcgcuaucggggggaaugucuccuuccgcccgaaaucagcggaugauuaccugcgcccgggcaagaccagcgccuucggcuaccgcagcgguuacgacucugcggaucgcagcuggcacaacggggugaccgucgccggcggcgaugaguuccugcgcgggauuuuggucuauagccgccgugacggccaggaaacugaaaacaacagcggcaccgucgacgccuacccggcgaacuggcacuccgaugcuuuucuggccuccgggaucuggcagccuaacgaugagcacaagcugaccagcaccuucgacuauuaccauaaaaccaaccacacccacuacgauaccugggacuccagcggcaacagcaccaucggcaccgccaaccagaccagccagacccggcgcuggggccugagccugaaggaugacuggacgccgaugaacgacuaccucgacagcgucuccacaaaaaucuacuaccagcauaccgaagcccaugacuggacuuauaugccggacagcgucacccgcaaaaugcagacggugaacucuaacuacgauaccgacaccuggggccugcagaccgcgcuggcgaaaacccugggccgccacgaucugagcgccgguuucaacgccagcaccagcaaaacccagcggccguucagccagucgccgauccccagcguuuacagcgagaucaugcagccggaggcagacagccgcagcuacacccucggcggcuuuguccaggauaagaucaacuucgaucucgacagccacaacuucgccguuauucccggcgugcgcguggugcaucaaucgacuaagccggaaaaucuguccgaucucgccgccaacagcagcgugcugagcgaaucgucgguggcgaaucuguacggcaaaaacagcgauacccagguucugccgucguugaccuuccaguacgaccucaccccgcgccugaugaccuaccugcaguaccagcgcggggcgcaguuccccaacgccagccagcuguauggcuccuggaaccucggcuccagcuacgccggcagccagcaguaugcccugaucggcaauaccgaucugaagacggaaaccagcgauaaucucgagugggggcugaaaggggaaguuaccgaaggcaucacccugcgcacggcgcuguucuacaacagcuauaagaacuuuaucgccuauacccgcuauacccgcgccaacaauccgggccaguucacgaaugugccgucgaacaucuacaccauuuaucaggcggaaaaccgcgauaaagccuauaucuacggcggugagauuagcaccaaauuuaacuuuggcaccugguuugagcagguggacggccugagcgccacccucgcccucggcuauagcgaagggaaaucgaaauccagcuacagcggcgauaaauacgucgaccucgacagcguggcgccaaugaaagccaucgucggcguggcgugggacgauccggcgaaacgcuacggcaccgcccugacggcgaccuuugucaaagggaaacaggcgaccgccaccaaccgcgaaagcuacagcaacagcggauccgccaucaccgaugccagcagcgacuauaugcgcgugccgggcuacggcaugcuggacuggaccgcguacuggcagguggcgaaaaacgugcgccucaauggcggggucuacaaccucaccgaucguaaauacugggauuaccugagcagccgcaauaucgagaccggcaccaaccaggacgccaacgauaaagcgcuggcggugaugccgggccgcaccuggcagcugggcgucaacgucgacuucuga

SEQ ID NO: 86 - RNA, 2430 nt, Klebsiella pneumoniae
auggcgaugaaaaaguugcucauagcgucgcugcuguuuagcagcgcgacuguauacggugcugaaggguucguggugaaggacauucauuucgaaggcuugcagcgugucgcuguuggugcggcccuccucaguaugccagugcguccuggcgauacggugaccgacgaugauaucaguaacacuauucgcgcgcuguuugccacuggcaacuucgaggacguccgcguccugcgcgauggugauacccugcugguucaggugaaagagcguccgacgaucgccagcaucacuuucuccggcaacaagucggugaaagaugacaugcucaagcagaaccuugaggccucaggcguucgggugggcgagucgcuugaccgcacgaccaucgcggauaucgagaagggucuugaagacuucuacuacagcgucgguaaauacagcgccagcgucaaagcagucguuacgccgcugccgcguaaccgugucgauuugaagcuggucuuccaggaaggcgucuccgcaaaaauucaacagaucaacaucgucggcaaccaugcguuuucgaccgaugagcugaucucccacuuccagcugcgcgaugaggugccgugguggaacguggucggcgaccguaaauaccagaagcagaagcuagcgggcgaccuugaaacccugcgcagcuacuaccuggaucgcggcuaugcccguuucaacaucgauucuacccaggucagccugacgccggauaagaaagggaucuacaucaccgucaacaucaccgaaggcgaucaguacaaguuuuccggagugcaggugacgggcaaccucgcuggccauuccgcggaaaucgaagcgcugacuaaaguugagccaggcgaacuguacaacggcgcgaaagugaccaagauggaaaacgacaucaagaaacuguugggucguuaugguuacgccuauccgcgcgugcagucgcagccggagaucaacgacagcgauaaaaccguuaagcugcacguuaacgucgacgcaggcaaccguuauuacgugcguaaaauucgcuucgaaggcaacgacaccucuaaagaugccguacugcgccgcgaaaugcgccagauggaaggcgcauggcugggcagcgaccucgucgaucaggguaaagaccgucucaaucguuuagguuucuuugaaacgguggauacugauacccagcgcgugccgggcagcccggaccaggucgacguugucuacaaggugaaagagcguaacaccgguagcuucaacuucgguaucggcuacggcaccgagagcggcgucagcuuccaggcgggcguucagcaggauaacugguuagguacuggcuaugcugucgggaucaacgguaccaaaaacgacuaccagaccuauaccgagcugucggugaccaacccguacuucaccguagacgguguaagccucggcggucgugucuucuauaaugacuuugaugcgaacgaugcggaucugucugacuauaccaacaaaagcuaugguacagacauuacgcugggcuucccggucaacgaauacaacacgcugcgcgccggcgucgguuaugugcauaacucccuguccaauaugcagccgcagguggcaauguggcguuaccuuaacucgaugggccaguauccggacaacaccaacgaccggaacucguucagugcgaaugacuucaccuucaacuacgguuggaccuauaacaagcuugaccgcggcuucuucccaacggaagguucgcgcgucaaccugaacgguaaggugaccauuccgggcucagacaacgaguacuacaaagcgacgcuggauaccgcgaccuacgugccgaucgacaacgaucaucaguggguaguacugggucguacgcgcuuugguuauggcgaugguaucggcggcaaagagaugccguucuaugagaacuucuaugccggugguuccagcaccgugcguggcuuccagucgaacaccauugguccgaaggcgguguacuucccggcaagcagucgucaugaugaugacgauaguuacgauaaugaauguaagagcaccgaauccgcaccguguaaauccgaugaugcggugggcgguaacgcgauggcgguggccagccuugagcugauuaccccgacgccguuuauuagugacaaauaugcgaacucgguccguacuuccgucuucugggauauggguaccguaugggauacucacugggauucgagcgcguacgcugguuauccggauuacagcgauccgagcaacauccguaugucugcggguauugccgugcaguggaugucgccguuggggccguuggucuucuccuacgcccaaccguucaaaaaguacgauggagacaaagccgaacaguuccaguuuaacauugguaaaaccugguaa

SEQ ID NO: 87 - RNA, 2691 nt, Klebsiella pneumoniae
augacagaugugacuauuaaagcgcuggccucagagauucagaccucuguggaucgccugauacagcaauuugcugacgcaggcauccgcaaaucggcugaugauucugugaccucgcaagagaaacaaacuuuguugacgcaccugaaccgugaacacggcucggcgccagacaagcugacguuacagcguaagacgcgcaguacguuaaauauuccagguaccgguggaaagaguaaaucgguacaaaucgaaguccgcaagaaacgcaccuuugugaaacgcgauccgcaagaggcugaacgccuggccgcggaagagcaggcgcagcgugaagcggaagagcaggcccgucgugaagcugaagaagcagcgaaacgcgaggcgcaauuaaaagcugaacgugaggccgcagaacaagcuaaacgugaagucgcugauaaagcgaaacgugaagcugcggaaaaagacaaagugagcaaucaacauaccgacgaaaugaccaaaaccgcccaggcugaaaagauccgucgcgagaacgaagccgcggaauugaagcgcaaaucggaagaagaagcacgccgcaaacuugaagaagaagcgcgccguguagcggaagaagcacgccguauggcugaagaaaacgaaaaaaauuggucugaaaccucagacagcccggaagauagcagcgacuaucacgucaccacaucacagcaugcucgucaggcugaagaugauaacgaucgugaagucgaaggcggucgcggccguagccguagcagcaaagcggcucguccggcgaagaaaggcaacaaacacgcugaaucgaaagcugaucgugaagaagcccgcgcggccgugcgcggcgguaaaggcgguaagcaccguaaagguuccgcucugcagcagggcuuccagaagccagcgcaggccguuaaccgugacgucguaaucggcgaaaccaucaccguuggcgaacuggcuaacaagauggcggugaaagguucucaggucaucaaagcgaugaugaagcugggcgccauggcgaccaucaaccaggucaucgaccaggaaaccgcacagcugguugccgaagagaugggccacaaaguuauccugcgucgugaaaacgaacuggaagaagccguaaugagcgaccgugacaccggcgcggcggcugaaccgcgcgcaccggucgugaccauuaugggucacguugaccacgguaaaaccucgcugcuggacuacauucguucuaccaagguugccuccggcgaagcgggugguauuacccagcacaucggugcuuaccacgucgaaaccgacaacggcaugaucaccuuccuggauaccccgggccacgccgcguuuaccuccaugcgugcucguggcgcgcaggcgacggauaucgugguucuggugguggcggcagacgacggcgugaugccgcagacuaucgaagcuauccagcacgcuaaagcggcgcagguaccggugguaguggcggugaacaagaucgauaagccagaagccgauccggaucgcgugaagaacgaacugucccaguacggcauccugccggaagaguggggcggcgagagccaguucguccacguuuccgcgaaagcggguaccggcaucgacgaccugcuggacgcgauccugcugcaggcugaaguucuugagcugaaagcgguccgcaacgguauggcgagcggcgcggucaucgaauccuuccuugauaaaggucgugguccgguagcuaccguucugguucgcgaagguacucugcacaagggcgacauuguucugugcggcuucgaauauggccgugugcgcgcgaugcgugacgaacugggucgcgaagugcuggaagcggguccguccauuccgguggaaauccucggccuguccggugugccggcugccggugaugaagugaccguagugcgugacgagaaaaaagcgcgugaaguggcgcuguaucgucagggcaaauuccgugaaguuaagcuggcgcgucagcagaaaucuaaacuggaaaacauguucgcuaacaugaccgaaggcgaaguucacgaagugaacaucguacugaaagcggacguacaggguucugucgaagcgauuuccgauuccuuacugaaacugucuaccgacgaagugaaagugaagaucaucgguuccggcguaggugguaucaccgaaaccgacgcuacccuggcagcagcauccaacgcgauucugguuggcuucaacguucgugccgaugccucugcgcguaaaguuaucgaagcggaaagccuggaucugcguuacuacuccgucaucuauaaccugaucgacgaagugaaagcggcgaugagcggcaugcugucuccggaacugaaacagcagaucaucggucuggcugaagugcgugaugucuucaaaucgccgaaauucggcgccaucgcgggcuguaugguuaccgaagggacgaucaaacgucacaacccaauccgcguucugcgugacaacgugguuaucuaugaaggcgagcuggaaucccugcgccgcuucaaagaugacguuaacgaaguccguaacggcauggaaugugguaucggcgugaagaacuacaacgacguucgcguuggcgauaugaucgaaguguucgaaaucaucgaaauccagcguagcaucgauuaa

SEQ ID NO: 88 - RNA, 3234 nt, Klebsiella pneumoniae
augaaaagaauguuaaucaacgcaacucagcaggaagaguugcgcgucgcccuuguugaugggcagcgccuguacgaccuggauaucgaaagccccgggcacgaacagaaaaaagcgaacaucuacaaaggcaaaaucacccgcauugaacccagccuugaagccgcguuuguugauuacggcgccgagcgucaugguuuccucccccucaaagaaaucgcccgcgaauacuuccccgccaacuacaaugcgcauggucguccuaauaucaaagacguacugcgggaaggucaggaaguuaucgugcagauugauaaagaagaacgcggcaacaaaggcgcugcgcucaccaccuuuaucagccucgcgggcagcuaucugguacugaugccgaacaacccgcgcgccgggggaauuucccgccguaucgagggcgacgaccguaccgaacugaaagaagcgcuggcgagccuggagcuuccggacggcaugggccugaucguucgcaccgcuggcgucggcaaauccgccgaagcccugcagugggaccugagcuuccgccugaagcacugggaagcgauucagaaagccgcggaaagccguccggcgccguuccugauccaccaggaaagcaacgucauuguccgcgccuuccgugacuaccugcgccaggacaucggcgaaauccugaucgauaacccgaaagugcuugagcuggcgcgccagcauaucgccgcgcugggucguccggauuucagcagcaaaauaaaacuguacaccggugaaaucccgcuguucagccauuaucagaucgaaucgcaaauugaguccgccuuccagcgcgaagugcgccugccuuccggcgggucuaucguuaucgauagcaccgaagcgcugaccgcgaucgauaucaacuccgcccgcgccacccgcggcggcgauaucgaagagacagccuucaauaccaaccucgaagcggcugacgaaauugcccgccagcugcgucugcgcgaccucggcggccugaucguuaucgacuucaucgauaugaccccgguucgccaccagcgcgccguggagaaucgucugcgcgaagccguccgucaggaccgugcgcgcauucagaucagccauauuucgcgcuucggccugcuggagaugucccgucagcgccugagcccgucgcugggcgaguccagccaccacgucugcccgcgcugcuccggcaccggcaccgugcgugauaacgaaucgcugucgcucucuauucugcgucugaucgaagaagaagcgcugaaagagaauaccaaagaaguccacgccauuguuccgguaccgaucgccuccuaucugcugaacgaaaaacgugccgcagugagcgcuaucgaaucccgucagggcgaugugcgcguuauuaucgugccaaacgacgaaaugcaaacgccgcacuacuccguccugcgcgugcgcaaaggugaagaaaccucaacgcugagcuaucugcugccgaagcugcaugaagaagaaauggcgcugccaggcgacgaugagccggcggagcggaaacguccggaacagccggcccuggccgcuuuugucaugccagaugcgccgccagccccgaugcucgaagagccugccgccgcgccugucgccgcagcggcaccggucgcggccgccgcaccggcgcagccuggccugcucucacgcuucuucagcgcgcugaagaauaucuucucuggcgccgaagaggccaaaccggcugaaguucaggucgagaagaaagcggaagaaaaaccggagcgucagcaggagcgucguaaaccgcgcgccaacaaccgccgcgaccgcaacgaccgccgugauaaccgcgacaaucgugacaaccgcgauaaccgugacaaucgcgacacccgugcggacaaugccgagggccgugaaccgcgcgaaucgcgugaagagaaccgucgcaaccgucgcgagaagccgucgcagaacguggaagcccgugauguucgccaaaccucaggcgacgacgcggagaaagcgaaaucccgugacgagcagcagccgcgccgcgaacgcacccgccgccgcagugacgacaaacgucaggcgcagcaggaagccaaagcgcagacucgcgaagagccgguugugcaggagacggagcaggaagagcguguacaaacucugccgcgucguaaaccgcgccagcuggcacagaaagugcgcguugaguccgcugucgucgagccaguugccgagaucgugccagaagccguaguggcugaaguuaucgcuccgcacagcgagccggugaaagccgagcugccggcagggguggagagcguggcggaccaggacgaaaauggcgaaucccgugaagcgaacgguaugccgcgucgcucacgucgcuccccgcgucaccugcgcgucagcggucagcgucgucgucgcuaucgugacgaacgcuauccgacccagucgccuaugccgcugaccguagccugcgcaucgccggagauggcuuccgguaaagucuggauccgcuacccggugguucguccgcaggaucagcagccggaagagguucagguucaggacgccagcgucgcgaaaacugucgaggccguagcggccccggucgccgucguugaaaccguuaccgcugcgccggucaccgucgagccggcuaccauggaaccaguaaccgcugagccgguagucgucgagccgguagcggccgccgagccgcuggucguugaugcugcggaaguugucgcgccagcagccgucgagccagcgccucaggagccggucaccgaagcaccggcugucgaagcgccucaggcuaucgcgccagugacgcucgacgccgagccgguggugguagaaccugaagcgguggaaacgacgccugucguugcagcgccaguggaaacuaucgccccggucgcagaaaccguggagcaagcgccagugaccgaagcggccccugccgaaccggucaaagccgagcccccggugagcaagccggucguaguggcgggucaucgccaugccaccgcgccaaugacccgugcgccagcuccggacuaugucccggaagcaccgcgucauagcaccugggugcgcccgccguucgccuuugaagguaaaggcgccgccgguggucauagcgcgacccauaaagccaccgcugaaccgacucgcccacagcccgucgaguaa

SEQ ID NO: 89 - RNA, 3480 nt, Klebsiella pneumoniae
augcgcaagcucucacuaaguuuacucacgcugucccucggcguugcgcugcugccguuagcgcaggcggcgacgacgccugcccaggagcaucugcuggagcagguccgccucggcgaggccagcaaucgugaagaccuggugcgccagucgcuguaccgucuggagcugauugaucccaacaacccggagcugauugccgcgcggaugcgcuaucugcugcgucagggggaugccgccggggcgcaaaaagagcuggaacgacugacgaagcaggcgccggacuccccggagcugaaggcgucgcgcaaugagaugaaaagcaacaccggcgagggccgccaggcgcugcagcaggcgcgacugcugggcguggccgggaaggucgaugaagccaucgccgccuaugaaaaacuguacggcggggugccggaugacguugacgucgccauugaguacuggacgcugguggcgcgccugccggcccgccauagcgaaggcgucagccaguugaaaaaacugaacgccagcgcgccgggcaacgucagccugcugacuucgcuggcgaagcagauguucgccgauaacaaaccgcaggagggguucgccuaucuggcggagauggcccgaucggccucgggacgcgguaucgccgccgauaugugguucagugaggugaaaagcaugccggugaguaaggccagcgugcaggcguugcagcaauuucuucugcaguuucccaccggcucgguggcggcgaacgcccgcguucugcucgaccaacagcaggcgcagcugcaggauccgacuuuccgcgcccgcucggaagggcuggcggcggucaaguccgggaauaccacgcaggcggucgcggaucugcagaaagccguucaggccgacagccgcgacagcgacgcggugggcgcucucggccaggccuauucccagcgcggcgaccgcgcgcgggcaguggcgcagcucaguaaagcgauugcuauggacccugacagcccgaaccgcggcaagugggacagccugcugcaaacuaaccgcuacuggcugcugauaaagcagggggauaacgcccugaaagccggccagcuuucgcaggcgcagaacuauuaugcccaggcgcagcgggucgaucgcaccgacagcuaugccgugcuggggcugggggacgucgcggcggcgcgcaaagaggcggcggcggcggagcgcuauuaccagcaggcguugcgccuggaucgcggcaauaaccuggcggugcgcggccuggccaaccucuaucgcgccgaaucgccggagaaagccagcgccuggaucgccggccucccucccgcucagcggcggagcaucgaugauauugagcgcagccugacuaacgaccggcuggagaaacaggcgcaggcucuggagagccagggcaacugggcgcaggcggcggaaguucagcgucggcgccuggcgcuggauccggacagcgucuggauaaccuaccgucuggcgcgggaucuggucagcgccggcgaacgccaggaggccgacgcgcugaugcggacgauggucaaccgccagccgcaggacgccgaacgggucuacgccucgggacucuaccugucggggaacgaccaggacgaucuggcucuggcgcaaaucgccgcucugccgcgcagcgcguggacggauaacauucgugagcucgaagcgcguuugcaaagcgaccgggugcugcgccaggccaaccagcugcgcgacagcgguaacgaagcgcaggcgaucgcccuuauccgacagcagcccgccucggugcgcuaugaccugacgcucgccgacugggcgcagcagcgcggcgacagccagacggcgauugccaacuaucagcgggugcugcgccaggaggccgacaacggcgaugcgcgccucggccuugcggaagucuaccuggccgagggcgauaaaccggccgcccgggcgcaggucaugcagcugaaaggcgcagagaccgaauccaugaacaugcagcggcggguggcgcuggcgcgagcuggccuuggcgauaccgcugacgcgcaacggauuuuuaaucagauugugccgcaggcgaaggcgcagccgcccucgauggagagcgcgcuggugcugcgcgaugccgcgcgcuuugccacccagagcggggcgccgcagcaggcgcugacgcacuaccgggaagcuaugguggccuccggcauuacccccgcgcagccgcaggauaacgauacuuuuacgcggcugacgcgcaacgacagccaugaugacuggcugaagcgcgggauccgcagcgaugccgccgaccuuuaucgucagcaggaucugaacgucacccuggaacaugacuucugggguuccagcggcaccggcggcuauuccgaccugaaggcgcauaccaccaugcugcagauggaugcuccgcuggcggauggccggauguucuuccgcaccgaccuggucaauauggaugccggcagcuuuuccacccacagcgacgggagcuacucgcccagcuggggcaccugcggggagaucgccuguaccagcggcaguaaaaaucagaccgacagcggggccagcguggcggucggcuggaagaaugacaccuggagcggggauaucggcaccacgccgaugggcuucaaugucgucgauguggugggggggcugagcuacagcagcgacgucgggccggugggguacacggucaacguccaccggcggccuaucuccagcucgcugcucuccuuuggcgggcagaaggacagcagcagccauaccggcgccaccuggggcggcguccgcgccgacggcggcggccugagccugagcuacgaucgcggggaggcucacggcaucugguccucgcugggcgccgacucgcugaccgguaaaaacguggcggauaacuggcgcgugcgcuggaugaccggguacuacuacaaggucaucaacgagaauaaucgucgcgucaccgucggccucaacaauaugaucuggcacuacgacaaagaucucagcggcuacacccucggccagggcggcuauuacagcccacaggaguaucucucguucgccgugccggugaccuggcgucagcgcaccgagaacugguccugggagcucggcgggucggugucauggucccauucgcgcacccagacgcaagcccgcuauccgcugcugaaccugaucccguccgacuaccggcagcgcgccagcgagcugacggaggaggggagcagcagccauggauucgguuacaccgccagagcgcugguggagcggcgggugaccagcaacugguucgucggcgccgcggucgauauucagcaggcgaaggauuacaccccgagccaugcgcugcuuuacguccgcuacucggcggccggcuggcagggggaucuggauaugccgccccagccgcuggugcccuacgccgacugguag

SEQ ID NO: 90 - RNA, 4236 nt, Klebsiella pneumoniae
augagccaggaauacaccgaagacaaagaagucaaacuaaccaaacucagcagcgggcgccgacuccuugaggcgaugcucauccuuugcucccucuucgccaucuggcugauggcggcacuacugagcuuuaaccccucggaccccagcuggucgcaaacggcauggcaugagccuauucauaauuuaggcggcgcccccggcgcguggcuugccgauacccucuuuuucauuuuuggcgucauggccuacaccaucccggugaucaucaucggcggaugcugguuugccuggcggcaucaggaaaacgacgaauacauugauuauuuugccguuucccuucgccucaucggugcguuagcccugauccugaccuccuguggucuggcggcgauuaacgccgaugauaucugguacuucgccuccggcggggugaucggcagccugcugagcaccacgcugcaaccccugcugcacagcagcggcggcaccaucgcccuguuguguaucugggcggccgggcugacgcuguucaccggcuggucgugggucagcauugcggaaaagcugggcggcggcauccuguccguucucaccuuugccagcaaccguacccgucgggaugauaccugggucgaugaaggcgaauaugaagacgacgaggaagaguacgacgacgaagaggcggccaggccgcaggaaucgcgucgcgcccguaucuuacgcagcgcgcuggcgcggcguaagcgucuggccgagaaguuuaccaacccuauggggcguaaaaccgacgcugcgcuuuucuccggcaaacggauggaugacggcgaagagguggugcaauacagcgccagcggggcgccuguugccgccgacgauguacuguuuuccggcgccagcgccgcgcgucccgcagaggaugaugugcuguucuccggcgccagcgccgugcgcccgggcgauuucgacccuuacgauccguuguugaauggccacaguaucgcugagccgguaagcgcagcggcggcggcuacagccgcgccgcaggcgugggcagaaucaccggugggccaucacggcgcugcgccagcuuaucagccggaagccagcuauccgccgcagcaggccuaucagccugaacccgcuccguuccagcaggccuaucagccugaacccgcuccguuccagcaggcugcuuaucagccgccagcggggcaaaccgcaccgcaggcguaucagccugagccagcgccguaucaacagccgguuuacgauccgcgugccggucaaccugcgccgcaggccuaucagccugagccagcgccguaucagcagccggcuuacgauccguaugccggucaaccugcgccgcaggccuaucagccugaaccugcgccguaucagcagccggcuuacgauccgcaugccggucaaccugcaccgcaggccuaucagccugagccagcgccguaucagcagccggcuuacgaucccuaugccggucaaccugcgccgcaggccuaucagccggagccagcgccguaucagcagccaacuuacgaucccuaugccggucagccugcgccucagaccuaucagcagccggcuuacgauccgaaugccggucagcccgcgccgcagccguaucagccggagccagcggcguaucagccgcaaagcgcgccaguucccccaccggagccagagcccgaggucgugcaggaggaagugaaacguccgccgcucuauuauuucgaggaaguggaagagaagcgggcgcgcgaacgcgagcuguuggccuccugguaucagccaauuccugagccggaaaguccgauugccacuaaaccgcugacgccgccgaccacugcguccaaaccgccaguggagacaaccguagucucugcgguagcggcuggggugcaucaggcuaccgccgccagcggcggcgcggcggcagcaaccucguccacugccgcauccgcugcggcuacgccauuguucagcccggcguccagcggcccaaggguucaggugaaagagggcaucgguccaaaacuaccgcggcccaaucgcgugcguguuccuacgcgucgggaacuggccuccuacggcaucaagcuaccgucgcagcgggaggcggaacagcgcgcgcggcaggcggagcgcgauccgcauuaugaugaugagcugcucucggaugaggaagcggaugcuauggagcaggaugaacuggcucgccaguucgccgccacccagcagcagcgcuacggucaucgcugggaagacgauaacgcgacugaugacgaugaggccgacgccgcggcggaagcggagcuggcgcgucaguuugccgcuacccagcagcagcgguacgcuaccgagcagccgccgggcgccaacccguucucgccggcagauuaugaauucucgccgaugaaaacguuggucaaugacggcccgagcgaaccgcuguuuacgccgacgccggaaguccagccgcagcagccggcccagcgcuaucaacaaccggcggccgcuccgcagcaggguuaucaaccugcgcagcaucagccgauacaccaucagccugugccgccacagccgcaguccuauccgacugcgucgcagcccguacagccgcaacaaccgguugccccgcaggggcaucagccugccgccccugcgccgcaggagagccugauccacccgcugcugaugcgcaauggcgauagucgaccgcugcaaaagccgaccacgccacugccgucgcuggaucugcuuaccccgccgccgagugaagucgagccgguggauaccuuugcucucgagcagauggcacgccugguggaagcgcgacucgcugauuuccgcauuaaagcggauguggugaacuacucaccggggccggugaucacccgcuucgaacugaaucuggcgccuggcguuaaggccgcacggaucucuaaccugucacgggaccuggcgcgaucgcugucaacggucgccgugcgcgugguggaggugaucccgggcaaaccguaugucgggcuugagcugccgaauaaaaaacgccagaccgucuaccugcgugaagugcucgacaacgccaaguuccgugauaacccaucuccgcucaccgugguguuggguaaagacaucgcuggcgauccgguaguagccgaucuggcgaaaaugccgcaucugcugguggccgguaccaccgguuccgguaagucuguuggcgucaacgccaugauccucagcaugcucuacaaggcgcagccggaagaugugcguuucauuaugaucgacccgaaaaugcucgagcugucggucuacgaaggaauuccgcaccugcugacggaaguggucaccgacaugaaagacgccgccaaugcgcugcgcuggagcgucaaugagauggagcgccgcuacaagcugaugucggcgcugggcgugcguaaccucgcgggcuacaacgagaagaucgccgaagccgcgcgcaugggacguccgaucccggauccguacuggaagccuggcgacagcauggacgccguacauccggugcuggaaaaacugccguacaucguggugcugguggaugaauucgccgaucugaugaugaccgucggcaaaaagguggaagagcugaucgcucgccuggcgcagaaagcgcgcgcggcggggauccaccuggugcuggcgacacagcguccgucgguagauguuauuaccggccugauuaaggccaacaucccgacgcgcaucgccuuuaccgugucgaguaaaauugacucacguaccauucucgaucagggcggcgcggaaucgcugcuggguaugggggauaugcuuuacuccgggccgaacucuaccacgccggugcguguccacggggcguuugugcgcgaccaggaaguccacgccgugguucaggacuggaaagcccgcggucgcccgcaauauguggauggcauuaccuccgacagcgaaagcgaaggcggcgguggcggcuucgacggcggggaagaguuggauccguuguucgaucaggcagucaacuuugugaccgagaagcgcaaagcgucgauuuccgggguucagcgucaguuccgcaucggcuauaaccgugccgcgcguauuaucgaacagauggaagcgcaggguaucgucagcgagcagggccauaacgguaaccgcgaagugcuggcgccgccgcccuuugaauga

SEQ ID NO: 91 - protein, 742 aa, Klebsiella pneumoniae
MNNRIKSLALLVNLGIYGVAFPLSAAETATDDKNSAAEETMVVTAAEQNLQAPGVSTITADEIRKRPPARDVSEIIRTMPGVNLTGNSTSGQRGNNRQIDIRGMGPENTLILIDGKPVTSRNSVRLGWRGERDTRGDTSWVPPEMIERIEVIRGPAAARYGNGAAGGVVNIITKKTGDEWHGSWNTYMNAPEHKDEGSTKRTNFSLSGPLGGDFSFRLFGNLDKTQADAWDINQGHQSERTGIYADTLPAGREGVKNKNIDGLVRWEFAPMQSLEFEAGYSRQGNLYAGDTQNTNSNDLVKENYGKETNRLYRNTYSVTWNGAWDNGVTTSNWAQYERTRNSRKGEGLAGGTEGIFNSNQFTDIDLADVMLHSEVSIPFDYLVNQNLTLGSEWNQQRMKDNASNTQALSGGSIPGYDSTGRSPYSQAEIFSLFAENNMELTDTTMLTPALRFDHHSIVGNNWSPSLNLSQGLWDDFTLKMGIARAYKAPSLYQTNPNYILYSKGQGCYASKDGCYLQGNDDLKAETSINKEIGLEFKRDGWLAGVTWFRNDYRNKIEAGYAPVYQNNKGTDLYQWENVPKAVVEGLEGTLNVPVSETVNWTNNITYMLQSKNKKTGDRLSIIPEYTLNSTLSWQVRDDVSLQSTFTWYGKQEPKKYNYKGQPVTGSEKNEVSPYSILGLSATWDVTKYVSLTGGVDNVFDKRHWRAGNAQTTGGATGTMYGAGAETYNESGRTWYLSVNTHF

SEQ ID NO: 92 - protein, 356 aa, Klebsiella pneumoniae
MKKTAIAIAVALAGFATVAQAAPKDNTWYAGGKLGWSQYHDTGFYGNGFQNNNGPTRNDQLGAGAFGGYQVNPYLGFEMGYDWLGRMAYKGSVDNGAFKAQGVQLTAKLGYPITDDLDIYTRLGGMVWRADSKGNYASTGVSRSEHDTGVSPVFAGGVEWAVTRDIATRLEYQWVNNIGDAGTVGTRPDNGMLSLGVSYRFGQEDAAPVVAPAPAPAPEVATKHFTLKSDVLFNFNKATLKPEGQQALDQLYTQLSNMDPKDGSAVVLGYTDRIGSEAYNQQLSEKRAQSVVDYLVAKGIPAGKISARGMGESNPVTGNTCDNVKARAALIDCLAPDRRVEIEVKGYKEVVTQPAA

SEQ ID NO: 93 - protein, 245 aa, Klebsiella pneumoniae
MDGWQRAFVLHSRPWSETSLMLDVFTEESGRVRLVAKGARSKRSNLKGALQPFTPLLVRFGGRGEVKTLRSAEAVSLALPLSGITLYSGLYVNELISRVLEHETRFSELFFDYLHCIQALAGASGSPEPALRRFELALLGHLGYGVDFLHCAGSGEPVDDTMTYRYREEKGFIASLVIDNNTFTGHHLKALASREFPDVDTLRAAKRFTRIALKPYLGGKPLKSRELFRQFMPARKARADNTNND

SEQ ID NO: 94 - protein, 1649 aa, Klebsiella pneumoniae
MKPFRLAALSLALLTAFSLTGCDDSGTPQASAPAPAADSNPGATAKPDRAQLAALAEKSQGKALTLLDASEVQLDGAATLVLTFSVPLQPDQDFSRSVHLVDKKSGKVDGAWELAPNLKELRLRHLEPKRELIVSVDPTLTALNKATLDKPFEKTLTTRDIAPSVGFASRGSLLPGNVVAGLPVMALNVDNVDVNFFRIKPESLSAFVSQWEYRNSLSNWESDELLKMADLVYSGRFDLNPARNTREKLLLPLSDIKPLQQPGVYVAVMNPAGRYSYSNAATLFTLSDIGVSAHRYHNRLDVFTQSLENGAAQSGIEVQLLNAKGQTLAEAKSDSQGHVTLQTDKEAALLLARKEGQTTLLDLKLPALDLAEFSIAGAPGFSKQFFMFGPRDLYRPGETVILNALLRDSDGKPLAEQPVKLEVVQPDGQVIRSVMSKPVNGLYQFTYPLDSGAATGMWHIRASAGDNQPREWDFHVEDFMPERMALNLTPQAAPVAPDADVTFGVSGAYLYGAPASGNQLQGKLFLRPLRDAVAALPGFQFGDIAEENLSRSLDEVQLTLDEKGHGEVTTSSQWQDSHSPLQVVLQASLLESGGRPVTRTVKQPIWPAEALPGIRPQFTLKDVYDYRTDTTVKQPVVDENSNAAFDIVYADVKGEKKAISGLQVRLIRERRDYYWNWSDSEGWQSQFDQKDLQEGEESLDLQAGQIGKVSFPVEWGSYRLEVKGPDDVVSSVRFWAGYSWQDNSEGAGAARPDRVTMKLDKPSYKPGDTIRLHIAAPAAGKGYAMVESSEGPLWWQEIDVPAEGMDLSIPVDKTWNRHDLYLSTLVVRPGDKSRSATPKRAVGLLHLPLGDENRRLTLALEAPDKMRPNQPLTVKVKASVKEGEAPKQVNVLLSAVDSGVLNITDYATPDPWNAFFGQKRYGADIYDIYGQVIEGQGRVASLRFGGDGDELKRGGKPPVNHVTIVAQQAQPVVLNDQGEGTVTLPIGDFNGELRVMAQAWTADDFGSSEDKVVVAAPVIAELNTPRFLASGDTTRLALDLSNLTDKPQTLQVHLTASGLVTLSEGQLPPVQLAPGARSTLFIPVSALAGFGDGQVNATISGLSLPGETFAPLQKQWKIGVRPAYPAQTVNSGAVLQPGESWQPPAAQSQGFAPQTLQGQLLLSGKPPLNLARYIRELKAYPYGCLEQTASGLFPSLYTSAAQLKALGISGDSDEKRRAAIDVGISRLLQMQLENGGFALWDREGPEEYWLTAYAMDFLVRASEQGYSVPVNAINKGNERLLRYLQEPGLMTVRYSDDAQASRFAAQAYAALVLARQQKAPLGALREIWSRHDQARSGLPLLQLGIALKTMGDAPRGDAALKLAVATPRQDENRWLGDYGSPLRDNALKLALLEENKLLPEVQTQLLSTLSEEAYGQRWLSTQETNALFLAGRTLADLPGSWQAQTSLQAEPLAGDKAQTRNLDGDRLAALQVSNTGSQPLWLRLDSSGYPQSAPQPGGNVLGIERTIFDTQGQQKSLSSLRSGELVLVKLEVTAKRNVPDALVVDLLPAGLELENQNLANSSASLQENGDAVQNLLNQMQQADIQHIEFRDDRFVAAVAVNEGQPVTLVYLARAVTPGTYQVPQPQVESMYAPQWRATGAASGPLTVTP

SEQ ID NO: 95 - DNA, 2229 bp, Klebsiella pneumoniae
atgaataacaggatcaaatccctggccttgctggtcaatctgggaatttacggggttgcttttccgttaagcgcagcggaaaccgccaccgacgataaaaacagcgccgctgaagagaccatggtggtcaccgccgccgagcagaacctgcaggcgccgggcgtctccaccatcaccgccgatgagatccgcaaacgccccccggcgcgcgacgtctcggagatcattcgcaccatgccgggggtcaacctgaccggcaactccaccagcggccagcgcggcaacaaccgccagattgatatccgcggcatgggcccggaaaataccctgatcctgatcgacggcaagccggtcaccagccgcaactccgtgcgccttggctggcgcggcgagcgcgacacccgcggcgataccagctgggtgccgccggagatgatcgaacgtatcgaagtgattcgcggcccggccgccgcccgctacggcaacggcgccgccggcggcgtggtgaatatcatcaccaaaaaaaccggcgatgagtggcacggctcatggaacacctatatgaacgccccggagcacaaggatgaaggctccaccaaacgcactaacttcagcctcagcggcccgctgggcggcgattttagcttccgcctgttcggtaacctcgacaaaacgcaggctgacgcctgggatatcaaccagggccatcagtccgagcgtaccgggatctatgccgatactctgccggccgggcgcgaaggggtgaaaaacaaaaacatcgatggtctggtgcgctgggaattcgctccgatgcagtcgctggagtttgaggccggctacagccgccagggcaacctctacgccggcgatacccagaacaccaactccaacgacctggtaaaagagaactacggcaaagagaccaaccgtctgtatcgcaacacctactcggttacctggaacggcgcctgggacaacggggtgaccaccagcaactgggcgcagtacgaacgcacccgcaactcgcgcaaaggcgaaggcctggccggcggcaccgaggggatctttaacagcaaccagttcacggatatcgatctggcggatgtgatgctgcacagcgaagtcagcattcccttcgactatctggttaatcagaacctgacgctgggcagcgagtggaaccagcagcggatgaaggataacgcctccaatacccaggcgctgtcgggcggcagcatcccgggctacgacagcaccggccgcagcccgtactcgcaggcggaaatcttctcgctgttcgctgagaacaacatggagctgaccgacaccaccatgctgaccccggcgctgcgtttcgatcatcacagcatcgtgggcaataactggagcccgtccctcaacctgtcgcagggcctgtgggatgacttcacgctgaagatgggcatcgcccgcgcctataaagcgccgagcctgtatcagaccaacccgaactacattctctacagtaaaggccagggctgctatgccagtaaagacggctgctatctgcagggtaacgacgacttaaaagccgagaccagcatcaacaaagagattggcctcgagtttaaacgcgacggctggctggctggcgtcacctggttccgcaacgactaccgcaacaagattgaagcgggctatgccccggtctatcaaaacaataaaggtaccgatctctaccagtgggaaaacgtgccgaaagcggtggtggaaggtctggaggggacgttgaacgttccggtgagcgagaccgtcaactggaccaacaacatcacctatatgctgcagagtaagaacaaaaagaccggcgatcgtctgtcgattatcccggaatacacgctgaactccaccctgagctggcaggttcgcgatgacgtttcgctgcagtcgaccttcacctggtacggcaagcaggagccgaagaagtacaactacaagggtcaaccggtcaccggcagcgagaagaacgaggttagcccctacagcatcctcggcctgagcgcgacctgggacgtcaccaaatacgtcagtctgaccggcggcgtggataacgtcttcgataagcgccactggcgcgcgggcaacgcccagaccaccgggggcgccaccggcacgatgtacggcgccggcgccgagacctacaatgaatcgggccgcacctggtacctgagcgtcaacacccacttctga

SEQ ID NO: 96 - DNA, 1071 bp, Klebsiella pneumoniae
atgaaaaagacagctatcgcgattgcagtggcactggctggcttcgctaccgtagcgcaggccgctccgaaagataacacctggtatgcaggtggtaaactgggttggtcccagtatcacgacaccggtttctacggtaacggtttccagaacaacaacggtccgacccgtaacgatcagcttggtgctggtgcgttcggtggttaccaggttaacccgtacctcggtttcgaaatgggttatgactggctgggccgtatggcatataaaggcagcgttgacaacggtgctttcaaagctcagggcgttcagctgaccgctaaactgggttacccgatcactgacgatctggacatctacacccgtctgggcggcatggtttggcgcgctgactccaaaggcaactacgcttctaccggcgtttcccgtagcgaacacgacactggcgtttccccagtatttgctggcggcgtagagtgggctgttactcgtgacatcgctacccgtctggaataccagtgggttaacaacatcggcgacgcgggcactgtgggtacccgtcctgataacggcatgctgagcctgggcgtttcctaccgcttcggtcaggaagatgctgcaccggttgttgctccggctccggctccggctccggaagtggctaccaagcacttcaccctgaagtctgacgttctgttcaacttcaacaaagctaccctgaaaccggaaggtcagcaggctctggatcagctgtacactcagctgagcaacatggatccgaaagacggttccgctgttgttctgggctacaccgaccgcatcggttccgaagcttacaaccagcagctgtctgagaaacgtgctcagtccgttgttgactacctggttgctaaaggcatcccggctggcaaaatctccgctcgcggcatgggtgaatccaacccggttactggcaacacctgcgacaacgtgaaagctcgcgctgccctgatcgattgcctggctccggatcgtcgtgtagagatcgaagttaaaggctacaaagaagttgtaactcagccggcggcttaa

SEQ ID NO: 97 - DNA, 738 bp, Klebsiella pneumoniae
gtggatggatggcagcgcgcctttgtcctgcatagccgtccgtggagcgaaaccagcctgatgctggacgtcttcacggaagaatccggtcgcgtgcgcctggttgccaagggcgcacgctccaaacgctctaatctcaaaggcgctttacagccctttacccccttgttggttcgcttcggcgggcgcggcgaagtcaaaaccctgcgcagcgcggaagccgtttcgctggcgctgccgctcagcggcatcaccctctacagcggtctctacgttaacgagcttatctcccgcgtgctggagcacgaaacacgcttctccgaactctttttcgactacctgcactgcattcaggcgctcgccggggccagcggctcgccggagcccgcgctgcggcgttttgagctggcgctgctcgggcacctgggctatggcgtggattttctccactgcgccgggagcggcgagccggtagacgacaccatgacctaccgctatcgtgaagaaaaaggctttattgccagcctggtgattgataacaacacgtttaccgggcaccatttgaaagcattggcgagtcgcgagtttcctgatgttgatacgctgcgcgccgcgaagcgctttacccgtatcgccctgaagccctatctcggcggcaaaccgctcaagagccgggagttgtttcgccagtttatgcccgcgcgaaaggcgcgagccgataatacgaataatgattaa

SEQ ID NO: 98 - DNA, 4950 bp, Klebsiella pneumoniae
atgaaaccatttcgtttagcggcgctatcactggcgctccttaccgcattttcattaaccgggtgtgatgacagcggtacaccgcaggcctcggccccggcgccagccgcggatagcaacccaggcgcgacggcaaaaccggaccgcgcccagctggcggcgctggcggaaaaaagccagggtaaagcgctgacgctcctcgacgcctcggaggtgcaactggatggcgccgcgaccctggtgctgacgttttccgtcccgctgcagccggaccaggatttctcccgcagcgtgcatctggtcgacaagaaaagcggtaaggtggacggtgcctgggagctggcgccgaatctgaaagagctgcgtctgcgtcaccttgagccaaagcgcgagctgattgtctcggtcgacccgacgttgaccgccctgaacaaggcgacgctcgacaaaccgtttgagaagaccctgaccacccgcgatatcgcaccgagcgttgggtttgccagccgcggctcgctgctgccgggcaatgtggtcgccgggctgccggtgatggcgcttaacgtcgataatgtcgacgttaatttcttccgcattaagccggaatcgctctccgcctttgtcagtcagtgggaataccgtaactcgttaagcaactgggaatctgatgaactgctgaagatggcggatctggtctacagcggccgcttcgatctcaacccggcgcgtaatactcgcgaaaagctgctgctgccgctgagcgacatcaagccgctccagcagcctggcgtctacgtggcggtcatgaacccggcgggccgttatagctacagcaacgcggcgacgctgtttaccctcagcgatatcggcgtctcggcgcatcgctaccataaccggctggacgtttttacccagagtctggaaaacggcgccgcccagtcgggtattgaggtgcagttgctcaatgccaaagggcagaccctggcggaagcgaaaagcgacagccagggccacgtcaccctgcaaaccgataaagaagccgcgctgctgctggcgcgcaaagaggggcagaccacgctcctcgacctcaagctgccggcgctggatctggcggaattctctatcgcaggcgcgcccggctttagcaaacagttctttatgtttggcccgcgcgatctctatcgtcccggcgaaacggtgatccttaatgcgctgttgcgcgatagcgacggcaagccgctggcggagcagccggtgaaactggaggtggttcagccggacggccaggtgatccgctcggtgatgagtaaaccagtgaatggcctgtaccagtttacttatccgctcgacagcggcgcggctaccggcatgtggcacattcgcgccagcgccggcgacaaccagccgcgcgaatgggatttccacgttgaagactttatgccggaacgcatggccctgaacctgacgccgcaggccgcgccagtcgcgccggatgccgacgtcacctttggcgttagcggcgcttatctctacggcgcgccggccagcggcaaccagctgcagggcaagctgttcctgcgcccgctgcgcgacgccgtcgctgcgctgccgggcttccagttcggcgatattgcggaagaaaacctctcccgtagtctggatgaagtccagctgacgctggacgaaaaaggccatggcgaagtgaccacctcaagccagtggcaggatagccattcgccgctgcaggtggtgctgcaggccagcctgctggaatccggcggtcgcccggtgacccgtacggttaagcagccgatctggcccgccgaggcgctgccggggatccgcccgcaatttacgctgaaggacgtttacgattaccgcaccgataccaccgtgaaacagccggtggtggatgaaaacagtaacgccgcgtttgatatcgtctatgccgacgtcaaaggcgagaaaaaagcgatctccggtctccaggtgcggctgatccgcgagaggcgcgactactactggaactggtccgacagcgaaggctggcagtcgcagttcgatcaaaaagatctgcaggagggcgaggagtcgctggacctgcaggccggccagatcggcaaagtgagcttcccggtggagtggggatcctatcgcctggaggtgaaaggaccggacgacgtggtcagcagcgtgcgcttctgggcgggctacagctggcaggataacagcgaaggcgccggcgcggcgcgtcctgaccgggtcaccatgaagctggataaaccgagctataaaccgggcgacaccatcaggctgcacatcgccgccccggcggcgggtaaaggctacgcaatggtggaatccagcgaagggccgctgtggtggcaggaaattgacgtcccggcggaggggatggacctgtcgatcccggtggataaaacctggaatcgccacgacctctacctcagcacgctggtggttcgtcccggcgataaatcgcgctcggcaacgccgaaacgcgcggtgggcctgctgcatctgccgctgggcgatgaaaaccgtcgcctgacgctggcgctggaggccccggacaaaatgcgccccaaccagccgctgacggtgaaagtgaaagccagcgtcaaagagggcgaggcgccgaaacaggtcaatgtcctgctctcggcggtggatagcggggtactgaatatcaccgattacgctaccccggatccgtggaacgccttctttggccagaagcgttacggcgcagatatctatgacatctacggccaggtgatcgaagggcagggacgtgtggccagcctgcgcttcggcggcgatggcgacgagttaaaacgcggcggcaaaccgccggttaaccacgtgacgatcgtcgcccagcaggcgcagccggtggtattgaacgatcagggcgaaggcacggtgacgttacccattggcgattttaacggcgagctgcgggtgatggcccaggcgtggacggcggatgacttcggcagcagcgaagataaagtggtggtggccgccccggtcatcgccgagctgaacactccgcgcttcctcgccagcggcgatactacgcgtctggcgctggatctcagcaatctgaccgataaaccgcaaaccctgcaggttcaccttaccgccagcgggctggtaacgttgagcgagggtcaactgccgccggtacagctggcgccgggggcgcgcagcacgctgtttataccagtgagcgcgctggcgggcttcggcgatggtcaggttaatgccaccatcagcggcctgagcctgccgggcgaaaccttcgccccgctgcaaaaacagtggaaaatcggcgtgcgtccggcgtacccggcacagaccgtcaacagcggcgcagtgctgcagccaggtgaaagctggcagccgccggcggcgcagagccagggctttgccccgcaaacgctgcagggccaactgctgctcagcggtaaaccaccgttgaatctcgcccgctatatccgcgagctgaaagcctatccttacggctgccttgagcagaccgccagcggcctgttcccgtccctgtataccagcgcggcgcagctaaaggcgctgggcattagcggggacagcgacgaaaaacgccgcgcggccatcgatgtcggtatttcacgcctgctgcagatgcagctggaaaacggcggctttgcgctatgggatagagaggggccggaagagtactggctgaccgcctacgccatggacttcctcgtgcgcgccagcgagcagggctatagcgtaccggtcaacgccattaataaaggcaacgagcgcctgctgcgctatctgcaggagccgggcctgatgaccgtgcgctacagcgacgacgcccaggctagccgctttgccgcccaggcatacgccgcgctggtgctggcgcgtcagcaaaaagcgccgctcggcgccttgcgtgaaatctggagccgtcacgaccaggcgcgatccggcttgccgctgctgcagctcggcattgcgctgaaaactatgggcgatgcgccgcgcggcgacgccgccctgaagctggcggttgccaccccgcgccaggatgagaatcgttggctgggcgattacggtagcccgctgcgcgataacgccctgaagctggcgctgctggaagagaataagctgctgccggaggtgcaaactcagctgttgagcacgctgtcggaagaggcctatggccagcgctggctgtcgacccaggaaaccaacgccttgttccttgccggacgtacgctggcggacctgccgggcagctggcaggcgcaaacctcgctgcaggcggagccgctggccggcgacaaagcgcaaacccgcaacctcgacggcgatcggctggcggcgctgcaggtgagtaataccggcagtcagccgctgtggctgcgtctcgacagcagcggctatccgcaaagcgcgccgcagccgggcggtaacgtcctggggattgaacgcactattttcgatacccaggggcagcagaaatcgctgtcttcactgcgcagcggcgaactggtgctcgtcaagctggaggtgaccgccaaacgcaacgtgcctgacgcgctggtggttgatctgttgccagccggtctggagctggaaaaccagaatctggccaacagcagcgccagcctgcaggagaatggcgacgcggtgcaaaacctgcttaaccagatgcagcaggcggatattcagcatatcgagttccgcgatgaccgtttcgtcgccgccgtcgctgtcaatgaaggccagccggtgacgctggtctatctggcgcgggcggtgacgccgggcacttatcaggtcccgcagccgcaggtggaatcgatgtatgcgccgcagtggcgggcgacaggagcggccagcggtccgctcaccgtgacgccgtaa

SEQ ID NO: 99 - RNA, 2229 nt, Klebsiella pneumoniae
augaauaacaggaucaaaucccuggccuugcuggucaaucugggaauuuacgggguugcuuuuccguuaagcgcagcggaaaccgccaccgacgauaaaaacagcgccgcugaagagaccaugguggucaccgccgccgagcagaaccugcaggcgccgggcgucuccaccaucaccgccgaugagauccgcaaacgccccccggcgcgcgacgucucggagaucauucgcaccaugccgggggucaaccugaccggcaacuccaccagcggccagcgcggcaacaaccgccagauugauauccgcggcaugggcccggaaaauacccugauccugaucgacggcaagccggucaccagccgcaacuccgugcgccuuggcuggcgcggcgagcgcgacacccgcggcgauaccagcugggugccgccggagaugaucgaacguaucgaagugauucgcggcccggccgccgcccgcuacggcaacggcgccgccggcggcguggugaauaucaucaccaaaaaaaccggcgaugaguggcacggcucauggaacaccuauaugaacgccccggagcacaaggaugaaggcuccaccaaacgcacuaacuucagccucagcggcccgcugggcggcgauuuuagcuuccgccuguucgguaaccucgacaaaacgcaggcugacgccugggauaucaaccagggccaucaguccgagcguaccgggaucuaugccgauacucugccggccgggcgcgaaggggugaaaaacaaaaacaucgauggucuggugcgcugggaauucgcuccgaugcagucgcuggaguuugaggccggcuacagccgccagggcaaccucuacgccggcgauacccagaacaccaacuccaacgaccugguaaaagagaacuacggcaaagagaccaaccgucuguaucgcaacaccuacucgguuaccuggaacggcgccugggacaacggggugaccaccagcaacugggcgcaguacgaacgcacccgcaacucgcgcaaaggcgaaggccuggccggcggcaccgaggggaucuuuaacagcaaccaguucacggauaucgaucuggcggaugugaugcugcacagcgaagucagcauucccuucgacuaucugguuaaucagaaccugacgcugggcagcgaguggaaccagcagcggaugaaggauaacgccuccaauacccaggcgcugucgggcggcagcaucccgggcuacgacagcaccggccgcagcccguacucgcaggcggaaaucuucucgcuguucgcugagaacaacauggagcugaccgacaccaccaugcugaccccggcgcugcguuucgaucaucacagcaucgugggcaauaacuggagcccgucccucaaccugucgcagggccugugggaugacuucacgcugaagaugggcaucgcccgcgccuauaaagcgccgagccuguaucagaccaacccgaacuacauucucuacaguaaaggccagggcugcuaugccaguaaagacggcugcuaucugcaggguaacgacgacuuaaaagccgagaccagcaucaacaaagagauuggccucgaguuuaaacgcgacggcuggcuggcuggcgucaccugguuccgcaacgacuaccgcaacaagauugaagcgggcuaugccccggucuaucaaaacaauaaagguaccgaucucuaccagugggaaaacgugccgaaagcggugguggaaggucuggaggggacguugaacguuccggugagcgagaccgucaacuggaccaacaacaucaccuauaugcugcagaguaagaacaaaaagaccggcgaucgucugucgauuaucccggaauacacgcugaacuccacccugagcuggcagguucgcgaugacguuucgcugcagucgaccuucaccugguacggcaagcaggagccgaagaaguacaacuacaagggucaaccggucaccggcagcgagaagaacgagguuagccccuacagcauccucggccugagcgcgaccugggacgucaccaaauacgucagucugaccggcggcguggauaacgucuucgauaagcgccacuggcgcgcgggcaacgcccagaccaccgggggcgccaccggcacgauguacggcgccggcgccgagaccuacaaugaaucgggccgcaccugguaccugagcgucaacacccacuucuga

SEQ ID NO: 100 - RNA, 1071 nt, Klebsiella pneumoniae
augaaaaagacagcuaucgcgauugcaguggcacuggcuggcuucgcuaccguagcgcaggccgcuccgaaagauaacaccugguaugcaggugguaaacuggguuggucccaguaucacgacaccgguuucuacgguaacgguuuccagaacaacaacgguccgacccguaacgaucagcuuggugcuggugcguucggugguuaccagguuaacccguaccucgguuucgaaauggguuaugacuggcugggccguauggcauauaaaggcagcguugacaacggugcuuucaaagcucagggcguucagcugaccgcuaaacuggguuacccgaucacugacgaucuggacaucuacacccgucugggcggcaugguuuggcgcgcugacuccaaaggcaacuacgcuucuaccggcguuucccguagcgaacacgacacuggcguuuccccaguauuugcuggcggcguagagugggcuguuacucgugacaucgcuacccgucuggaauaccaguggguuaacaacaucggcgacgcgggcacuguggguacccguccugauaacggcaugcugagccugggcguuuccuaccgcuucggucaggaagaugcugcaccgguuguugcuccggcuccggcuccggcuccggaaguggcuaccaagcacuucacccugaagucugacguucuguucaacuucaacaaagcuacccugaaaccggaaggucagcaggcucuggaucagcuguacacucagcugagcaacauggauccgaaagacgguuccgcuguuguucugggcuacaccgaccgcaucgguuccgaagcuuacaaccagcagcugucugagaaacgugcucaguccguuguugacuaccugguugcuaaaggcaucccggcuggcaaaaucuccgcucgcggcaugggugaauccaacccgguuacuggcaacaccugcgacaacgugaaagcucgcgcugcccugaucgauugccuggcuccggaucgucguguagagaucgaaguuaaaggcuacaaagaaguuguaacucagccggcggcuuaa

SEQ ID NO: 101 - RNA, 738 nt, Klebsiella pneumoniae
guggauggauggcagcgcgccuuuguccugcauagccguccguggagcgaaaccagccugaugcuggacgucuucacggaagaauccggucgcgugcgccugguugccaagggcgcacgcuccaaacgcucuaaucucaaaggcgcuuuacagcccuuuacccccuuguugguucgcuucggcgggcgcggcgaagucaaaacccugcgcagcgcggaagccguuucgcuggcgcugccgcucagcggcaucacccucuacagcggucucuacguuaacgagcuuaucucccgcgugcuggagcacgaaacacgcuucuccgaacucuuuuucgacuaccugcacugcauucaggcgcucgccggggccagcggcucgccggagcccgcgcugcggcguuuugagcuggcgcugcucgggcaccugggcuauggcguggauuuucuccacugcgccgggagcggcgagccgguagacgacaccaugaccuaccgcuaucgugaagaaaaaggcuuuauugccagccuggugauugauaacaacacguuuaccgggcaccauuugaaagcauuggcgagucgcgaguuuccugauguugauacgcugcgcgccgcgaagcgcuuuacccguaucgcccugaagcccuaucucggcggcaaaccgcucaagagccgggaguuguuucgccaguuuaugcccgcgcgaaaggcgcgagccgauaauacgaauaaugauuaa

SEQ ID NO: 102 - RNA, 4950 nt, Klebsiella pneumoniae
augaaaccauuucguuuagcggcgcuaucacuggcgcuccuuaccgcauuuucauuaaccgggugugaugacagcgguacaccgcaggccucggccccggcgccagccgcggauagcaacccaggcgcgacggcaaaaccggaccgcgcccagcuggcggcgcuggcggaaaaaagccaggguaaagcgcugacgcuccucgacgccucggaggugcaacuggauggcgccgcgacccuggugcugacguuuuccgucccgcugcagccggaccaggauuucucccgcagcgugcaucuggucgacaagaaaagcgguaagguggacggugccugggagcuggcgccgaaucugaaagagcugcgucugcgucaccuugagccaaagcgcgagcugauugucucggucgacccgacguugaccgcccugaacaaggcgacgcucgacaaaccguuugagaagacccugaccacccgcgauaucgcaccgagcguuggguuugccagccgcggcucgcugcugccgggcaauguggucgccgggcugccggugauggcgcuuaacgucgauaaugucgacguuaauuucuuccgcauuaagccggaaucgcucuccgccuuugucagucagugggaauaccguaacucguuaagcaacugggaaucugaugaacugcugaagauggcggaucuggucuacagcggccgcuucgaucucaacccggcgcguaauacucgcgaaaagcugcugcugccgcugagcgacaucaagccgcuccagcagccuggcgucuacguggcggucaugaacccggcgggccguuauagcuacagcaacgcggcgacgcuguuuacccucagcgauaucggcgucucggcgcaucgcuaccauaaccggcuggacguuuuuacccagagucuggaaaacggcgccgcccagucggguauugaggugcaguugcucaaugccaaagggcagacccuggcggaagcgaaaagcgacagccagggccacgucacccugcaaaccgauaaagaagccgcgcugcugcuggcgcgcaaagaggggcagaccacgcuccucgaccucaagcugccggcgcuggaucuggcggaauucucuaucgcaggcgcgcccggcuuuagcaaacaguucuuuauguuuggcccgcgcgaucucuaucgucccggcgaaacggugauccuuaaugcgcuguugcgcgauagcgacggcaagccgcuggcggagcagccggugaaacuggaggugguucagccggacggccaggugauccgcucggugaugaguaaaccagugaauggccuguaccaguuuacuuauccgcucgacagcggcgcggcuaccggcauguggcacauucgcgccagcgccggcgacaaccagccgcgcgaaugggauuuccacguugaagacuuuaugccggaacgcauggcccugaaccugacgccgcaggccgcgccagucgcgccggaugccgacgucaccuuuggcguuagcggcgcuuaucucuacggcgcgccggccagcggcaaccagcugcagggcaagcuguuccugcgcccgcugcgcgacgccgucgcugcgcugccgggcuuccaguucggcgauauugcggaagaaaaccucucccguagucuggaugaaguccagcugacgcuggacgaaaaaggccauggcgaagugaccaccucaagccaguggcaggauagccauucgccgcugcagguggugcugcaggccagccugcuggaauccggcggucgcccggugacccguacgguuaagcagccgaucuggcccgccgaggcgcugccggggauccgcccgcaauuuacgcugaaggacguuuacgauuaccgcaccgauaccaccgugaaacagccggugguggaugaaaacaguaacgccgcguuugauaucgucuaugccgacgucaaaggcgagaaaaaagcgaucuccggucuccaggugcggcugauccgcgagaggcgcgacuacuacuggaacugguccgacagcgaaggcuggcagucgcaguucgaucaaaaagaucugcaggagggcgaggagucgcuggaccugcaggccggccagaucggcaaagugagcuucccgguggaguggggauccuaucgccuggaggugaaaggaccggacgacguggucagcagcgugcgcuucugggcgggcuacagcuggcaggauaacagcgaaggcgccggcgcggcgcguccugaccgggucaccaugaagcuggauaaaccgagcuauaaaccgggcgacaccaucaggcugcacaucgccgccccggcggcggguaaaggcuacgcaaugguggaauccagcgaagggccgcugugguggcaggaaauugacgucccggcggaggggauggaccugucgaucccgguggauaaaaccuggaaucgccacgaccucuaccucagcacgcuggugguucgucccggcgauaaaucgcgcucggcaacgccgaaacgcgcggugggccugcugcaucugccgcugggcgaugaaaaccgucgccugacgcuggcgcuggaggccccggacaaaaugcgccccaaccagccgcugacggugaaagugaaagccagcgucaaagagggcgaggcgccgaaacaggucaauguccugcucucggcgguggauagcgggguacugaauaucaccgauuacgcuaccccggauccguggaacgccuucuuuggccagaagcguuacggcgcagauaucuaugacaucuacggccaggugaucgaagggcagggacguguggccagccugcgcuucggcggcgauggcgacgaguuaaaacgcggcggcaaaccgccgguuaaccacgugacgaucgucgcccagcaggcgcagccggugguauugaacgaucagggcgaaggcacggugacguuacccauuggcgauuuuaacggcgagcugcgggugauggcccaggcguggacggcggaugacuucggcagcagcgaagauaaaguggugguggccgccccggucaucgccgagcugaacacuccgcgcuuccucgccagcggcgauacuacgcgucuggcgcuggaucucagcaaucugaccgauaaaccgcaaacccugcagguucaccuuaccgccagcgggcugguaacguugagcgagggucaacugccgccgguacagcuggcgccgggggcgcgcagcacgcuguuuauaccagugagcgcgcuggcgggcuucggcgauggucagguuaaugccaccaucagcggccugagccugccgggcgaaaccuucgccccgcugcaaaaacaguggaaaaucggcgugcguccggcguacccggcacagaccgucaacagcggcgcagugcugcagccaggugaaagcuggcagccgccggcggcgcagagccagggcuuugccccgcaaacgcugcagggccaacugcugcucagcgguaaaccaccguugaaucucgcccgcuauauccgcgagcugaaagccuauccuuacggcugccuugagcagaccgccagcggccuguucccgucccuguauaccagcgcggcgcagcuaaaggcgcugggcauuagcggggacagcgacgaaaaacgccgcgcggccaucgaugucgguauuucacgccugcugcagaugcagcuggaaaacggcggcuuugcgcuaugggauagagaggggccggaagaguacuggcugaccgccuacgccauggacuuccucgugcgcgccagcgagcagggcuauagcguaccggucaacgccauuaauaaaggcaacgagcgccugcugcgcuaucugcaggagccgggccugaugaccgugcgcuacagcgacgacgcccaggcuagccgcuuugccgcccaggcauacgccgcgcuggugcuggcgcgucagcaaaaagcgccgcucggcgccuugcgugaaaucuggagccgucacgaccaggcgcgauccggcuugccgcugcugcagcucggcauugcgcugaaaacuaugggcgaugcgccgcgcggcgacgccgcccugaagcuggcgguugccaccccgcgccaggaugagaaucguuggcugggcgauuacgguagcccgcugcgcgauaacgcccugaagcuggcgcugcuggaagagaauaagcugcugccggaggugcaaacucagcuguugagcacgcugucggaagaggccuauggccagcgcuggcugucgacccaggaaaccaacgccuuguuccuugccggacguacgcuggcggaccugccgggcagcuggcaggcgcaaaccucgcugcaggcggagccgcuggccggcgacaaagcgcaaacccgcaaccucgacggcgaucggcuggcggcgcugcaggugaguaauaccggcagucagccgcuguggcugcgucucgacagcagcggcuauccgcaaagcgcgccgcagccgggcgguaacguccuggggauugaacgcacuauuuucgauacccaggggcagcagaaaucgcugucuucacugcgcagcggcgaacuggugcucgucaagcuggaggugaccgccaaacgcaacgugccugacgcgcuggugguugaucuguugccagccggucuggagcuggaaaaccagaaucuggccaacagcagcgccagccugcaggagaauggcgacgcggugcaaaaccugcuuaaccagaugcagcaggcggauauucagcauaucgaguuccgcgaugaccguuucgucgccgccgucgcugucaaugaaggccagccggugacgcuggucuaucuggcgcgggcggugacgccgggcacuuaucaggucccgcagccgcagguggaaucgauguaugcgccgcaguggcgggcgacaggagcggccagcgguccgcucaccgugacgccguaa